European Patent Application EP 4 272 754 A1, published November 8, 2023. Title: METHOD FOR PRODUCING CELLS EXPRESSING A CHIMERIC ANTIGEN RECEPTOR (CAR). Applicant: Universitätsklinikum Hamburg-Eppendorf. The sequence listing filed with the application follows.

SEQUENCE LISTING (12 sequences)

SEQ ID NO: 1 - protein, 1306 aa, Homo sapiens
  CD45RABC
MTMYLWLKLLAFGFAFLDTEVFVTGQSPTPSPTGLTTAKMPSVPLSSDPLPTHTTAFSPASTFERENDFSETTTSLSPDNTSTQVSPDSLDNASAFNTTGVSSVQTPHLPTHADSQTPSAGTDTQTFSGSAANAKLNPTPGSNAISDVPGERSTASTFPTDPVSPLTTTLSLAHHSSAALPARTSNTTITANTSDAYLNASETTTLSPSGSAVISTTTIATTPSKPTCDEKYANITVDYLYNKETKLFTAKLNVNENVECGNNTCTNNEVHNLTECKNASVSISHNSCTAPDKTLILDVPPGVEKFQLHDCTQVEKADTTICLKWKNIETFTCDTQNITYRFQCGNMIFDNKEIKLENLEPEHEYKCDSEILYNNHKFTNASKIIKTDFGSPGEPQIIFCRSEAAHQGVITWNPPQRSFHNFTLCYIKETEKDCLNLDKNLIKYDLQNLKPYTKYVLSLHAYIIAKVQRNGSAAMCHFTTKSAPPSQVWNMTVSMTSDNSMHVKCRPPRDRNGPHERYHLEVEAGNTLVRNESHKNCDFRVKDLQYSTDYTFKAYFHNGDYPGEPFILHHSTSYNSKALIAFLAFLIIVTSIALLVVLYKIYDLHKKRSCNLDEQQELVERDDEKQLMNVEPIHADILLETYKRKIADEGRLFLAEFQSIPRVFSKFPIKEARKPFNQNKNRYVDILPYDYNRVELSEINGDAGSNYINASYIDGFKEPRKYIAAQGPRDETVDDFWRMIWEQKATVIVMVTRCEEGNRNKCAEYWPSMEEGTRAFGDVVVKINQHKRCPDYIIQKLNIVNKKEKATGREVTHIQFTSWPDHGVPEDPHLLLKLRRRVNAFSNFFSGPIVVHCSAGVGRTGTYIGIDAMLEGLEAENKVDVYGYVVKLRRQRCLMVQVEAQYILIHQALVEYNQFGETEVNLSELHPYLHNMKKRDPPSEPSPLEAEFQRLPSYRSWRTQHIGNQEENKSKNRNSNVIPYDYNRVPLKHELEMSKESEHDSDESSDDDSDSEEPSKYINASFIMSYWKPEVMIAAQGPLKETIGDFWQMIFQRKVKVIVMLTELKHGDQEICAQYWGEGKQTYGDIEVDLKDTDKSSTYTLRVFELRHSKRKDSRTVYQYQYTNWSVEQLPAEPKELISMIQVVKQKLPQKNSSEGNKHHKSTPLLIHCRDGSQQTGIFCALLNLLESAETEEVVDIFQVVKALRKARPGMVSTFEQYQFLYDVIASTYPAQNGQVKKNNHQEDKIEFDNEVDKVKQDANCVNPLGAPEKLPEAKEQAEGSEPTSGTEGPEHSVNGPASPALNQGS

SEQ ID NO: 2 - protein, 1145 aa, Homo sapiens
  CD45R0
MTMYLWLKLLAFGFAFLDTEVFVTGQSPTPSPTDAYLNASETTTLSPSGSAVISTTTIATTPSKPTCDEKYANITVDYLYNKETKLFTAKLNVNENVECGNNTCTNNEVHNLTECKNASVSISHNSCTAPDKTLILDVPPGVEKFQLHDCTQVEKADTTICLKWKNIETFTCDTQNITYRFQCGNMIFDNKEIKLENLEPEHEYKCDSEILYNNHKFTNASKIIKTDFGSPGEPQIIFCRSEAAHQGVITWNPPQRSFHNFTLCYIKETEKDCLNLDKNLIKYDLQNLKPYTKYVLSLHAYIIAKVQRNGSAAMCHFTTKSAPPSQVWNMTVSMTSDNSMHVKCRPPRDRNGPHERYHLEVEAGNTLVRNESHKNCDFRVKDLQYSTDYTFKAYFHNGDYPGEPFILHHSTSYNSKALIAFLAFLIIVTSIALLVVLYKIYDLHKKRSCNLDEQQELVERDDEKQLMNVEPIHADILLETYKRKIADEGRLFLAEFQSIPRVFSKFPIKEARKPFNQNKNRYVDILPYDYNRVELSEINGDAGSNYINASYIDGFKEPRKYIAAQGPRDETVDDFWRMIWEQKATVIVMVTRCEEGNRNKCAEYWPSMEEGTRAFGDVVVKINQHKRCPDYIIQKLNIVNKKEKATGREVTHIQFTSWPDHGVPEDPHLLLKLRRRVNAFSNFFSGPIVVHCSAGVGRTGTYIGIDAMLEGLEAENKVDVYGYVVKLRRQRCLMVQVEAQYILIHQALVEYNQFGETEVNLSELHPYLHNMKKRDPPSEPSPLEAEFQRLPSYRSWRTQHIGNQEENKSKNRNSNVIPYDYNRVPLKHELEMSKESEHDSDESSDDDSDSEEPSKYINASFIMSYWKPEVMIAAQGPLKETIGDFWQMIFQRKVKVIVMLTELKHGDQEICAQYWGEGKQTYGDIEVDLKDTDKSSTYTLRVFELRHSKRKDSRTVYQYQYTNWSVEQLPAEPKELISMIQVVKQKLPQKNSSEGNKHHKSTPLLIHCRDGSQQTGIFCALLNLLESAETEEVVDIFQVVKALRKARPGMVSTFEQYQFLYDVIASTYPAQNGQVKKNNHQEDKIEFDNEVDKVKQDANCVNPLGAPEKLPEAKEQAEGSEPTSGTEGPEHSVNGPASPALNQGS

SEQ ID NO: 3 - protein, 1258 aa, Homo sapiens
  CD45RAB
MTMYLWLKLLAFGFAFLDTEVFVTGQSPTPSPTGLTTAKMPSVPLSSDPLPTHTTAFSPASTFERENDFSETTTSLSPDNTSTQVSPDSLDNASAFNTTGVSSVQTPHLPTHADSQTPSAGTDTQTFSGSAANAKLNPTPGSNAISDAYLNASETTTLSPSGSAVISTTTIATTPSKPTCDEKYANITVDYLYNKETKLFTAKLNVNENVECGNNTCTNNEVHNLTECKNASVSISHNSCTAPDKTLILDVPPGVEKFQLHDCTQVEKADTTICLKWKNIETFTCDTQNITYRFQCGNMIFDNKEIKLENLEPEHEYKCDSEILYNNHKFTNASKIIKTDFGSPGEPQIIFCRSEAAHQGVITWNPPQRSFHNFTLCYIKETEKDCLNLDKNLIKYDLQNLKPYTKYVLSLHAYIIAKVQRNGSAAMCHFTTKSAPPSQVWNMTVSMTSDNSMHVKCRPPRDRNGPHERYHLEVEAGNTLVRNESHKNCDFRVKDLQYSTDYTFKAYFHNGDYPGEPFILHHSTSYNSKALIAFLAFLIIVTSIALLVVLYKIYDLHKKRSCNLDEQQELVERDDEKQLMNVEPIHADILLETYKRKIADEGRLFLAEFQSIPRVFSKFPIKEARKPFNQNKNRYVDILPYDYNRVELSEINGDAGSNYINASYIDGFKEPRKYIAAQGPRDETVDDFWRMIWEQKATVIVMVTRCEEGNRNKCAEYWPSMEEGTRAFGDVVVKINQHKRCPDYIIQKLNIVNKKEKATGREVTHIQFTSWPDHGVPEDPHLLLKLRRRVNAFSNFFSGPIVVHCSAGVGRTGTYIGIDAMLEGLEAENKVDVYGYVVKLRRQRCLMVQVEAQYILIHQALVEYNQFGETEVNLSELHPYLHNMKKRDPPSEPSPLEAEFQRLPSYRSWRTQHIGNQEENKSKNRNSNVIPYDYNRVPLKHELEMSKESEHDSDESSDDDSDSEEPSKYINASFIMSYWKPEVMIAAQGPLKETIGDFWQMIFQRKVKVIVMLTELKHGDQEICAQYWGEGKQTYGDIEVDLKDTDKSSTYTLRVFELRHSKRKDSRTVYQYQYTNWSVEQLPAEPKELISMIQVVKQKLPQKNSSEGNKHHKSTPLLIHCRDGSQQTGIFCALLNLLESAETEEVVDIFQVVKALRKARPGMVSTFEQYQFLYDVIASTYPAQNGQVKKNNHQEDKIEFDNEVDKVKQDANCVNPLGAPEKLPEAKEQAEGSEPTSGTEGPEHSVNGPASPALNQGS

SEQ ID NO: 4 - protein, 1259 aa, Homo sapiens
  CD45RAC
MTMYLWLKLLAFGFAFLDTEVFVTGQSPTPSPTGLTTAKMPSVPLSSDPLPTHTTAFSPASTFERENDFSETTTSLSPDNTSTQVSPDSLDNASAFNTTDVPGERSTASTFPTDPVSPLTTTLSLAHHSSAALPARTSNTTITANTSDAYLNASETTTLSPSGSAVISTTTIATTPSKPTCDEKYANITVDYLYNKETKLFTAKLNVNENVECGNNTCTNNEVHNLTECKNASVSISHNSCTAPDKTLILDVPPGVEKFQLHDCTQVEKADTTICLKWKNIETFTCDTQNITYRFQCGNMIFDNKEIKLENLEPEHEYKCDSEILYNNHKFTNASKIIKTDFGSPGEPQIIFCRSEAAHQGVITWNPPQRSFHNFTLCYIKETEKDCLNLDKNLIKYDLQNLKPYTKYVLSLHAYIIAKVQRNGSAAMCHFTTKSAPPSQVWNMTVSMTSDNSMHVKCRPPRDRNGPHERYHLEVEAGNTLVRNESHKNCDFRVKDLQYSTDYTFKAYFHNGDYPGEPFILHHSTSYNSKALIAFLAFLIIVTSIALLVVLYKIYDLHKKRSCNLDEQQELVERDDEKQLMNVEPIHADILLETYKRKIADEGRLFLAEFQSIPRVFSKFPIKEARKPFNQNKNRYVDILPYDYNRVELSEINGDAGSNYINASYIDGFKEPRKYIAAQGPRDETVDDFWRMIWEQKATVIVMVTRCEEGNRNKCAEYWPSMEEGTRAFGDVVVKINQHKRCPDYIIQKLNIVNKKEKATGREVTHIQFTSWPDHGVPEDPHLLLKLRRRVNAFSNFFSGPIVVHCSAGVGRTGTYIGIDAMLEGLEAENKVDVYGYVVKLRRQRCLMVQVEAQYILIHQALVEYNQFGETEVNLSELHPYLHNMKKRDPPSEPSPLEAEFQRLPSYRSWRTQHIGNQEENKSKNRNSNVIPYDYNRVPLKHELEMSKESEHDSDESSDDDSDSEEPSKYINASFIMSYWKPEVMIAAQGPLKETIGDFWQMIFQRKVKVIVMLTELKHGDQEICAQYWGEGKQTYGDIEVDLKDTDKSSTYTLRVFELRHSKRKDSRTVYQYQYTNWSVEQLPAEPKELISMIQVVKQKLPQKNSSEGNKHHKSTPLLIHCRDGSQQTGIFCALLNLLESAETEEVVDIFQVVKALRKARPGMVSTFEQYQFLYDVIASTYPAQNGQVKKNNHQEDKIEFDNEVDKVKQDANCVNPLGAPEKLPEAKEQAEGSEPTSGTEGPEHSVNGPASPALNQGS

SEQ ID NO: 5 - protein, 1240 aa, Homo sapiens
  CD45RBC
MTMYLWLKLLAFGFAFLDTEVFVTGQSPTPSPTGVSSVQTPHLPTHADSQTPSAGTDTQTFSGSAANAKLNPTPGSNAISDVPGERSTASTFPTDPVSPLTTTLSLAHHSSAALPARTSNTTITANTSDAYLNASETTTLSPSGSAVISTTTIATTPSKPTCDEKYANITVDYLYNKETKLFTAKLNVNENVECGNNTCTNNEVHNLTECKNASVSISHNSCTAPDKTLILDVPPGVEKFQLHDCTQVEKADTTICLKWKNIETFTCDTQNITYRFQCGNMIFDNKEIKLENLEPEHEYKCDSEILYNNHKFTNASKIIKTDFGSPGEPQIIFCRSEAAHQGVITWNPPQRSFHNFTLCYIKETEKDCLNLDKNLIKYDLQNLKPYTKYVLSLHAYIIAKVQRNGSAAMCHFTTKSAPPSQVWNMTVSMTSDNSMHVKCRPPRDRNGPHERYHLEVEAGNTLVRNESHKNCDFRVKDLQYSTDYTFKAYFHNGDYPGEPFILHHSTSYNSKALIAFLAFLIIVTSIALLVVLYKIYDLHKKRSCNLDEQQELVERDDEKQLMNVEPIHADILLETYKRKIADEGRLFLAEFQSIPRVFSKFPIKEARKPFNQNKNRYVDILPYDYNRVELSEINGDAGSNYINASYIDGFKEPRKYIAAQGPRDETVDDFWRMIWEQKATVIVMVTRCEEGNRNKCAEYWPSMEEGTRAFGDVVVKINQHKRCPDYIIQKLNIVNKKEKATGREVTHIQFTSWPDHGVPEDPHLLLKLRRRVNAFSNFFSGPIVVHCSAGVGRTGTYIGIDAMLEGLEAENKVDVYGYVVKLRRQRCLMVQVEAQYILIHQALVEYNQFGETEVNLSELHPYLHNMKKRDPPSEPSPLEAEFQRLPSYRSWRTQHIGNQEENKSKNRNSNVIPYDYNRVPLKHELEMSKESEHDSDESSDDDSDSEEPSKYINASFIMSYWKPEVMIAAQGPLKETIGDFWQMIFQRKVKVIVMLTELKHGDQEICAQYWGEGKQTYGDIEVDLKDTDKSSTYTLRVFELRHSKRKDSRTVYQYQYTNWSVEQLPAEPKELISMIQVVKQKLPQKNSSEGNKHHKSTPLLIHCRDGSQQTGIFCALLNLLESAETEEVVDIFQVVKALRKARPGMVSTFEQYQFLYDVIASTYPAQNGQVKKNNHQEDKIEFDNEVDKVKQDANCVNPLGAPEKLPEAKEQAEGSEPTSGTEGPEHSVNGPASPALNQGS

SEQ ID NO: 6 - protein, 1211 aa, Homo sapiens
  CD45RA
MTMYLWLKLLAFGFAFLDTEVFVTGQSPTPSPTGLTTAKMPSVPLSSDPLPTHTTAFSPASTFERENDFSETTTSLSPDNTSTQVSPDSLDNASAFNTTDAYLNASETTTLSPSGSAVISTTTIATTPSKPTCDEKYANITVDYLYNKETKLFTAKLNVNENVECGNNTCTNNEVHNLTECKNASVSISHNSCTAPDKTLILDVPPGVEKFQLHDCTQVEKADTTICLKWKNIETFTCDTQNITYRFQCGNMIFDNKEIKLENLEPEHEYKCDSEILYNNHKFTNASKIIKTDFGSPGEPQIIFCRSEAAHQGVITWNPPQRSFHNFTLCYIKETEKDCLNLDKNLIKYDLQNLKPYTKYVLSLHAYIIAKVQRNGSAAMCHFTTKSAPPSQVWNMTVSMTSDNSMHVKCRPPRDRNGPHERYHLEVEAGNTLVRNESHKNCDFRVKDLQYSTDYTFKAYFHNGDYPGEPFILHHSTSYNSKALIAFLAFLIIVTSIALLVVLYKIYDLHKKRSCNLDEQQELVERDDEKQLMNVEPIHADILLETYKRKIADEGRLFLAEFQSIPRVFSKFPIKEARKPFNQNKNRYVDILPYDYNRVELSEINGDAGSNYINASYIDGFKEPRKYIAAQGPRDETVDDFWRMIWEQKATVIVMVTRCEEGNRNKCAEYWPSMEEGTRAFGDVVVKINQHKRCPDYIIQKLNIVNKKEKATGREVTHIQFTSWPDHGVPEDPHLLLKLRRRVNAFSNFFSGPIVVHCSAGVGRTGTYIGIDAMLEGLEAENKVDVYGYVVKLRRQRCLMVQVEAQYILIHQALVEYNQFGETEVNLSELHPYLHNMKKRDPPSEPSPLEAEFQRLPSYRSWRTQHIGNQEENKSKNRNSNVIPYDYNRVPLKHELEMSKESEHDSDESSDDDSDSEEPSKYINASFIMSYWKPEVMIAAQGPLKETIGDFWQMIFQRKVKVIVMLTELKHGDQEICAQYWGEGKQTYGDIEVDLKDTDKSSTYTLRVFELRHSKRKDSRTVYQYQYTNWSVEQLPAEPKELISMIQVVKQKLPQKNSSEGNKHHKSTPLLIHCRDGSQQTGIFCALLNLLESAETEEVVDIFQVVKALRKARPGMVSTFEQYQFLYDVIASTYPAQNGQVKKNNHQEDKIEFDNEVDKVKQDANCVNPLGAPEKLPEAKEQAEGSEPTSGTEGPEHSVNGPASPALNQGS

SEQ ID NO: 7 - protein, 1192 aa, Homo sapiens
  CD45RB
MTMYLWLKLLAFGFAFLDTEVFVTGQSPTPSPTGVSSVQTPHLPTHADSQTPSAGTDTQTFSGSAANAKLNPTPGSNAISDAYLNASETTTLSPSGSAVISTTTIATTPSKPTCDEKYANITVDYLYNKETKLFTAKLNVNENVECGNNTCTNNEVHNLTECKNASVSISHNSCTAPDKTLILDVPPGVEKFQLHDCTQVEKADTTICLKWKNIETFTCDTQNITYRFQCGNMIFDNKEIKLENLEPEHEYKCDSEILYNNHKFTNASKIIKTDFGSPGEPQIIFCRSEAAHQGVITWNPPQRSFHNFTLCYIKETEKDCLNLDKNLIKYDLQNLKPYTKYVLSLHAYIIAKVQRNGSAAMCHFTTKSAPPSQVWNMTVSMTSDNSMHVKCRPPRDRNGPHERYHLEVEAGNTLVRNESHKNCDFRVKDLQYSTDYTFKAYFHNGDYPGEPFILHHSTSYNSKALIAFLAFLIIVTSIALLVVLYKIYDLHKKRSCNLDEQQELVERDDEKQLMNVEPIHADILLETYKRKIADEGRLFLAEFQSIPRVFSKFPIKEARKPFNQNKNRYVDILPYDYNRVELSEINGDAGSNYINASYIDGFKEPRKYIAAQGPRDETVDDFWRMIWEQKATVIVMVTRCEEGNRNKCAEYWPSMEEGTRAFGDVVVKINQHKRCPDYIIQKLNIVNKKEKATGREVTHIQFTSWPDHGVPEDPHLLLKLRRRVNAFSNFFSGPIVVHCSAGVGRTGTYIGIDAMLEGLEAENKVDVYGYVVKLRRQRCLMVQVEAQYILIHQALVEYNQFGETEVNLSELHPYLHNMKKRDPPSEPSPLEAEFQRLPSYRSWRTQHIGNQEENKSKNRNSNVIPYDYNRVPLKHELEMSKESEHDSDESSDDDSDSEEPSKYINASFIMSYWKPEVMIAAQGPLKETIGDFWQMIFQRKVKVIVMLTELKHGDQEICAQYWGEGKQTYGDIEVDLKDTDKSSTYTLRVFELRHSKRKDSRTVYQYQYTNWSVEQLPAEPKELISMIQVVKQKLPQKNSSEGNKHHKSTPLLIHCRDGSQQTGIFCALLNLLESAETEEVVDIFQVVKALRKARPGMVSTFEQYQFLYDVIASTYPAQNGQVKKNNHQEDKIEFDNEVDKVKQDANCVNPLGAPEKLPEAKEQAEGSEPTSGTEGPEHSVNGPASPALNQGS

SEQ ID NO: 8 - protein, 1193 aa, Homo sapiens
  CD45RC
MTMYLWLKLLAFGFAFLDTEVFVTGQSPTPSPTDVPGERSTASTFPTDPVSPLTTTLSLAHHSSAALPARTSNTTITANTSDAYLNASETTTLSPSGSAVISTTTIATTPSKPTCDEKYANITVDYLYNKETKLFTAKLNVNENVECGNNTCTNNEVHNLTECKNASVSISHNSCTAPDKTLILDVPPGVEKFQLHDCTQVEKADTTICLKWKNIETFTCDTQNITYRFQCGNMIFDNKEIKLENLEPEHEYKCDSEILYNNHKFTNASKIIKTDFGSPGEPQIIFCRSEAAHQGVITWNPPQRSFHNFTLCYIKETEKDCLNLDKNLIKYDLQNLKPYTKYVLSLHAYIIAKVQRNGSAAMCHFTTKSAPPSQVWNMTVSMTSDNSMHVKCRPPRDRNGPHERYHLEVEAGNTLVRNESHKNCDFRVKDLQYSTDYTFKAYFHNGDYPGEPFILHHSTSYNSKALIAFLAFLIIVTSIALLVVLYKIYDLHKKRSCNLDEQQELVERDDEKQLMNVEPIHADILLETYKRKIADEGRLFLAEFQSIPRVFSKFPIKEARKPFNQNKNRYVDILPYDYNRVELSEINGDAGSNYINASYIDGFKEPRKYIAAQGPRDETVDDFWRMIWEQKATVIVMVTRCEEGNRNKCAEYWPSMEEGTRAFGDVVVKINQHKRCPDYIIQKLNIVNKKEKATGREVTHIQFTSWPDHGVPEDPHLLLKLRRRVNAFSNFFSGPIVVHCSAGVGRTGTYIGIDAMLEGLEAENKVDVYGYVVKLRRQRCLMVQVEAQYILIHQALVEYNQFGETEVNLSELHPYLHNMKKRDPPSEPSPLEAEFQRLPSYRSWRTQHIGNQEENKSKNRNSNVIPYDYNRVPLKHELEMSKESEHDSDESSDDDSDSEEPSKYINASFIMSYWKPEVMIAAQGPLKETIGDFWQMIFQRKVKVIVMLTELKHGDQEICAQYWGEGKQTYGDIEVDLKDTDKSSTYTLRVFELRHSKRKDSRTVYQYQYTNWSVEQLPAEPKELISMIQVVKQKLPQKNSSEGNKHHKSTPLLIHCRDGSQQTGIFCALLNLLESAETEEVVDIFQVVKALRKARPGMVSTFEQYQFLYDVIASTYPAQNGQVKKNNHQEDKIEFDNEVDKVKQDANCVNPLGAPEKLPEAKEQAEGSEPTSGTEGPEHSVNGPASPALNQGS

SEQ ID NO: 9 - DNA, 8468 bp, Homo sapiens
  vector pRSF91_CD45-CD28c-T-CAR _iB_prePuroR
cgggcctcttcgctattacgccagctggcgaaagggggatgtgctgcaaggcgattaagttgggtaacgccagggttttcccagtcacgacgttgtaaaacgacggccagtgaattagtactctagcttaagaatgtagtcttatgcaatactcttgtagtcttgcaacatggtaacgatgagttagcaacatgccttacaaggagagaaaaagcaccgtgcatgccgattggtggaagtaaggtggtacgatcgtgccttattaggaaggcaacagacgggtctgacatggattggacgaaccactgaattgccgcattgcagagatattgtatttaagtgcctagctcgatacaataaacgcgccagtcctccgattgactgcgtcgcccgggtacccgtattcccaataaagcctcttgctgtttgcatccgaatcgtggactcgctgatccttgggagggtctcctcagattgattgactgcccacctcgggggtctttcatttggaggttccaccgagatttggagacccctgcccagggaccaccgacccccccgccgggaggtaagctggccagcggtcgtttcgtgtctgtctctgtctttgggcgtgtttgtgccggcatctagtgtttgcgcctgcgtctgtactagttggctaactagatctgtatctggcggtcccgcggaagaactgacgagttcgtattcccggccgcagcccctgggagacgtcccagcggcctcgggggcccgttttgtggcccattctgtatcagttaacctacccgagtcggactttttggagctccgccactgtccgaggggtacgtggctttgttgggggacgagagacagagacacttcccgcccccgtctgaatttttgctttcggttttacgccgaaaccgcgccgcgcgtcttgtctgctgcagcatcgttctgtgttgtctctgtctgactgtgtttctgtatttgtctgaaaattagctcgacaaagttaagtaatagtccctctctccaagctcacttacaggcggccagcgctcgtctagcaggatccgccaacatggggtggagctgtattatcttgttccttgtagccacagcgacaggggcccattccatggaagtgaagctgctggaatctggcggcggactggttcaacctggcggatctctgaagctgagctgtgccgccagcggcttcgacttcagcagatactggatgagctgggtccgacaggcccctggcaaaggactggaatggatcggcgagatcaaccccaccagcagcaccatcaacttcacccctagcctgaaggacaaggtgttcatcagccgggacaacgccaagaacaccctgtacctgcagatgagcaaagtgcggagcgaggacacagccctgtactactgtgccagaggcaactactacagatacggcgacgctatggactactggggccagggaacaagcgtgaccgtgtctaagatttctggcggaggcggatcaggcggcggaggaagcggtggcggaggatcaggtggtggtggatcaggcggaggtggcagctctgatatcgtgctgacacagtctccagccagcctggccgtttctctgggacagagagccaccatcagctgcagagccagcaagagcgtgtccacaagcggctacagctacctgcactggtatcagcagaagcccggccagcctcctaagctgctgatctacctggccagcaacctggaaagcggagtgcctgccagattttctggcagcggctctggcaccgacttcaccctgaatatccatcctgtggaagaagaggacgccgccacctactactgccagcacagtagagagctgcccttcacattcggcagcggcaccaagctggaaatcaaagcggccgcaggcaaacacctgtgtccttctccactgttccccggacctagcaagcctgtcgacttctgggtccttgtggttgtaggtggagtcctggcctgttattctcttctggtcactgttgcatttatcattttttgggtgcgcagtaaaaggagccgcggagggcacagcgattacatgaatatgacgccgcgcaggcctggacccacaaggaagcattaccagccatatgcgcccccccgggacttcgcagcctaccggagcaaaagaggtaggaagaagcttctgtatatttttaagcaaccgtttatgcggcccgtccaaacaacacaagaggaagacgggtgttcctgccgctttccggaggaagaagaaggcggctgcgagctgcgcgtgaagttttctcgctccgcagacgcgccagcgtatcagcagggacagaaccaactgtataatgaacttaatctcggccgacgagaggagtacgacgtgcttgataagaggcggggtagagacccggaaatgggcggaaagcctcagcggcgaaagaatcctcaagagggcctttacaatgagttgcaaaaagacaagatggctgaagcctactcagaaataggtatgaagggggaaagacgccggggtaaaggccatgatggtctgtaccagggactctccacggctacgaaagatacttatgatgcacttcacatgcaggccttgccgcctcggtgataatctagatacgtaaattccgccccccccccccctctccctcccccccccctaacgttactggccgaagccgcttggaataaggccggtgtgcgtttgtctatatgttattttccaccatattgccgtcttttggcaatgtgagggcccggaaacctggccctgtcttcttgacgagcattcctaggggtctttcccctctcgccaaaggaatgcaaggtctgttgaatgtcgtgaaggaagcagttcctctggaagcttcttgaagacaaacaacgtctgtagcgaccctttgcaggcagcggaaccccccacctggcgacaggtgcctctgcggccaaaagccacgtgtataagatacacctgcaaaggcggcacaaccccagtgccacgttgtgagttggatagttgtggaaagagtcaaatggctctcctcaagcgtattcaacaaggggctgaaggatgcccagaaggtaccccattgtatgggatctgatctggggcctcggtgcacatgctttacatgtgtttagtcgaggttaaaaaaacgtctaggccccccgaaccacggggacgtggttttcctttgaaaaacacgatgataatatggccacaaccatgagcgagctgattaaggagaacatgcacatgaagctctacatggagggcaccgtggacaaccatcacttcaagtgcacatccgagggcgaaggcaagccctacgagggcacccagaccatgagaatcaaggtggtcgagggcggccctctccccttcgccttcgacatcctggctactagcttcctctacggcagcaagaccttcatcaaccacacccagggcatccccgacttcttcaagcagtccttccctgagggcttcacatgggagagagtcaccacatacgaagacgggggcgtgctgaccgctacccaggacaccagcctccaggacggctgcctcatctacaacgtcaagatcagaggggtgaacttcacatccaacggccctgtgatgcagaagaaaacactcggctgggaggccttcaccgagacgctgtaccccgctgacggcggcctggaaggcagaaacgacatggccctgaagctcgtgggcgggagccatctgatcgcaaacatcaagaccacatatagatccaagaaacccgctaagaacctcaagatgcctggcgtctactatgtggactacagactggaaagaatcaaggaggccaacaacgagacctacgtcgagcagcacgaggtggcagtggccagatactgcgacctccctagcaaactggggcacaagctgtacaagggcagcggcgccaccaacttcagcctgctgaagcaggccggcgacgtggaggagaaccccggaccggtgaccgagtacaagcccaccgtgcggctggctaccagggacgacgtgcccagagccgtgagaaccctggccgctgccttcgccgactaccccgccacccggcacaccgtggaccccgaccggcacatcgagagagtgaccgagctgcaggaactgttcctgaccagagtgggcctggacatcggcaaagtgtgggtggccgacgacggagccgccgtggccgtgtggaccacccccgagagcgtggaggccggagccgtgttcgccgagatcggccccagaatggccgagctgtccggcagcagactggccgcccagcagcagatggaagggctgctggccccccaccggcccaaagagcccgcctggttcctggctaccgtgggcgtgagccccgaccaccagggcaagggcctgggcagcgccgtggtgctgcccggcgtggaagccgccgagagggccggagtgcccgccttcctggaaaccagcgcccccagaaacctgcccttctacgagcggctgggcttcaccgtgaccgccgacgtggaggtgcccgagggccccagaacctggtgcatgacccggaagcctggcgcctgatgtacaagtaagatcccccgggctgcaggaattcgagcatcttaccgccatttatacccatatttgttctgtttttcttgatttgggtatacatttaaatgttaataaaacaaaatggtggggcaatcatttacatttttagggatatgtaattactagttcaggtgtattgccacaagacaaacatgttaagaaactttcccgttatttacgctctgttcctgttaatcaacctctggattacaaaatttgtgaaagattgactgatattcttaactatgttgctccttttacgctgtgtggatatgctgctttaatgcctctgtatcatgctattgcttcccgtacggctttcgttttctcctccttgtataaatcctggttgctgtctctttatgaggagttgtggcccgttgtccgtcaacgtggcgtggtgtgctctgtgtttgctgacgcaacccccactggctggggcattgccaccacctgtcaactcctttctgggactttcgctttccccctcccgatcgccacggcagaactcatcgccgcctgccttgcccgctgctggacaggggctaggttgctgggcactgataattccgtggtgttgtcggggaagctgacgtcctttcgaattcgatatcaagcttcctaacacgagccatagatagaataaaagattttatttagtctccagaaaaaggggggaatgaaagaccccacctgtaggtttggcaagctagctgcagtaacgccattttgcaaggcatggaaaaataccaaaccaagaatagagaagttcagatcaagggcgggtacatgaaaatagctaacgttgggccaaacaggatatctgcggtgagcagtttcggccccggcccggggccaagaacagatggtcaccgcagtttcggccccggcccgaggccaagaacagatggtccccagatatggcccaaccctcagcagtttcttaagacccatcagatgtttccaggctcccccaaggacctgaaatgaccctgcgccttatttgaattaaccaatcagcctgcttctcgcttctgttcgcgcgcttctgcttcccgagctctataaaagagctcacaacccctcactcggcgcgccagtcctccgacagactgagtcgcccgggtacccgtgttctcaataaaccctcttgcagttgcatccgactcgtggtctcgctgttccttgggagggtctcctctgagtgattgactgcccacctcgggggtctttcattctcgagagctttggcgtaatcatggtcatagctgtttcctgtgtgaaattgttatccgctcacaattccacacaacatacgagccggaagcataaagtgtaaagcctggggtgcctaatgagtgagctaactcacattaattgcgttgcgctcactgcccgctttccagtcgggaaacctgtcgtgccagctgcattaatgaatcggccaacgcgcggggagaggcggtttgcgtattgggcgctcttccgcttcctcgctcactgactcgctgcgctcggtcgttcggctgcggcgagcggtatcagctcactcaaaggcggtaatacggttatccacagaatcaggggataacgcaggaaagaacatgtgagcaaaaggccagcaaaaggccaggaaccgtaaaaaggccgcgttgctggcgtttttccataggctccgcccccctgacgagcatcacaaaaatcgacgctcaagtcagaggtggcgaaacccgacaggactataaagataccaggcgtttccccctggaagctccctcgtgcgctctcctgttccgaccctgccgcttaccggatacctgtccgcctttctcccttcgggaagcgtggcgctttctcaatgctcacgctgtaggtatctcagttcggtgtaggtcgttcgctccaagctgggctgtgtgcacgaaccccccgttcagcccgaccgctgcgccttatccggtaactatcgtcttgagtccaacccggtaagacacgacttatcgccactggcagcagccactggtaacaggattagcagagcgaggtatgtaggcggtgctacagagttcttgaagtggtggcctaactacggctacactagaaggacagtatttggtatctgcgctctgctgaagccagttaccttcggaaaaagagttggtagctcttgatccggcaaacaaaccaccgctggtagcggtggtttttttgtttgcaagcagcagattacgcgcagaaaaaaaggatctcaagaagatcctttgatcttttctacggggtctgacgctcagtggaacgaaaactcacgttaagggattttggtcatgagattatcaaaaaggatcttcacctagatccttttaaattaaaaatgaagttttaaatcaatctaaagtatatatgagtaaacttggtctgacagttaccaatgcttaatcagtgaggcacctatctcagcgatctgtctatttcgttcatccatagttgcctgactccccgtcgtgtagataactacgatacgggagggcttaccatctggccccagtgctgcaatgataccgcgagacccacgctcaccggctccagatttatcagcaataaaccagccagccggaagggccgagcgcagaagtggtcctgcaactttatccgcctccatccagtctattaattgttgccgggaagctagagtaagtagttcgccagttaatagtttgcgcaacgttgttgccattgctgctggcatcgtggtgtcacgctcgtcgtttggtatggcttcattcagctccggttcccaacgatcaaggcgagttacatgatcccccatgttgtgcaaaaaagcggttagctccttcggtcctccgatcgttgtcagaagtaagttggccgcagtgttatcactcatggttatggcagcactgcataattctcttactgtcatgccatccgtaagatgcttttctgtgactggtgagtactcaaccaagtcattctgagaatagtgtatgcggcgaccgagttgctcttgcccggcgtcaatacgggataataccgcgccacatagcagaactttaaaagtgctcatcattggaaaacgttcttcggggcgaaaactctcaaggatcttaccgctgttgagatccagttcgatgtaacccactcgtgcacccaactgatcttcagcatcttttactttcaccagcgtttctgggtgagcaaaaacaggaaggcaaaatgccgcaaaaaagggaataagggcgacacggaaatgttgaatactcatactcttcctttttcaatattattgaagcatttatcagggttattgtctcatgagcggatacatatttgaatgtatttagaaaaataaacaaataggggttccgcgcacatttccccgaaaagtgccacctgacgtctaagaaaccattattatcatgacattaacctataaaaataggcgtatcacgaggccctttcgtcttcaagctgcctcgcgcgtttcggtgatgacggtgaaaacctctgacacatgcagctcccggagacggtcacagcttgtctgtaagcggatgccgggagcagacaagcccgtcagggcgcgtcagcgggtgttggcgggtgtcggggcgcagccatgacccagtcacgtagcgatagttactatgcggcatcagagcagattgtactgagagtgcaccatatgcggtgtgaaataccgcacagatgcgtaaggagaaaataccgcatcaggcgccattcgccattcaggctgcgcaactgttgggaagggcgatcggtg

SEQ ID NO: 10 - DNA, 783 bp, Homo sapiens
  scFv anti-CD45, codon-optimized
atggaagtgaagctgctggaatctggcggcggactggttcaacctggcggatctctgaagctgagctgtgccgccagcggcttcgacttcagcagatactggatgagctgggtccgacaggcccctggcaaaggactggaatggatcggcgagatcaaccccaccagcagcaccatcaacttcacccctagcctgaaggacaaggtgttcatcagccgggacaacgccaagaacaccctgtacctgcagatgagcaaagtgcggagcgaggacacagccctgtactactgtgccagaggcaactactacagatacggcgacgctatggactactggggccagggaacaagcgtgaccgtgtctaagatttctggcggaggcggatcaggcggcggaggaagcggtggcggaggatcaggtggtggtggatcaggcggaggtggcagctctgatatcgtgctgacacagtctccagccagcctggccgtttctctgggacagagagccaccatcagctgcagagccagcaagagcgtgtccacaagcggctacagctacctgcactggtatcagcagaagcccggccagcctcctaagctgctgatctacctggccagcaacctggaaagcggagtgcctgccagattttctggcagcggctctggcaccgacttcaccctgaatatccatcctgtggaagaagaggacgccgccacctactactgccagcacagtagagagctgcccttcacattcggcagcggcaccaagctggaaatcaaa

SEQ ID NO: 11 - DNA, 118452 bp, Homo sapiens
agtaaaaccgaatctgacatcatcacctagcagttcatgcagctagcaagtggtttgttcttagggtaacagaggaggaaattgttcctcgtctgataagacaacagtggagagtatgcatttatttatttacttttacatttttgattcgtttttacagagaaaaacttctacagagataacaattattttgcttttcagaaggacgcatgctgtttcttagggacacggctgacttccagatatgaccatgtatttgtggcttaaactcttggcatttggctttgcctttctggacacagaagtatttgtgacaggtaagtacaaggatattaatattttttaaattattttttctcttttggaggaatgtttgaaatagacataaaaataatttaaatgtgttggtaactggaagtgagaagcctgctgtaaaccatcaagattgttgtctcagggagacatagctagttgtgtgacagaatacattgtttctgtttacaaagacataaatgtttcgggacaaaaaatacaattttaaaaggaaagcaatgtctatctgtatctttatttacaactgttcaaagatattacaaaagcaacattattacttaacttccaaagtgacaataacacacatttataaaagcctgagaattttttaatgataaaataagtgagtttttattcttttaacaaatttgatcttttaaaaagtcataaaacagctttggttgtatgtaagccactccctcttttcagacctgaagtttgcttcctcaaattttgaatttaattgacatattttattgaatacttgggtatataatagttcaaaaatatattgagatatttagtaaaatattaactttctgcaatttttatcacagaatgtattttaaatcaagtttttagtttcttgttaatagttttaatacatttttgctttagaaattcttgtggagccaccgcccttcctgggtggtgggtaaatattacagccttgatgagatagaaatatttaaactcttaaaaatcatgcaaatgctgtattcagtaggaaaatgcaactagttggacttccagtgcctattaaagtttgaaatctttgcacatttatggtctattcaatggatagttcttgagcggcgtcaatatgaatcatgagtacatttcaatagattatagaatgtaactaataattaatatttaatatttctctttatgatgtagtatctaaaaggacattgaaaataaaatttttgtagaaattccaaaaagtataaaaagtattttaaaacaacttgcttattacaattcactttgaagtctttttttgacttttaccgttcttctttcctctgaaagtcagggaagtagctacctcttgagcatgttacattgacaatttctatttggagaggaaagaaagaggaaagaaaaacaacataagatttttgttgttgttgttgtggctgttttgctttttattgcaaaggtgaattttttaaaaatctatatatttgcagcatttgtcttagtacagaaaatgtttatcaagttaccatccctttaaagcttatgataataaaaagtaaattataaagaataataatctcaatgaagtgatatatgtatattatcacaaatcagaacagattttcatttaaaattcccactcaggaaatgtcgaaaagcatttttaaatgagcataaagaaatactgagacattttgtaagccagaatatttttcttctcttcatattcatttaacttctattattttcttcaggtctagctccattgctttttattccaggcaaacttcccaacctcctgaatagaccaaatatcctattatatgcttaaatcagagtgtgaaatatttcctttgtgaataaaaattcaactcattctattacaggatgtttttttaaccataagacacatctttgaatttataattgaaataatatgatggggtctagaaacctttatatcaactttgctgaatgatttataccatagcaaataaatggatatacataaatttattttgaaaactcaactttatcttcagttgctcacataaatattgagagcaaacatttttctaaaagacatttgtagactccctgagatatatgcttatttgtggaaaaacatatacagatataatcatttgtatctgcaaatattgtttataatcctttcaagttgcaagaaacattttgtgatttaatgtataatttggaaaattcttaatgctttaaattatttatttttcttttttagcaacaaatgagttggattctatgtttcattttaacgtgttaaaattagtttagtgcctacaggaaataataaacttttggggaacaaaatttatattgtatgctgtaaaggcataaagaaatagagccaaatgtagagagccatcaatggtaactctatgcataattcaaatattttatttaatatctaaaatgcacacacggacaaggccaaagttaatctttgccacggcaacaaccaggcagggttcagttttactcaagacttcctaatcctcttgctctgtgcctctttgccatggcaactggaagccaaactttgtttagaatttctaaataatgttaggggacaatgatggttttaagaaggcaggtgaaggtgagtgttctctggttctaataaagttgtaatgccaggcagatctaccacactatagcatggcagttaggagtatatgagttatggtatgtgaggtatatgatgagttttgttatgagtcataacagttaagactcatttcctggacataattcttcatttttccatctgtattaaaaatatatatctcatgttataaacatggactgtgccttgcacatcacagacattcaatgaaaattatttaattgaatttggtaagcagtcctattaagttctaaatactccataatttagagatttgggaatgtgattagaattacttattaatttgaaaaaaaatgtcctactaaaaacctgcctgtgacctttatcattgctaaagtttgaaatgtactttgttacaggaaagactacggctagggcctatattatctttttctcttttgttctgtgtaagtaagtataggggcagagtagttagcttgaacttagttctttctttgttctggactatttgctatcctctcaccagtgacaattaaccagtatagaaatatagatgtttctacattgttcatatacttgaacatatatttctttatgtagatactcacacataaactagttatatatttgtgggttatatatactagtcaatctatctatctgtctatctatctatctatctatctatctatcagttctccatgtttgtctatttggcgttcccatgaacttcagaccttcgcctgtgttctcttttctccatttggttacgtatcattgcctactatgtgttgatcactctgattctccatctctagactcatccctcagaaacacggaacttactacctttcctaaatccagacattaacatgctccccaagtcctgaaattttgctttgtaataatctctaataacttcttgctttgacacctccattgccatcatcttaattcatggctttattatttctcacctgtaaaattgtaatagtttttttaatcagtctgaagtctcatcctttttttaatgtaatctacagcttaaaaagtaaaataaaaagtgaagggttactgatttcttctcattgcctttggtataaattctaatcttttttgccagagaaactggttccactaatgatctgggggctaggcctggagctgggaagggatcttttttcttttctttctttcttcctttctttctttctttctttctttctttctttctttctttctttctttctttctttctttcttttttctttctttttcttctatgattgattaaaagaaaacaaacaggaggtagttttaacacccacctctatactttctcaaggtgtttaaggttctgggcaaatcctacttcttctattatgttctcttatgtcacttttgccacaaaatatttccattgaattgcacactttttatcaccttttcttggcatttttcaagtcatttcaatctgctcttttttgtgatgatgattgatgatgatgatgacatgtgaattagtggatttcttgacattgtaacctacatgaaatcaggtataggagacacaaaaggcataaactcatagttcccatacctaatttttcaccagacactgaataaatcatagattaaaaaaataaaactgcatattgtagtgacaaaggaaaggaaaattttcaaagagggaagtcaaaaagagggagaatatgagataaaaaaattaaccagaggcgaagtgggaggatgaagacagcaggactattttgtccagattaaattaagttgattttggatctagatgtttacagtcttgcctttttgtttttgtttgtttgtttgtttgttttttctttgctccctttcttactctccttatctcacctctcgtctggaaagagcctcctgacttcctaaaagttcatagtttgagaatgtttttcctaaattttctttgatctgctctttggacattctaggtaatgtaatttggagggtcaattttatttttcagatacacatacccataggagaaaaagcaaggaatgggagggaaatacaaatgtagcggagtgataacacaaacagatcaggtccagtcatggcaattgctggtttgaacactgatgctagtgctctgggattgcttgcaagggcagatggaatatggtgcaccctaggtgttgcattatttgcacgacaaaagtttgtagagagctgggaataatttctttacagacagtgtggtgatgaatgtcaatctgagtaggtaaggggcagagatttgtactgaggttgattcattctcttggtaaatacacaatgttcacaaaggcaaggtttcatcttcagaccatgtgtgtatatgtcaccttggtgcagagagagaaatttttcatcagtgctgacctttgatttttttttctagacatcttatagatttatgtagttatttacatgggaaacaattagaatggaaatttaacatatcttcagtttaaaattaatttctgtctagtctaaatatctttgtaagtactagatactcaatcccatagcagtggccttttaccaaaggcttagtgctatgacttttgcatacataaagacctcactttttaagatatgatacaccagaaaaaaaatatggcaagactttagcaatatgatttgatgcctatttctatataatacccaaatatacaggaataaaaattatggcaatcactggattttgtgtacctggctctaaccaatatttatattagaaaatatctaattattgtctaaaatatttaatcttcattcctgtttgtatgtcagtgtgctacttcaatatcagtctgttaaaagagtctaggaatgactactataagcagagaattatatgttcaggaatcacaacaaaaaacaagaacaaatagagaaacaaaagctttcctactctttcatctaggacaagaataaatacacataaagtcaatattagtgaagtaaacaagcatcttctatatccattcatagtaccttcaattgattgatttcttaacagacaatcagcaaaattatcagtttttattagagattttagtagagaccgagcttaaacaaatatattctatggtgcttaactctatagtatttaaagattcaatatttatttcctctaaaaatgagtcaagtgtctgaaaggaaaaagccacctaactgaaacttcagtttctactatacagggtatttattataaaactgtaattacaatgcaattatattgaagtataaatgatcatcattcatttatttaagaatataatcaaaatttgcatacctggaagaaaaccatccaccctccaaaatagggatttgctaatgtaggagtagaaggcaaaagttgagggtaactcaggtaacacactcatacgtattaggatatgaacagctggtatagcaaacttgatagaaatcactgatagacaagaagacattctctgcattttaaattaaagtacaatttgtctgtggtcattcaagagatagtttagagaaacctatacaaataacaatgatgctaagagacaatatcaaaatcacaataaatatcatggcaatacagtgtggccactatattttaaacacatccacttgatgaaaaatataataatttactgataaaacatattaagcataatagaaaatgaggcagaaaccactccaagctgggaaacatcatgacatctgtagtgataaatattttgaaaatctaactctatgaatcttgtgatttttagctaaatcaattttcacccttgagacccaatttcctcatctataaagtgttgtaagcattaaaagttataatatttgtgaaaatgctttgaaattatgtgatactctgagaagtaaattttttcatgtgagcccatgaaatcagagcacatagccttttagcataaacttgattccaaatgatatctcttcctttcagacactgtgagcagataaagggatagtttaaggttaagtgatagaggcataatcccttataggcctttgaattcttttaactttgcattctttatttcagagatttttcaggcttctccagattctacagtctaaatagtttgtaaatccacacacttctactttgccagggatttcttagtgtaaaaatatcctgaagtctcacctgccttcaatccttactgtgtccatacccaccattaccaggataatctttgtaaaaggcagaacttacctttgtccattcctcttttaaaagctcctattggtagaaaatatactgaacccgtgatttgataccaagtatgttttggctcaacttttatgaaaacaaatatttaattagaatataccaacatttatgagttttccttaaagataaattttggaggaaaaaaactccattagaccaatttaattccctgatgattatatatatattacctagtgaaatccttggcagtttttccattttaattttaattttactgaactaatgtttagcagcatcactttcatttaatttttacaataactattagattcatgaatccattttacccatgtcaagttctactgaatatagcttatgcttggaattttcctttgtgattattacttttctaaaggtaattcttcttttcaaacaatacagatctaaattttccaaaaccatttaaattcttctctttggccagaaacattttctgtgtgtagttttggctaccgctagtttagtttttttaattggttttgtgtctcaatgctacaaaaaatataatttatgtaatttttcatttttgtcaaacttaaatcgggcaatattaaccattctcaattttttgttgtgttgaaatttctatcagtgacattaatgtggagattgacagctctttgagctagattcattttgaaattttaagactttcgattatttcttatctagccaatagaaactttagaaacacttttaagactgcttgatagcctggaattattatgtttgaattctcattcatttgtatggtattcctcttattagctttcacacttagtaccaatttcttattcattattggagcaaaaagtaaagagaagaatcaaggtgataagtttaaaatcttctcaatgtaaaatagtgtgtggggaaagtgtcaaatcatcctactttggtctttgtgcatttaggaaaaataaaagcaattagcattgcacacacatatgtaattgaatctcttcagatttgtctggctttatctctaaccactttgtgactctttttgtaacttgcatttttctaaaaatgtgaccttgtttggtcttcctactgttggccatgctgtttttccttctctccacatctttttatcaatggtgcaaattataaattgtattcaaatttactgtaaagatcatgtcctctagacagcccctatcccacttgtataacccttgctcttcagcccctttcacacctgcataggtattcttctgctgtgatgatcctttgaataattctcttggagttctctttaccaggctctcttgcagcaactggtgagctcatgtaggctatcactgggtctctgcttatttgccagtgcctgcaggtcctcagtacctgtttgctgaacaaacgaatggtctgtcagcttaacccaactctgtatgtagaaggcacttaataattcttaaaaacaattttgattctgtccttttattgttatttatgggaattatttatggtaaaaatttctacataatagaaaatttggaaaatgtcaagaaatagaaggaaaaagaaattgcttagagcccatgctaacattttgtttttcttcctctatcttttgatcacatgctgtgtatgaaatttcatgttcaattttttcccaagtaaaccttgattattctagacaatttgaaaaatatagaaatgaatagaaaaataagaatttcaggtttccagttctcaggatctaaaaactttttgagtatttcatttgactaggacaactagatctattcagttatttattaacttattagttcatttgataaacaactattttgtgagtgttttccatgtaatttgggctgaggacacctatcccatgaagcccgtattttctatcagtggcttcttggagatggtgttttaaatcttccaaaatcttcatcagcaccccaaaacttcctcctcaaagtaacaacataccttgctacagataattattggtgttatcaatgttttataaattataaatttaaaaatcactatcttaagatctatatataacatattaagtaaaacttatattcttacaagacttcctccaggtccctgttacaaccagattttctttgcagacttttaaattatggaagttctggtgctgccactgagttgtgtagattattattagatattcaataaataaagttggtagatgtgaagaggtactagacaatagtcctattttgttttggtttgtttgttttgtaatttattctgaaaaaatgtttatgtggagagaaaagggaaaacatacagaaatacacagcacacaaacaaattcttacttttttttggtagtctttctaattttccaaggtcaccagctaatagcaaatgagagttgtagggggtggggtgaaggctggggtcttaatcggggtctatctgattctagatagaccagattctagattttccactcggttactcaatcttcttagtggtcagtttaataacctggaatttaagacatgactgtgtgatgatgggcaaatcacagcaggactgaatgggagctggtaatttctcagaggttgtttgtgtgacatatgcatgtaagttcattcacctgatttagctacttacatgaaccattgtgcactgagctgcttctatatctttagcatattctgtatctatgtaaaattcacataagattgtatgacttttataaaaaacaaaaagacatctttgattaatttgtcttcactatgaatactgatgtgatgtgttacaatcatcctgaaaaggaggctaacaaaggacaggactgagtctgtcttgaggtgagtgatatgatggaaagaatggattttcccccacccaactcatttttgatattacataaagtgaaaaacattaaataattcaccaaagtatctagatttttttttgtttttgaagtgcaagggaagtaacttgacctttgttaaacactttgatcatggaaaacacataaggttctcatcttattccaggaagtgtagacactagataatcttttcatagtcatccaaaaagcatattaagtgaaccaggtaaatccatcctacactttttattccagagacaagttggctaaactttgaggagactaaaacaaaacaaaaaaaaattattgtttggttcatttgataaatgtggattccaatcatataatttaggccaaatattatactttgacttcttagacttagatttccagatagtctggtttataaaataagattttaactatgcttactaaactctatgtatttctactttccaatgacccatgttcttattttctgaatttacttattgatgctttaggtatgataaaggtatgtaatggctaaggaaacataaatgaagcataagacatcagttgagagttttgacggaaaggaagtggtgatatgaaggaaacagataaaccaaagaaaaaggaaaaggtcagggagctgataaaagtaacttgaagaaactttagtgcaaatgttggattcagacaatcgctacttttaaagtacttaaagaagtcagtctttgaaatcttgcccggattccattccagtttcatcattggagacttccaatgatgaaaaattggggaagaattaccttccaaagcctcagtttcctcgtgtgtaaaatggaaataatagcaagagatattaaatgagatgattcactcatcgattcatcaattgtttatagagcccctgctaagctaaaaactgttttaagtgttgacacagtggtaaagaaagcagaaagtgtaactacttttatgaaactgacttcctagtggtgagagataacaagaaaacaaacaacaaattgagataacttcagttatagataaatgctgtgaagaaaattaagtagtgtaatatggtagagtttaatctggccagacccagatttaggggtgaatgcacttttagacagagtgatcggggaagatccttatgaagaagaatcattgagctacctgttggctgacaagaatatggggatccatgtgagggagactggcaagagtaaaggttatctggcaaaaccaaacaaattggtaggttcgaggcacagaaaggtcaggcatctgtagtatggtgagtaagaactgagcaggttgtggtgaggctagaaagataagcagaaggcaggtcccacagggccttgatggaaatggaaagagcttgaattttacctgaagtataaagggaaggaaccattttaagttcttaagtacagaataacctaatcttctttctgtgttgaagagatcactttgactgttatgaagagaatagattggaagtaaggcaaagcctggaagcagttatgaggagactgaatgggaggatggagaaaggggatggtgatctggaccaagtgttggcagtgcaggtggaaagaaaggaaagactgacatagaattaagagaagtggctgcatggaaaagacaaagacattttagagaatgactttttttccccatgagcactgggatgggaaagagccaaattagggggtcagaaatccagagttatgtttgggctgttattgatgtctgattttcattaggtggtagagaggtcaagaaatccgttggagataagaggctgaggcccattcagtaggtctcaactggagacataaacataggagtcattgcattcagatggagcttaaagctaagggactgcatgtgacagtgtaaataaacatgtagagagtagcagatgactggtttctgagccttgggaaacttcatatttggaagagacacaaggaggagctaggaaaagatagtgagaagaggtagccagtgaaaaaaagtagaactatactttgctttgaatgttgaaaagggttggcattatagtgagaattcagtaaattccacataaaaatctgaatttatgtctcccctagaaaggttggttgtgaacatgcaattggtaaatatctctattaactttaatattgttacaaaagtaatattaaggaatttataatatttggaagaattagatgtctttacctaatatatcccttgctagcttaacaattagaaaaagaaagaggtacatcttaacataatttgttttaataaaaactacagaatatattgagagactaaagaattagaaatttaactgaaaatttcatgcaaaggtaatgctctgttgaaccattttgtagcttatgttttgttttgatacatattttaaaatattgtttaagacaatacttgaacagattgggattgtgtgtgtgtgtgtgtgtgtgtgtgtgtgtattggttaaataactggtttatttttaaactgaaattaaaccttccatttctttgagaaatttaaaaagtagttgttatcaatgtggcagatattaggtagaatctaatatcgtgaaaattaaactgcacataaatagatataaatccttttgtcagtgtgtgtatatctctgtgtgtaattttgatctcaggcttggcaggtttccttaaaacttttttttagagctacttaattttgtacttactggtggttagctaataagaaaaagctaataaaaaatagtgcttactctgtgccaggcacttctgttaacattttataaatgttatctcatttaacaagctcatgtcattgtatagtctagcttatacttgtctttaacataagcaaatttgttaatttgtgtttcctgatattatcataaaatttactggttgtcatatcctaaaagggaatagttcaatttaattttccttgttctaattttaaatacagtactaaggttgagaaagaaggggtcaggaaagggaagtaacattgagtgtctcgtgtgcctggcactccatatgatgcttcaatgcacaccaggctattcagcctcagatttgtttctacattgcttctagttctacagattattcaacgaatgtacaatccttggtcactagtcttaatagggaaaacagaattatggttaaaacaaaagagtaagtaacttaaatatgatctatcggtatttattttgtattatgatattttgcttaagttgaaaaaagggcgcatcaggtgttttggcagtttactgtgatctcaatagtgagaatgtattgaaaaatctcagtacaggagaaagctgtgcagctttctcttcctgtcgctgcttaattttcatgtagatataaagccgcagtttaagcacatctgcttaatccttatttaaaagactaggagagaactagaaagggagggagggagaggaggggaagggggaagagattgagagaaatctctcccatataacacaaacactgtattagtgtgtgagaagcagataatcgtgcatgtaggcactatcatttgtgaaatcagaaagcataatttactcccaatgctgaataatctagttgtgtgtaagcaccagagagatatttaaatacctatccaataaaagataataaaagcctagcaaacctaagtaatccattttcagatgttaatccaattacgtaaacaaatattacccttttttttttttggtcattgtttcaaggataaagtgtaaatgaaagaaatagcattccatctaggtaaaagaggaatcagcatcattgaaatgtgaatagctgtgattcctccttgctgaatggtaactttagaagagagggaacccaggagtccatccagaggctcaaggaataagaggttctcacccataggaagatgaaaaatactttcagggtgacccatgagggaaaatcaccaaagcctttgaaataaaagattttcccttttctaagaataaaagatggtgttatgtcaagggcggctcgatggtgtggatgaaagaactattgggaatggctactgaaagatcaaaggcaagtggaacctcaaaattctggaagtagaacgagtcagatacaatataagaagtacttcaaaggcaagaaaataagaataataaaaatacctttagttgtcaaatgtaaaatttgtgccagttttgtcacattccatttttcaggaacactgtaaaggtattttctattaatatcaatttaactgtacatatcttcccatctatcttaattagtcacttttcaagaacaaatgtgttatgctcaaagcatccaaaggacttttttgttagccttaataaaatgctttctcttaaactaaattttaatttagtttacatgtctacgtataaggtggttatagaaaatgaatgtaaaatcacttcattaagtgtaacaaaacaaaataatatgaggaattgttatactgtttaagcatttgaaaaacgataaaggagtatagaaattttgttaccactactatgattagtttctcatttggtttttcactttaagaattggaataaaagttgaaatcttgattaaaaaaacaagaaatgattcacaaattattttacaaattgaaatactgaaatacagaatgttcaaccactgtcaacatgaactcctattctgtaattaatctattctataaacatctgtatttgctaaagagcaacagatcaaggaaaagaaaaaataatccttgccatccatagagccatgatttttgtggaatcttcgctccagtttaagttttgtcagtgtctggaagaaaatacttcccatggatcatctttttgctaaagagtattctttacattttaaaacatatgaatatttacataaaggtgtttgtggaaaaggaaattatgtgccttttattttaattcacccattattctattccacatgtaaagtagaaaatactactttaagacaaaagtaaagcattatttatttaaagatctattttgtccatgaattttatcagaggtaacgcttcttaatgttattcagtgccataacttgccttttttctaggcctccattttatgaactgaacatctggatttgatggcaagaaaacatttccttccgctggcttttctaataactccctcttacagatatgcatgcctcatgtttgttaataaaattgacgtgattttaatatctggtattttaacacactgtgaattatggaattttcagtggctttatttaattaaatgcattttaaaatccttacaaaaaaatattaagagtaactctaaaatgtattagagccacagatgttttcctttatagtgttaattgatttaaggtccatcaaaatgctgttaaaatgtctagaggttaacaataacagtggcacatgggtcagattaaaattctttttgagtaaaataaataaataaatgacagcttattttcttctgatttaaaaaaattagctagtggattgaaacaacaatgtgatagctaagatttcattctctcactttataatgaaaggagatttaaaattagggattatatggtacacgaaaaatttatatacacagattacaagtactagtttttttagtgaagaaaagacaactatatattttctctttttatctgttgtcctattttacaattgtagcaattaatctgccaaactctttaatcaataaaatatggtatttaacaaccaaatttggcccctccctccccttaaatatatttccaatgctccttgctccattttaaacctgctgtcctttataagagaataatatattttgtaatttgagaaaatcatgcaaaggaaagtttctcaaaattcacattaatatgtaataatagtaataaatatgtataaccataatatcttagaattttacaatattttatagaaaacatgaatattaaagtgaaaatttaaacacatcaatttttcatgttaaaattactaagaatgaactacagattcatgaatactaagggcaacttttatctcaggaaatatatcagtggactgaaaatgtcaaatcaattcaattaaatcagtaataacactttgctgtttatgtggctgttttttcttctatttttattgtcttagattgcatggatacaatcaaaataagttaatttgtatacaggatataaatggaccagagaatgtgtcttctattaaataataacaaataagaataccttttattttgtgatggtctttactatttactgagagacaagtattgttcaagttgccggttttttttaattagctgacatatttcctgcttttatttgagttagaattcctgtaccaaacattttaaaaagagaaaaaaaattaaagaaagagaaaaggaatttggaaactactataatgtaaagtagcattatttatacaacaattaattttagagaagcaagagaccttagaaataatctatttcaacgcatctattttacaaaaaagaaaattgaaactcatagatatttagtgacttgtcctttgttacaccaaaaatgagggaacttggtctagaattcctccagcatattatgaggtatttgttctgtggcctgatacaatgaaatgaatgttggattaggcattttgggacaagttttgaatcctaactctattactaattcctcttcactagactgagattctggtatgtggtattcaataagtgacttgacttctttaagcctggtttctttttcagtgagatttacagcttagactagtttctgaatcttgaccctgtggacaatctagttggagaactgagatgacctgggcattgtaggatgtttagcaacattcctgcctctgtaaactagacacagcagcacatttacccaacctgctctgactgtgacaaccagaaatgtctccaggcattgccaaatgtcaactgagggcaaaattgcctaccctagccaccttaactgaaaactacaaacttcattgaaataatttctttatggctcccagcagtaacactgtgctattctagaccagttggttaaactactggatgcttcatcagaaagcacccactaagcatcactcaccatgaagttcgttgggtactctatacaatgaacaaaggagatatcacataatttttaaaaaacttaaaagattcacaggtgagaattttgtagtaacaattaagtattaactattagaaaaatttaagaagttttaacaaaatgatataaaaatatattcactataagtaggatgtaatttttgtcctgtaagagttatccatgtatttacgaattgtacctaccagaggttacaaaaatttggtcattatttgaaagattaacagggacttatttccaatcatagatgttcactatactattctaagacatttgcaactgtgtaaggcagtcatttccagtaagaattgctagaacaaacattaagcatttcacagtgaaaagggtcataggtatattttcatcctttgcatatagaagaaatagcaatctattattctcagtttttgacttaaaaggtattgttgcttccctttctttccctcccctactcaagtttttgcccatggatccagatacctacaagggcctaatacagggaaagtgcactgtgtatgagctatgaaggcacaatggaagcttgcctggcaatcagtgccagaacagacagctagtctgatgaattctgctacacatcacagggctactagttttttgttttttgttttttttttttttgtcatacattactgcaagttccctgaggaagtttactgatctgtagttttacgagaaatgcacgtcatggaggtggcgtgggggagcgggtgaacaaggaaactttagttgctataaaacaggagctgagagctcaagcaggttggttatgttctgccagatggagataaaactgtggcagccacatcctgtgactagaaattgtttaagtaggcagacctgttggaggactaaagaacattaggcaaggagattaaattagtgtaggaaaaaaaatcagttttgtttaaaacgaaatatctacttgtgttaatagaacattctaactccaccataggatggaatcaagaggttttttttttaatacatatagtgtatatatataaatatatatatacacacacacacactgtatgtattcctatgtagattaaatattttgatttacctctttctagtaaagcaaagttcattctgaaatccaaaatattcacttactagagcagaaaaaaattagctgtgcatttatgctgatcacagtgtagataattaatctttaagaaagtaggtttttatgtttatagttgataaagtgttagtggcaagaactttttctgttattgaatattatcatcagattactcgtgctttccattttattcctttaaaaaaatccaacttttgtaagccaccactattttctgaagattttatttctctctaagctaagaaaggatgtcaagaataaaccattttctccttttaaataaaaatgcattcactatagatattcatttgaaatctcaaacatacctgaattaagtatactcagttttgtgagtgaaaattaattattatttaaaacaaaacaaaacaaaaaaaatgttcagtgttttcattttacttctcttgctgcttttgggctctgactgggcccggaagcagaagttgcaaaacattatgagaaaacttttgctcttttcttttttttcttcaatctccacccatatggaaataccagaaatctgaaaccccattcttgctaaatattcttctcaggattgtatctctactgcaggtcttctatgacgttttacagctggcctctttccattcagaattgctgttcatctttgaatgtctctgctttactcctgaatgaacacaaacacattttttttaggtttcttgttgacattggctttctttatagcccataaaaaatgcatttgtggcatctcttccacagacaaaaatagtataattatgattcaatactcgatgaatgtgtgttaaactaaactgtgcccaagctctgtgcaacagtacaggtttttcacctttccaggggagagatgtggagcacatatacatttcagccatcctacatgcccacagggacatctttctggtctgtctcattggaatacccttccttatttggtttttagtttctttctgctttaagcacctttcagagagagagagatgttttcctttgtctttgtataggcagtgcctatcgttacagagtagcctttaaatacatatttgttgaattaataatgatacacatgaactgatgaggctctataattctatgagataatctggtatcgtgggaatattttagcatgttttgtatagatagactgacactatgactggtaatctgatagtaaaaatggcaaaatattgagcctgagtattattttattatgttgctttcttatacaaggagggaataaaataaagtgatgtggactgtaattgtgctcatgaaagacacaatgtatacatacctccttgagacggaatgataaggataacgtagaatgtttaccatgatttatcagtctctcctatataagaaaaatatttcttgtcctgaagtggtaactttggtgaagtcttttgcttgctcttttacagactaattaacaagttttctatgccggctctgtcctttcctctcctctcacccctgaaaagtggttaaaagtttggcatttgttacccagaatactaaatgtaacacatatgtggcaagatttgatggaattgcacttctgttcttattatgttcctttctggaaaattatgacaatttgtgtccccttagagagtgtagcacagttttctggttgctcctcatgataatccaaaaaaaaaaatccagctaacccttaccttttagagtaagaatctttagaagaaagagtgctttcatcaaatcatttgagaacgttaagttgaataactgatacggtactaccctacagacatgcgcaggaagtatctgcatttctgtggcgttctgctaaggaaaagaattttctttccagacaagatttttcaaaatcatattttaaaaatatcttaatgatgaatttgaagttgagaaccaacttatttcaagtaaaattaaaattttgagagataagagaatatactttttttaaggttagaactcagaggccattatgacaattaatgggctagtggagacacctggtctctaagaaggagacaccagcttcttcatgttttgatttctgccttgttctcttgtctgtcaccactagacacatactattttatagtaattacttgcatattttgtagaaaaggcagctgtgttttctacaaatatttcacaaatgttagtattgctctatgccaaggaacagaagacaaatttgtggaaaagatacatgtggcccctccccaggtgggatttcttgtgtaggccccatgcagtggagggacagagggggccagtgctcattttgaggacacgatagttcggactgtctgaggaaatcgacagtgtgtgtttaatgaccaaaccaacatggctttgaagaatacatatatatttttttttttgctttttttttttcattgcccaggctggagttcaatggcatgatctcagctcactgcaacctacgcttcccaggttcaaagaattctcctgcctcggacttctgagtagctgggattacaggcatgcaccaccatgccttgctaattttgtatttttagtagagacagggattttctatgttgttcaggctggtctcgagctcccaacctcaggacctcaggtgatctgcccgccttggcctcccaaagtattgggattacaggcgtgagccactgtgcctgaccaagaatatttttcttaatttttctgtaaaactagttgttttagttttcaaagaaagatattttggtagtttttctttaaaatgcatatcatcatacagaaatcattgtccacgtatatggacatatatatctatataaatagattatatctatataaatatatagatatatttgtccatatatatgtccatatatatatatatatatatatatatatatatatatatgatcttttttttgatatagtgtcctagacctggaattcctgtgttaaaaaatgaaaacattttcagtctcttcatatatattgacaaatggctttcagaaaagttgtttcctctattctcttcctaacattgtatgagtttcctttcacatacttttgtcagagtttaattttatcattttcaaaagtgttacttttataaaaactggtatttcttcaatttaccattttgtgattaatttaatttttactgtgttcagggttttatcatatgcttattatttacatttcctttgtgaattgtgttcctatgatttgcacatttatcttttgtgcagctgtgtttaaattttgaatataaagttatatgaaagaggaaatatgtaatttacataaacacacccaaatatatgtgtgtgtgtgtgtgtgtgtgtggtgtgtgtgtgtattctgtgttgaaataaatggtagaaccaggacaacaggtagaggttatgaggttgtcatctgtgacacagtctagaggagaaactgtgtgggcatctatcaacttacctttttgaaagaatcttaactattagtttctggaatattcagagaagacttgtaaggccaacatggactctagtttccatcctcctgagaagacattccattatgaaatctaagtaactttgacagcaaacccttcagtcttatcattttcattagataatctaccaccaacacaatgatccaaaaatgcattatattcttgcactggagttcttcactttttgcttcaccccaaaactgccgctcctaaccacatgcttagctgctaactttcacaccaggcttatgagaacagtattttcagtaagctctcttttcaattcctttcacaatggagctgcagaatctttgagttgaaagaagccttagaggtgactaggatcaatgtatatatatccctcttaccacacacactcactgaatattttctaaaaactacattaagaaaaaaagaaaagcctaatttagtgctgaactgctgaaatattttgaaatttgtggtttcaaaatcttaacactgttaattgaaaccaatgtttctcatgccttttagtctctggactcctttttaaacattcttaaacataaacctaatttttagcataattgtggaatataaagaggttttgtctatgtgggttatatatatttattgtaaaataaactagatagaattttaaaatatttaattatttattaaataataataaatcaatatattaatataaatagcacatattgtatgaaaaacaaccagatattataaaacaaagatttaataggaatagtgtcacttttttgcatttttacaaatcttttaaatgtctgtctgaataatagatagctggattctcatatatgctttaatattctctatctgttgtaatattatataccatatagtttctggaaacattaattttctactaatgagagaatgagagagaagaagaaaaataacttcttagtactgttaggtaaataataatactcataacacttaattaatattattttgaccttgaagaatctttaaaaggttcttggggactatcttgagtctccagaaaacactgagaaccactgatacgccaacaagataaaattcttatccttaccgcagcatggaataggaccatactttcttccttataataatacttcaagtatttgaatgtatttattgtattttcatctatactattattttttaggacaaaatagacttctttaagttttccgtatttgacacattatcttgctcccttccccactacctacctccggttagcctcctctgaatactcttggatttcaatttcatttataatgtgtgatattctggactggacacagcacttcagggacctggtatcttgaatcaacaaagacttgtcttccaaacgatggtgattaagaagccaccatgtccaactggtcagccagtttttatattgtacaaatcagcaatctcagagtcaacctaaccagatttaggcaaggcacttccatgatgtattgatgtattggctattttattaatagtaatatcaataaaaataatcattaagataactgataatattcaggacttcatatgtgctagatgctatgtttaatgcatacatttattcactcttctaattcttaacaactttataatgtatatgtatttcttattcttattttatagataaagaatctgaggcatggaaaatgtaggcaatttatttgagattacagagctaataagaggcagagccaatgtttgatctgaacaacttgattctaggatcattttggctgggaattttctgagagctgtgtgtgtgtgtgtgtgtgtgtgtgtgtgtgtgagagtgtgtgtgtataaacatgagaccatattagtatatacacaaatgtcaatatatattttaaactggaatgttttaatagagtggcttatatgatagaaataagagaaatagaggaggatggaaagggacaaaaaaagggaaaagtaattaggaatattgaaaaacctaaaatgtagttctctccatattctggatactcctgcctttttcttccactttccacacattgaccagtattcctttctcctttcctaaaatagttttacagatactatagatacccttagctatttgacagttatgtttctgttcttttaacatgtctgcttctataactgtcacacttaaatgttttcataggaatcatgaaaactatagtttttcctccaacgtaaggatctcatatcacgctttcattctgaactaaccattccctctctgcagttgatgtaactgtgccatgtgaccattgtacacatgtgggagggaggagctgaattacgcctgacccctggccagagcaagagctactggccaaaggggagattgagcatctgtgttgtacttcccacgtctcttcacctaggaagtgcaatagatttctgacgagtctatgattacccactgatgaataaagacaatctccctgcacaattgcactgcaggcaagactgaacttatgaccaccacttctgtgtaattttgaatttcttagacctgaaccctgctgagtacacctgcttccctctattccttgctgaagttcattcttttcagtgcgttaatggagccaaaccaagctggtggtggtaacaatttgaataataatagtctttaactttttatcttttgaaaaatagaattctcaggagcacttttagctataagattccttcatccaattaaataagctttaagcttcatgaaaagtgtaaaagggcacaggtgcatttgtggaaatagaaggaagcaatcttgagcctgaatacattgaggtactggcaagcttctggaagtagttgaagaagacttcagttagaagcttggtcaaatggacaaagccctgacctggacattggagacctgtagccaccttctgaatccacagctgacctagtggccttgatatataatattgattgcaggatagttttgtgatggttaagattgcaggctttaataactagatttcttggatttaaatcccaactctgccacttactgcttttctctgggaagagtgattaaccgctttgtgcctcagtttccttatctttaaatgaaaataatttgagtgcatacctcacaggtactaaagaataaatgattggaaaataaacattattgaatatatgttagtaattattattttcattgttatgctattattatttttattattaatgtatgacatcatgttacctgcctaacaacagagtattgagacaaaagcaaaatattttttctatattaataatcataataaacaccactaatgtttccaaactatacttttttttaaccctacatgcctttagttcatggaaagaaaagtatgttaaagatgctatgggggtgaagagaatgataaatattattatttaagacaatgtttgctataatttttatatatcaaataagtttatatgttctcagaaaattggtctttgaataattgaggacagtgtgggtttttattctgtttctggaaggcggtgcctgtggctgtgagaaataaggaacagaccatcttcccacatttgagagggaactatacaaaaatgggaaaatatttgttttaaatatcttttggatgtgaattttgtcataattgcaaactgttttggcagcaaaacgaattatttcggtagcaagaagagacttaacgatgctatgtgggagaaaaactaagtccctactatctttctgagagcacgtctcagaggacatgatgtgatcctgtaagtttgtagcaatcttattgtgccccagtgcagacactccttcctacttccctgtagaaaacagaactgtttttttaaaattctttctcaactaccatttttaatagtcatgttacttgatgacaaaatctgatacagtggcctttaatactatatagtgaatgatttttgaaaatttggaaaactctaaccgaaatataccaggaactgctctcctcttcatctcagatgtctacttcctcttcagacctgtgtgtgaagctctagaataggctgtttgggaagactacaaaatctcctctccgaggtcccttataaccctgatagttgctagatttgaaatcaaggatttattctccccctgccctgagcctctcccttatgtccacataggctctagcattggaagaaatattttaagatctctttctttttgactttgtgatactcccatattaaaaatggcttatgacaggaaaaggacaaatatgctatattttttcccttaaggctaatgttctcgggactaccatgaaaaatccaggtatcctaatctggagggttaccctttggatctgaatgggattggagtcagtacaaggggtggggagtgtttttagaacatcccggcagcatttttttttttttttttttttttttttgagacggagtctcgctctgtcgcccaggctggagtgcagtggtgcaatcgcggctcactgcaagctccgcctcccgggttcacgccattctcctgcctcagcctcccgagtaggggggactacaggcgcccgccgccacgcctggctaatttttctttttttttttttgtattcttagtagagacggggtttcaccgccctgctgccttttaaagcaatttaatacatgagttaaatatcatattttaaaaatagattttattttttattataattttgatgaatgcatttttgtcaaagttgtcaaagtcaagaagtcattattgagaccctgagggtaaggcaggagccaagtgagaacaagcagatgtcaaagatggtgaaaaactagaacagccaggtcccccaggcatatacagagaagttttgcaatggcaggtccccgtggttgtctgacccagacttccaccttgaggtaactggggtaactataacgatattttcatcctgatctcttcatgcagttatatgtttccaagaacagataaactgtgaacttaatacaagtgtctcctttccttggattctcaccatctgggtggtaaacatgacagaaacattcaagtatgttcaatgtagtacatggtaacaaatgctttagcacagactagggagcatgtctggcaacatgttggcaaataattaaattggcacattcaggataaaatgagaacatggaaaaacagaatatgattctctttccagccctggaaagacatcccaagtgtacgtattgtttatattatgttattagtatatctttaccagcaaagggcaggtcatcatcattcaatatgctcaaatactcacatttaaagacataggcactttgagaggccaaggggggagaatcacttgagcctaagagttcaagaccggcctgggcaacatggcaaatcccatctctacaaaaaatacaaaaattagctgggtatagtgcctgtggtcccagctacttgagaggctgaggtgaaaagattgtttgagtcgaggaaatggatgctgcagtgagccatggtcacaccactgcactccagcattctagcctgggcaacagagcaagaccctgtctcaaaaaaaaaaaaaaaaaaaagagagatgtagggagcattgtggacatctattcatggagggttaaacaatagaattagacaaccatgtgtatgtgtggaatcatgtgttttttccacacatgtaggaaggagaaggtaggaacaatgaaaagattcttttagtgatcatagtggctccaaaacagatgctttggtatatgtaatacccatttatcttataaagaaaataaagaaataataaaagcatttgctaaccatgttagatgctatagtaaatgtaaaaataaagggtctgttaatctattaactgagcttaatatatgatgtgatataacagcagccttcaaatatgcggagggctataacagagatcatgatgaacagacttttattctggcttagaaagactagacacagaaattaaaggcataaattactctacaagcaaagcaatcttaacataacactcctttcaaggtagactatgaatatttccaccaataatatatttattaaaatagattccttttcatttgtctttttaagttaaacataatcttgcttgaatgaggatgagtataagatacctcagtcatgaccttgtagatcactgcatcagccagctttgtattcagctatcaaacaaaataaaatgtgatcactagtggttcaaatacattggagttctacaactaaagatctaaaggaatgaaatccatgactagtacaaagacataataatgccctaagcaacttacgatattttgatgtttcttttctgacaccccattcgataggcttttgtcttcatgctcagcatctcctatctcatttgggatgctatgcgtccacacctttcatcacattccagcaaaaagaaagggaaggcaaagtggtaatatatttttcctagtgaggttttgcctctttattcagggatggaaaccttccccagaagcttttgtctacacttattggccagaaatttaacatataaccattcattgctgtcagaggtgggaaggagtccctgagaaagaaattattcttgttttccagcctctattgtagcatttaacaaggaagaatgggattatgaatagctttggaatgtttatcatgtcttctagttgccatagctcatagtcattttatatgattgaatctatattaggccttttatctgacaagtttcccaatgtacaaagactgaaaaaaaataattttcctcagatgggaataaagaatgtcaactggtctggccaagtgagtttggaaagctaagatttagccttgggtgcattattgatggacaataaaggagtaggtggcactcatccattcattcagttattctagctgtgctattgaatacttgctaactgcaaagcacagagctagatcctagtaagaatatagaaaagaaagtcacagtctctgccttgaaaacatatttattttatttctaggacaagacatctacacatatacaaactgtcaattcataacatgtcatggaaacataaaagaaggtatcagtgaaagtggagtgtttaaggaaatttccatgcagttgatagaattttaatcctataatttcaataggtagtagctgtgtctcaggcattctaggcagtgcacagcaagagaaaagattgagataaagataaaaactggaaagaagtaggcaatcagtcatatttctgcaaagcaatgttagaaaattgcatgtgttagcttgtatacacaacttagcttacaatgttagcttgtagctaactgaatacagatgtgagagttaaaatatactctcctaacagtagaataatgattgttagagtggcagggatgatcttatagaaataaacattggacaaccagcaaaaacagtgaaagccagccatatggctatctggaggaagagcattccagctactcaaatccaaagtggtatcatggtgtgatgtctttttttttatttttgttttagagacagggtctcactatattccccaggctggtttcaaactcctgagctcctgtgattctcctgcctcagcctcctgagtatagtcacatgccaccatgcccagctaagttatatataaacataagcacagagtaacatggtagcaaaaaataatgtcacccaaattagggttttgaagacaatacaggagttagatagataaagaagagagggaagggcataacacaaaggaacaggaagtattaaaatgtgcgtgttatggacttgcatacaaattgagtgctttaattttgccaagcatctttcataacactataaggaattaacagtatgagatagcataagtaagggggcctgagaacttacataaacacccttggtacatggaaagtaaatataaaatggtgctgataattctaattacatagtttatagaaaagatacatgaccaagcttgaagcaagaatgattgataaggaattaggtaggttctgtataaggaaaggtgatttcagatcccaaaagggcatggctgaatgtttagcctttcagagttggggaatccatttcttcctgtggaaggattagtctttaggtgaatagatatgtatcgaagggaaattaagagagcataagaaaaccccactttacctgccatctatccatggaagcagcaataagaccacctgagagctatggtacaattaaattgaagatatttgaacacataaagtaggtgtaatgtaacatataggctcaaacatttgaaagtgatgatatttggtcattgctggcctacaaaagaaatgattttatgtgattcagtctaatggtaatagttacaaaggattgacttcttcgcaaataaaatggttgaaatagtacccaaaactagcagattgggcaaaaattacaaagaaatatctaagtggttgcatagtaaccacaaaaatgaacacacttattttcagagttcaaaccgtggtagatttgagagtatgtttggaaatgactaatgcttagtgttgtttaccctgtcaccacattcctgcataaggctctttatctctgactggtcatgctcacatctgttttctgccagccttttctggtgcccgcaggcacccacctgcacccaatgtcctccttttatgctttctggcctcctttcatgtactgtgtggtccaccatactacctaatctgctatatactcacaaaactatttacttcttttgaaaaaaatgtattattagatttaaatatatgtatttatatttcccttcactttttaaagttttcactttatttttatactatgttttaagcttccctaatatcccactgctgaatcccaccgacatggaatccacggcatggtgaatccctgacttacccattcctactagaagtagagccagaatctaatccagacctcctgccagccactcccagaccccttctttcccccaaagaaaatgaagaacatattttttgtgcaaagagatacaatcaggaaatttttttaaaatcagcttttattttaactgaatagcttacttagtcctggggctgtaaagtcaactgaatgatggagtcatttttttcaaaatgcgacatcttcttacccacttctcttattactctcatcattatgaaaatcacatttgtgaaaggaaatgaatttatatcaggttttctttggcatcacccaaaggaccttagtaaagaaaattaatactaattttattttctattgtgagcaccttaatacggaactgtaagaataattactatttttaatgccaaatgaagcatgtaagtattactagcttcttttttgtattaacttctatacttatctcaggagtttttatagtgatatagacattttgtgaaatagatcatgagtgaaacatagacctggtatagcttgactggggcctactttacagatttgtccttaagtactgaatataaatgtttctgcttcttattttccttagcatttttaaagaaagtcctggaagccaaaaatctccatgatgaaatatttataattattaatcactgttatatgaccttattatgtatgaaaactatattcaacatcctaaatatgaaatgtgattagttctgattttaaagatttgtgataaaacaagacaccattgatgaaatacatagaaaaaggaagacaaaatagcttgggacacattaataacttacacaaaaaattttaaaaattaaatcttctaatagatttgatatataatataccccagaaatatttacattatattttcaaagtctagagcatttcttccatagactccaaaactatttgtatatattatcatcgaaacacaattttgagagaagttggaatggcagtgcagttagcagataaaaaaaatacccacttttctttacaagtctctatctaattcatactccctattgctctttcctgcttcacaaacttcttaaaagattttttcatgtggtgtgaatatttaaaatctgtcttagcaattttcaaatatacaatatagctggccatctgtatttgtgggttttgcatcctctgattcagccaaccatggattgaaaatattaggaaaaaatgacgaaatacaacaatacatcataaaaataatacaacttaaaagacaatacagtataacaactatttacatagcatttattttgcattaagtattataagtaatctaaagatgatttaaggtatatgggaaaatatacttaggtgatgtacaaaaactttaatcatttcatagtgtatacatatatcaaaatgtcacattgtaccttataaatactcataatcatttgtcaattaaaaataatttaaattttttgaaatgtaaaaaaaaaaaatttttctagcctcccagtctacactctcacttttcactaacccatttactgctttcttgcttgttctcccagcacaccacaaaaacaacttccatgcatacaccagtatcacccccctcacccccctgtttccaataaattaaacccaatggaccaagctaaagcatttattatacttcacctctcagaggcatttaacgctattgacaacttccttcttttcaaaaccctgtcctcccctaattttcatgaaacatgaaactaccttctagttctcttatttatctcagccatctggctcctctttctctattcccttgttacctattggtgttggtatgtattccattctagaactttgtctcctctactgtgatgctatcatttagggtgaaatcaactactcccattgcttaatttgtcttttataaatttgtgacttctacatctatagctccagttctgctgtcttttttgtattaaagaccaatttctccaactatgcactagacacttccaactagtatcccactggtatctcaaattcaacattattgaactcaaaaacttcttttgttaacttgccttgctgtcatatttcctgtattggtgaattatatcagcttccatagacttgcctgagccaatataacctaggacatattctccttttcccttaactcagcattgactgacaaagaacatgctaggaagtctgtattcttcatgtcttaaaatattcacctctgcttccattgccacagctttgatttgggccactcacatttctgcagtagtctctgagattgttatcatccatatctctgcatttttcttgctaatgagaccttcattaaaattattttgtaagtatttaattatttagcagttcatgcctttccatatgacttaaaattccattgggttttgcttttttcctgtaacctaaagttacatctgggttggtcaaagtgaagcatagtaactacattccctttgatagtgctgcaattaagaccaatgaaatgtgaaggagttttagggaagctttttcctcagtcttaaaaagagacaaaaggaaacaatacccctctcctgtctctggttcatatttgatgagaatgtggcacctagtctttttgagaccagtggggtagttaggcccacaccctgtggatgtcagagcaaaaatatggaaggaatctgggtcctgataccatcatcaaaccattgagctaattccgttttgtaagataataaattccttactgtttactctgttcgagttccttttttttctgttagttgtagctgaaaccattttaactgttgttttttgtttggtttggttttgtttaatacggagtcttgctctgttgcccaggctggagtgcagaggcgccatctgggctccctgcaacctccacctccagggttcaagcgactctcctgtctcagtctcccaagtagctgggattacaggtgcacgccaccatgcccagctattttttttttttttgtatttttttgcatttttagtagagatggggtttcaccatgttggccaggctagtctagaattcctgatctctggtgatctaccaatcttggctacccaaagtgctgggattacaacccactgtgcccagcaccattttaactgtattctaaaagcattttacagcctgctaatacataacctcatctccaaccttgcttcctaagttccactctgtgttccacaaatgggattaatcacctactgaaagctctataataattcctgtcacctgaggatattgttaaaacttctcagtttgtagaagagggccttcattatcagcatcacatttattttccagaaagatatctagcacccctctaccttacatcttgcttttcagccaggaagaacaactttttctttctgaaatgtactagaatctcagtgttgggccacattgcttttttttttctaaaagactaatcgtcttcctttcccacctaactcaaacatatccctcttaacttagacattacttattttggggaagtcttccatgattaccctaagaatagggtaggcattctttctctctgcttccatagaaagtaggaaactattgcacttactcattgtaatgtggctatattttgatcaaaataattaaaaaatactgtgtggattcaaatttttctcagctactcacaagctgaatgatctcacacaagttatttattgcaccttattgtgctttctttttctctgaaatagaggtaataattatacatacttcatattattacaatgattcaggaagctaatgtatatggtatacttacatatatatatgacctagtataacgcatgatacataataagtgctgtgtacatgctcagtcaaataatggtcatttgaaaacatttattgagtaaatgaagaggaaagtgtttattttcaatacattcaaagatattgttttggttatttccattacagaggcataatcagtttactattcagaaaaatgcaagagtacatttttactgctcctccagtgatactatggaaaacaatgttttagaaaaataaagaaggtgtgaataatgattaaagaatcatacactctcaaagtgaaacaatttcccaagaaatgcggtagaataagccttttggtttctgattttttttcttaactttgcttgtatgttgtagaaagctaatctaaatttaagaaattgaaattttgaagtattaataatgtacttctctcccaaaattgttttaatgtaatgatttttgccatatggatgaattatatatgcatctagaggctaaaaaccataaaaacaagcttcttcttagtagacttttgttgtttattttgtacagcataaagcagcagtcaaaaagttttccaaacaaattatcttatgtattttgactaaacccagatttatcttcttaaaatgaagacctttgttgtagttgcatttgttcctcatatgcagtagaatgacccagcctctttggcttagaggtagtgcctcctttttacgacacttggagcggcatctgatgctcatcacttcagttggataaggaatgctgtccagtcacagagactcatgagatcatgtccaatgaaggcatttaacaataaattcacaactagtgagtgagaattttataaagcagtttcaagtattaagtagataggtaggtaagctttattatattttttaaatgtgaaattttacaattgtgaaaatttacaattttacaattttacaatgtcaggatggataacattgcctttttagtaatggtagccttcactatctgcattatgactgtacaataataacatataataatatatatagcatatatattttatatatataacataatatataacatatataataacatataattataacataataactggggctatgattgcaaacatttataagatgtggtatgaaaatgtcccaatcacaaaaacactcaatttaaaaatgaaagaaaatgaatctatgctatgctttgcttcatctttctctgaactagttacaaacaaaccttttaaaaataagctttcaatttgggaataattttagatttacagaaaagttgcaaagatagtaaggaaagtccccatttgctcttcatttggcttcctctaatattaacatttgccaaggttacatttgttaaaactaagaagtaaccatgggtacaatgctattaaccaaattacagctttcatttgaattttgcccatttttccaatattgttcttttcctgctacagcatccaatctaggacctcatgttgcatttatttcttatgcatctttagtcccctaggatttgtgacggttttctgtcttttttcttttgaagactgttcattgcctctgttagtttaatgatcctctgagatgttattcacagtaaaatagcatgtgaatttcacctaactaaaaagtttatttgatccaaagccctgattttaagaatttgaaagaaaaaaatgactctatttttcccagttctaaacattttactagaataataattgtattctttcaacatggaattaatgttgatgagaagcaaacatctaaatttaaaagaaaatatagtttgttgagggaggtaatagacaataaaatgtatttattatagaaaaaattcccaaaactttctcattaaatgtgctttatctttacttcattactaatatttagcttttattcttttaaaaagcatatgccaatgataatatctcattaataataagaatccatctaattttagcttgatcttccccctgactaggtttgattggattaaatcatcataaagagacaaaataatgcaaaaagtgataaatctataagcctcccctaaggtttcccatagaatgatcaacccaaatgtgctctttattttatgccatgaaatgacatactgtgtcaagaactgaatttcatcatacatgagacgtaagactatttttatatctctgtaaattgggtatgaattataaaagtatgctggtaaactgatcacttgagaacataaagtcaactttccctggaagagtttctcattataaaagaaaggcaagcatcttcttcctaatatctagctttatcaggtcaggggctatattctcggaagggataagtaatttctgttgtatctactaatttcatttaaaaagataactagagaatattggaagcattattgtagaactgtgtcaaagaccgaaatatcattcctaccttagactgtacctcaagatcgaagctctggatgctatctggaattaaaatgtttgcattaagtttaaaactcagtaaaataaatgtttgaaatgaaaaccagaccaataatgaataattttacttagacctactctccaaatgtgctaaaagacttgtaaaagttgttgttgttttaataactaagtcaagccagttttatttaattcaatacatggagtattaatgcgctgtatgaatgccgaaggtagtattggacgccacaatctttaggaaccatgcttctgagttttaaaatggtgactagtttagcatagattcaacataagcattaggtgttcttttgacatttgggaatcagccaatcaacaggaggaatagtaaattgaatacgaacttgaaagagaccatgtctttttttcatccaactgtgaaaaactttctttgtacaattgttaaacttaagaaacagatggtagatctgtatcagtcagtgaggggtttctgaagtacttttctggatgaatgccaagaaaatgggtttctgagacttgcatggctctggatttgttctgagctgtttagtgaagtgagggctggcattcagaacccaggggagggggagtagtcattcccattgccttgcatagagatagaatcacaggtgacaggtcattggaaaatcacttcttgagagtgggtatctttattttgagttggtatctttttgagagttggccactcataagccttgcttttgataacatttctttaaattcctccaaggaacaaggggaagtgcaaaaggaatacgataaagtgcagcattgaatgagataagcatattcaacttaaggggcacactaaatactgtaatctgggagcataactcagatttcttttcttctttgctcagtataagttgcatgatcatagaagatttatgtagaagtcagaaatcaaggtcaagagggtaggcatatttagattcttaccctattcataattaacaataaaataagattttgtgtcctgattcagagaatggatggctcagtccttataacctcttaaattagttttatctataactggatttctgaatctcttttgaaaattactaccattgatggtcactgagtgaaaaaagcagaaggatagactggtgttaactgtaatgaacatttatccaacattacccgtgggcctgctatccattttaaattctaaaagcactttacagcttgctaatacatagcctcatctccaaccttgcattcctaagttccactctgcattccacaaatgggattaatcacctactgaaagctctataataattcctgtcacctggggataatgttaaaacttctcagtttgtgagagagggccttcattatcagtgtcacatttattttccagaaagatttctagcacccctctaccttacatcttgcttttcagccaggaagaacaacttttactttctgaaatgtactagattctcaatgttgggccacattgctattttttttttttctaaaagactcatcatcttcctttcctacctaactcaaacatatccctcttaacttagacattacttattttgggggagtcttccatgattaccctaagaatagggtaagcattcttcctccctgcttccatagaaagtaggaaactattgcacttacacattgtaatgtggctatagtatgatcaaaataattaaatctaaacaatactgtgtggattcaaatttttctcagctactcacaagctgctatccattttaccaagcctcctgcatgtattactatgtctaatcctcatatcaactcatatataaactagattttatgattatggctctaaaaacaaggagactaaacctcggaaatatcatttaacctgtacaagaccttacttggctgagctaggattcaaaactaggtcattccgaggagaatataaagtccagcttttttttttccacacagggatgtatatttccaggtacagttttacattttgttctttattgtatgaacataaatatagatacatatgaaaattcgaaagcacatgaaagtgccaagaggaaatgcaataccatcttatgaaatgagaaattacacatatcttacagtgagtttcaaaattatattgctcaaagtatttttactgtggaaccataggcacaaactatagcaagagtaaatccaaaaatgtttattgttcttctataaactaactactgtgtaggatacaagggatgctgatttcaccagtgcctttaagaaggacaaatcaaattaaaaagtcaaaatgactgaaggtgataatccagatggtggtaacaataatgactaccatttatagaactttttgatgttgttcactcaacgtttctatttttattcaattataagcaaacagcagaattaacccaacattcagcaactccagatcagcttttcttacccccatgaagagctatcaatttaacaaccacagttgtaaggattcttaataagctgtcaatgagcactgctgccggtctagatggccatgccccaacaaaagcaaagccactctccctaatgctttttccaggattgctttttaaaggcaccagagcgagatactgacgcctattaaggcatctgagatgcaccgtgttggggtttagcctccatgccagccagcctctggttgtctaggtgagcgacagcaccataaaaacacgctgcgtacaattctggtattaggatcacaaaggcagagaggtgacaaatcctttttctttttctttttttttttgtaacctcccttaaagattctttgatgctttgctctattactgtgggcctggtctttttttcccccccagttttttcttctttaaactctggattgctattttcatattaatttgatgaccccatcacagtaccagaatattcctgaaaatagagttccaatttgatcaaaacataaaccagagtgagtgagtgagtgactagaattataaaggccaggcagcaggaaaagttaccctaaaccatctgactgctcaggtcttgcatgtgcaaaggggagccggaagaggagaaatctattatacatgcaacactgaactggagaacacggcttggggcctctgggacagttcaggtccctgagctgccccctacttcccagacagctgctcctgcagtttgggcacatagtcgtcccactcagcctggtaacgctttctggccactggggccacgagcacgagctcgtacttttttttttttttttttgagacggagtctcgccttgtcgccaggctggagtgcagtggcctgatctcgcctcactgcaacctctgcctcccgggttcaagcaattctcctgcttcagcctcccgagtagctgggactaaagccgtgccaccacgcccagctattttttttttttttttttttgtatttttgtatttttagtagagacggggttttaccatgttggccagcatggtcttgatttcctgacctcgtgatccacccgcccccgtgatccacccgccccagcctcccaaagtgctgggattacaggagtgagccaccttgcccggccaagctcgaacttttgacagaaggatgccattttgaatttgccactgtggcctccagatccattgctgaggatgggctcgtcacacttcagcagcctgtcctgtttgtaaaccagccagacatagcggtggagatctgtgccctccggaggcccgagcccacgtaatggagatgactgggccactgctaacgtcattacccttcatgttgaccaccaggaaatgacgccattcagtgtattggggcttcttcctgccgggagcgtccgggtctgttaggaccaaggtgtagagtttccttgactcaagatcatcccatgaaatgctggtgggtctgttaacctaggtgggcgtcagcactttgcccagctcgtccaccgtcgccctggcgtaggcgacatgcagcgagtgctgcggctgcccgtccacttcctgcaggctcaagggcctggaccgcttgctgaggtccctggcatggctgtgcaagaacgcagcgcgcagctgggagtgccactaggcaaggcgcaggcgcagcggcgactcggcagcctctgaaaactagccagggaagccggggctcatttataggattttaaaaatattattaaaggcttcacaaactgtcttgtttaatagccacaacattgggaggccgaggcaggcggattacctaaggacggagttcgagaccagcctggacaacatggtgaagccccgtctctactgaaaatacaaatattagccgggtgtagtggcgcatgtttgtaatcccatatactcaggaggctgaggcaggagaaccgcgtgaacccggcaggcggaggttgcagtgagctgagatagtgccacggcactccagcctgggccacagagcaaaactctctcagaaaaaaaaaaaaaaatagatacaacaatctccttttaactgaagaggaatgatgtaaagttatataaagttcagaggaattgatgtaaagtgaatcgtaaagactttggaatctcctactaaaatattttaacaggaaagagacacatcagtgcattttacaagcagatcaatgtggcggtatctagcatgcatggggaagggatggaggaagttgtcagtttagaaactgagtataaacattattgaaataggacatgataagtacctggaccagggtaaaggcaatggaaaggaaaaggaagccacagaccacagataggaggaattcaaggactgtgtaccgaaattcaggagaatgatgtgaaatagatgctctgaatcctctattcccaggaggcagcattatggagttaggagaaaatgcaggagctttggattctagtagacctgggattgagtttttacactgttactctatattcgaagcaatatatttaaaccagctgtgtcttccttttgtcctttataaaacaagaataataatgcttatcacatagagatattatgaggattgtataagacaatgtatcaaatagtaggtattcggtaaatgttccttctttactaaagatagagaaaccattttctgatgtacaaagggatgaagagctggcccaatatgaattttcccaaagaagttaaatgaaaaggatctcatgatccttttcaggatttattatttacgaatgttaatatattattttaatattttctatcttatgaaataattatttggtcaaaacataagacaattgataggaatatacagcatggaaaatggttaccaactagagctgcagggtatcagggaatgtgacaaggcagcaaaatgtttctacacatgtctgttttttcaggcattatctttcttgagactatcaagtgtgtatttaaggagccattcaacttacttcagtgcatttgcttgcaaagggtgcaatgtgatgtttcctactggtagggtcgtatttcatatgtggtgatagtgttgctgaacaaataggaaatatccttgcctagactatattttatcatttcattatctagtggtaaaggaatgtgagttctatttacaaataaacattttgtcttacttttttctttgtgatctattttctccaagttgcataatgtaatgaattaataaagcttagttgctggccaaatcaatggtgactttttatgtttttaaatataatattaggtttaacttatttttgtcattaaaatatcatttgtgagtgcttttcaaaatgaagtgcttctgaaataaatcacataataaaactaaccttacttttgaaatacatttttattgaagcaaacacaaatcaatctgaaattcagcattttgtagcagttaaatgtatagtcaggcagcttcaacgtcaactagagaagttgtggttttaaccccgagatagggctgattatgctggtgctatggcaacctattgcaccatttggtagcgcctgtgtgcttaaccgcatgagctgcgcctcttcctttcctataaagactcagaataagaaaaacagaagtacaccgaagagaagaaaccacaagagcagtaaagacactgctgttagcttttagctgtgcaaacagcagtcttatgagaacaacacattgaaaacctcttctatttgaaagtgtagcttttcccattatgcctgggttcctttaatgattttgaaagtaagccaagtgtttctgttcagagttttcattaaagggaaataagaagaaataagcagtgcatttatcagcctttgcttttattgtcctcagctttaggagtgggaggcttttgtgcagcctcagcagacattttattctgtttgtgagatgggagattagtttctattaggtggactccctataatctagcatttattttctgcttttttttattatattgtagttagttcacaaaaaaaagtacaattttaattcatctcctggctcatttagaaagggttgtggttggtgctgtaaacacgtttctacataactagattaaattcacagacactcactgtcctagcactgtttattttctatggggagcttcatttacctattctttccctcaccccacttcttttacaaggtataggttgatcagcaaaggcttttgtatgttttcctttgtttcaaagtacagacataatataatcataacttttttttgcatgttctactatttttccttccttaaagatttgggtaaaaatactgaaggacagacaagttcatgctaccatttttgttaggcataggcctgttcacttttcttcccatttttctgaaaaataagaatctaccccttttgtagtcattgtccagcaatttacactttttaacaataagttttaatgtgtggtactctgaatcccattttgatggttatacataatatttactcatttttgagtccctaatagctctttagcacaaatactggatttagcattaaatattttttccttacagtgcaatgcagttgaacaagcatgggggtttttacagtcagacagatctgcatttaaatctagactcattttgctacaagttctttatttagccttgcatacacgtttttatgattttgagctttcatctgtgaaaagaagagaataccatctactttgtaggatttctataatgattagataaaataatatgtaacagtatttaggacagtgccattcacatagtacccgcttattaaatagtaaacactgttgatagcaccaaatacactaataaaagatttcaccacttatgcaaacatcttttgatgattctttgttctttaatgatgatcgtaacctatcctagaggaagcaaagagctacaaaaacatacacttactaagggattaatataattaaatggtttttgctatctgaagtatattgcataaatcaggtatatatccctggatttaggtaaatgaaaacagacattttcataagaagcaaaaagataattaatatgggaacaaacctattctggaaaatgtttaaaaagagaatatgggtaaggaagcatctttctcagttgttcttaacccttgtttccatcataatcaccatcagagctttaagaaaataccagtgcacagatcacgttaccccacaaacctactaaatcagattttccagcgctggagcccagaaatagtcacctttaatctaattcccagtcaggattaatacaaataaaggattgatattttttcttcctcaggataataatactggttacacacacataaatatacataactgataacaagccagaattttgtaaactatgttctcagaaacattgcagttacattgtacaaatgtcctatagtatgtccatgggaaaaaaatgggtttgtggcaaatacttttaggagatcttgagctaaacgaagtgacataagtttctatgcttttaatatattaacacactttataaatatctcaaaagggcatgtagcatgaattacttctgaaacaaatttgactatgggacatttaaaggcacacaaatctaaatcaaagacttcaatttgaccatcattgcacaggaagcgataaaattttccccctgacttgtagataaatagtttaagacagaaaaaaagcagtgtaactgattgttcttaaatggttatctagtagcctttattaatttttttgtcattaattgtttcgttaatcaacatgcctgaaatatataacatgatgttttaaaccaaatataaaatacctacaaatgcattcctagttttgaggtgtgtgtttgcaaagtcatatgtattcacaagcaaaaaacattattgtaaatattggacaccataagtcattgggagacagctagatatggttgctatctttaaaattttttaattatttgattttattcctctcatggccacaaaaatttgccttctttatcctcaatactgctttacatactgatatttttctttattatttgcattattatttaaaagtgtgtatataatttgaaagtttaaatagtaccataaggcctagagtaagtaagaacagtcttttgctcccacgactctcccctcccttgatattttgtgatttttaaatgttatcttttattgtagtgctgtttctttaaaacaaaaaaaaagatttttgccagtatctattgacttcttctcttgatcttgagatgttgctttttataacctcttgctctttgttcatgggtgcaatgttttctcatttctgaaaatatgaattgtagttggttatcctctcttttgctccttgcattgcctcattctcccaagtgcctcttttgtttatttgagctctatctttctttcttattagaggctttgttctagtgtttcttggatgtccatttgtatttaataaaaggcctcaataaagggatgttgaaattctttggacattggtggagctcataaattcatgtgctttaactagattgaatgaaatcagaaaggcactacactcactgagtcttagtttccttatatatcaaatgaactgcatgtcaataatcactaaaatcctttgcttctgtctgagtagaaatctttggaattattttctgatgataagcagaaagtcctttactcatgagattccaaaaataatattaatatacccaatattttaacataacgtctacataaagaataagaaaattattaaatagacactatttcaaatctagcactttcctcgtgtgtgcctgtgagcaatttactaaactcttttaggtcccagtttcattccctataaaaaaggataaataatgctaactcattggcttactgggatgcttaaaagaaaaaaaatacatatatattatataaagaggtgtgcatagtgtctgctacataacatttcagtaaactgttgccatcattattatatttactgataagctaatggagggtagaaaagactgtttcctgtggttctctgaaatcataatacctggcttgtcgctgcccagagtgcttactccataaatacttaataatttaatatgatttgttagatttattgtctgtggaccatatagcagatttctagcataaaaaaagtgcaattctcttatttttattgtgcactttattattatcatgcattgctaagaaaggaaagccatacatatctgttttagctgacccttattttttgtcttgatttgcttttttccacttttgtacaggctttatgtttatggaggtcaagtatgcattctcaaccttcaaaacatgctatcattcattttagggcagatgctgagaataagtatttatttaatctattctattttacccttctgcccttgtacttttcccagatttgcagaactagacaggtttaaattccctaggaaatagcatcccatttttttttcttttttttttagcggggagggagaacgggtgatatttaaagcccaagtatgtcttttgaaatgccgttttcactcaaattgattcctagtttttgctgaaatctctgatcagggacttaggggtgtgacttcaaggtaactttgatttgtgatcatttaaacattttgagttgtaaaagaaacatattgggaaaggtaaattcagtaacaatacatgtgttagaataacacagctttgaagatcaagtgttctgttatctacattttcatctgtttaatgtatctagtcaattccattggtgattcacaacaggattataatgggaaaaagagctcttagataatttacagttttttagtgctatggtgccacctactgaaatattactaaatactcctttgactaaataatgaaaacacaagacatttaagttttaaaaaatgtagaaaatttcatccctagaagataaaagtcaaagtgtagaatgtagtaactgtaatatgtggaacactagatatattactgtgttttattttatatttatttgatgtgtttatagaatttgagagaaagctcaatgcagttcttactttgagaaatagtgatgccttctctttattgtcacacacctacacatgtgccctcttaatttccattgctatgtcacatattttgctttacctattttccacactttcccagtattgttcataaagaatgtttacatatattgtagtgtaatttgtattaaacaatctccaaatattaaatatttattgtgcactggttataaaatactttatgcaaaaattttgtttgcttttcccagatctatttgactccactaagaatatattgttgcttttaagtaatacaggaaatagggtagagtacaaggctgtctacatacataaaacaacttaggtaactacatcagttcatttgttttgcattggacaagcacagtaatatttaaccatatactccagtctaaatggataggtcatgaagtagttaaatatgttatacaaccaatcttttgttgttgttgttgttgttgttgtttttgagtcagggtctcaccctgtcacccaggctggagtacagtggcaccatcacatctcactacagcctcaacacacactcatgggcgtagcctcccaagtagctgggactataggtgtgcaccaccctacccggataatttttgtattttaagtagagacgaggttttgcatgtttcccagactggattgcttggttcaagcgatccagctgcctctccctcccaaagttctgggattacaggtgtgaaccattgcacctggccacaaccaatctcatcaggtcttttttttctatcagtgaagattcagcacagtggcttctatctatgattttggtaatgtttaataatgtttgcacatatgaagtgcaacagacaattgaagtcattgctcatgtaatttaggaagaattaaaatatgatagagaattaataaattattgcagatatttggttttatagttttctctaaatagttaagtaccttcacctactccctaccttgtttcatatataaaggcattctccaccaaagtatttgttagtgttctgctaacgttgatgtaaaaatcattagatgactgggggggcggggtgtggggaatgtcctttagatgttacgtaggtgttttaactaagctattttatataggtcacatttagcgtgttcctactttaagactggtaaaatgtttaacattaaaaagactgaaaaatagatttatgtaatctagtgcacatggcttattaaaattgatatgttgctttaagttgcatcactctagtgcataccttatttccttaggggcattggcttaaattttaaagtagtttttaatttaaaatttttattttaaatagattctatgtgtttttttcaggcacgaaaacatttttatgtcatttatcatgttgactaaaagtgttaccaaaactaaaaatctgtttatagggattttatgaccatgagaacaagcaagttgagtcttacactaagtctaaacagtgatgctgaagtcttggaattttcttttaaaaagataaaatggtgtgtggggtgtgtgtgtgtgtgtgtgtctgtgtgtgtgtgcacgcacatatttgaaatagtatataaaaatgaaataaaacatagattacaatgttttagtgtcacctaaaaatcactcagtggaggaatttagaatcatatccagtgataaatcagtgtacaagcaaacacatattcaattcaagaggcctttatgggaagtaagcatgaacatagaagaaaggaaaatgttggctctttagatattatactgttttccaggatattaaattttgctgcattaaagatgaaaagattcgaggaaattttgaatatggagcgatgatgagatcagaaaaaaatgtatatgtatgcccattattctgtcctctagctccagaaacctcttaacatctaaacaaaaggtctgtaaattttaataattgtgcttgatattagtgtagtttggttgactttcctgtcaaaatagtattctgtaataaattaacttgacacacctctaaattttctctaatatttgtttgtaccattatagagcattcactcagcacattgtgatttaatctgcatatctatttttagggtcaaggttattttagcatttgtagcactactagtaatttacttgcagccaaattatgattaagatgcatttttacttagctcatgagtttttaataaacaccttctgtaaaagaattctcatgcttaaaatttcatatgaagaggaaaggctgtaaggacaagttgatgggaaaaggggacgcctgatgaatgagagcatggcctgtaaagtcagacaggctcaggttcaagtctggctcacatatactagactggccttgtgaacttggccaagacacttgacttttctaagcttcttagggtttttgtggtgcttaagaaagaaaacataagcaaaagacttagtatagtgcctggcacccagtaaacactcaataaatattaacaattaataacaataaaatattatttctaaattattctttaaaaaagtaaatcattagaaacagtcttctccgttttggtaatttacctcttgtccttcttttcagaagttagattaaaataatatacatcatgtatttcttttaaaaaacgtattgcctttggaccacttggaagtttattaatctctctgagacatggaacatatacgtagtctgatgaatagtgtactggttggaaacagttctagtatatttactcaggcattcacagttcttttgttaaaaaacaaatagcttcacatagtgtcccagcatttttcttctcatttctgtggtaaacagatgatgaattataattttcttttatgaaactctatctatagttggtgctacacattttggtgacaacaaagtagtaaatcagaacaacagaatataggggtctgtggaattagtggtgcaggtaacattaagatttctcttttctctgtcatcaaatttgctttctgatttctcctctgtattaactgatccaatggcttccgtcattctgaggaaaaagttcaagctccttttcaaggcctacagtgcttgctccttggctcttctcctaaagctgttatcatcagatctgtttgatttctcctttgcacttactcatgcttaaaagaatccagcaattacttatcaatcacttcttatacacaagactctttgctacagctatttctctttcttctcctcctcttcctcatcttattatgtgattcatgctgatgttgatgcgagaaattttgattattagtcttaatcaggtgtatccatgactaaaatgtcattgcagatgactagatatatgtgttttatgggttataagcttatccagggcaagggtcatgcttttatcatgtttgaacctagtctccaacagcataccagcaaaacaatgtatgtttcttgaacctaagtgaactaaattaacttgtttcaagttccaaggaatgaggtgcttgcatgagaaggggcatatcaacctaattttagatatgtaagagctcatgtatttctcagataaagaagagatatgtgttgtataaagtatgttcacacactcaaaaacaatttgaatattttaaatttggtgatatgttttgttcttcacaaacaatgaaggacacttttcctttcacttcaaacatgagagctattagttattgctatactaatatttttttcttattacctcttttgcaaatcaacacaattctaagactgtaatttacaaggaaataagaacaaataaggagagcggaatgctgttaatgggaacataaacataacaatagtttacatgaaacagaaagataaaagctaactagataagaaaagggacaaaagtacaaacaatatcaattaaaaacaatatttaagtatgaattattaagaaaaagagaaatgtaatgagaaaacaagaaagtcattatgttaataattatgtatcacccatcaatgatataaaaatatatatatcaaaaatgcattttacttcaaggaataagccagggaatgtcattgaagaatacggggtgatgctccttggatggcaactctgaaggaagaaaatgttttcacatcagtttgttctcagaagataaaatataaaggcagaaagtcaccttaagtaccagctaattcactttcccatctgatctctgattctctttaacaacctgagtttacagtcatttggaaaagaactttacaatcttttaaataggcatttactaagatgagggatgaaaacattgcacttcactgtagactgaatctagttcccatcatgccaagaaagctgctcttttcaacatttccacaaacccagatgataaatccagttgacccatgttaatgcaccatgtttatcctgcatgtgaatccccatattatttgacttcaaccatttccttctcgaaacaccctctactctttattcttgtttgctacagttttcctcttacttggaaaatttgattacctatgctggctctctccttaatattcactgaacttcaggattctatcctggacacttctcttttatgtagttcggtgatctccttcacctctgtagctgcaaaatgtatctatatgctgatctatagcatcagcccagatgtatgtcatgagctacaaacctctatattcaaatgctattatacattttcacatgaaatctcaagcaaattctgattcacctctctactcactgtttattactctcaagttcagtgaaactataactcactagcatgttaaactatcaatctagatattttccttattactctttctcctttattctcacttgaaaggatttacaaagtcttggtgattcttgagtgtttcataggtccttttcccccaacctttcttttggggtatactcttcctacgtaggacatcatctctgtctgttttgctttggttttggtctcctgattttcctgcccccacctttgctctttaataatccattttccatttcctgaaaggttgatctaaaattcaaatgtttctcctttaggcctccctttaaagacatccctttaatggatatctaaagcctgtaagataaatcccagcttcttattcttctgggaccaagctagctatatgcaatcctttaggttgtagcttaaatacatccaagaaaccctctgtatcaactcctttaccagccaaccaccaactctggaaatataaataagatgatcctgttatgttctcctttagcacattctgtatcacctgtcatcacactgtattgattgattgtttttgtttatatctcacactaaattgagctcattgagggcagggaatttttatatgttggtcatattatatccctagcatgtggcataatgtctagcacaaaataggtgctcaattaatcatcattatctaaataaataatgcatttgggaaaaaaaagtttcaaaagtttttcaaaagtcttttgcaggcttgaaattaatcccaatagtgatcctttagtctgttatgtttctgatttagcctggggattcaaaaaataaataacataattttgatatatttgggctttgtaaacatggtactaagagaggaaatatagtttcattagggtaaaagctactgaaaattgccacttggtgaatgttctatcatagacttgaggtacatataaaaatctaatatatgtttacattaatatgaatgaaatttgaaattttctaagagatttttgtttcttctttgcagggcaaagcccaacaccttcccccactggtaagaattaatatttatatttttactaattttattttcttgttgcaaagtttatatatttaactacaattttctattattaacactgaaattatttttaaggataaattttataatcatgagtgattcttgacattcacttgttcttaaactttctgcttatacgttatagagtttaataactacctaaacatgttattaaatttgtatatatattttgtgtataaatagtaacttttcccaaacttgacagtaaatcacacaacaggtttctactctcttttaatattttaagactataaaaaaatgcatttaaattagataacaaaattttatagtctgaaagcaggttaacagctgtctatgtatgttatagatatgtagataacagatttgcatatgtctatatttctttaagagtatgttgcttttttcaatggtatgcaaaacctttgagactattgagatatttttaaataataattttcaaattctactgaacacttcaatagtccttataaatgtcttaatcatgagataaatttaaaacacagagatgctgcaaataaattcatacatagtacatacaaaataagagaaaaaattaaattgcagatggttaaatatcacatcacttaactgatgttactgaaaatgtattttcctgcataatcatatggttgacagtatgcattaagaaggtaagtaaaacaatgaagacaattttgatttaatatggtaatgcacaattccaactaacgtacattcaacagatcatgaaattgggttattaaaatgaatatttttgtcattaaataaaaattccgtccaaatgaagaaaacaaataaccatgaaaatagtaacaaaaacacttctgaatctgcataagaactatatttccttatttttaaagaaggtctaacacaattttacagcgtttagcatggcagtgatgttttataaataaataaaagtcattcttgcatagtagattgtgattggtttatgccagctactcaaatgcaacttagtatctccaacttttacagaagatagattcatctcaaccataccagatggttatttttgcaggaaagggataggtataaggtagaatggggagtgattctttaaaatgacacatgactcatcaccttattgagggagtttctgttatctctgaattgactctattatgacaagcctccaagtgatgaaaccaggtaagttaaaactgttaaccaaaatgcaaaggaaaatggtctctcccaaatattggccacaacaatgtcatcaatggaaaccaggagaatttgcaaagtggaggttcaagaacaatgtggaattggcaattgagtcaggttttctaattttaaattcttatttgtgaaagggaatgtgaactgaacttaagatgtgtgcaaagatatgaaggagagtagttctctgaaaacctttctccctacccctgggactgaatttgcttggctagaagtaatctttaggaatgctactcatcaaaatagcgtggtactatgtattagtctgggttctctagagggacagaactaataggttagatgtgtatatgaggggtagtttatgtgattgacacacaatcacgaggtgaattcccacaataggccatctgcaagctgaggagcaaggaagccaatccaagtcaccaaacctcaaaagtagggaagctgacagttcagccttcagttggtggccaaaggcccgagagcccctcacaaaccactggagtaagtccaagagtccaaaagctgaggaacttggagtctgatgttcaagagcaggaagcagccagcacgagagaaagatgaagaccagaagactcagcaagctcacttctcctaccttcttgtgcctgctttttctagccgtgctggcagttgcttggatgatgcccactcatattgggtgggggtgggggggttggggagggtctgcctcccccagtccactgactcaaatgttaatctcccttggcaatacgctcacaggcacacccaggaacaatactttgcatccttcaatccaatcaagttgacactcaatattaaccatcaaatactattataaggagaatgttgcatgattttccttctagtctgtttgtaattcacatctaatgaaagagtgagagtggacgataaagggaacttgttgaaacatttctctcaaagcaaaagggatcattggaagcaggcagacaccagaattggtttaacctaaaaataacaaattaataattatcaagtctataatgatgacagtgacttaatgtgaatagaaagaattctaaactctctccttccttcctccctcccttctttcctactttctttccactccctttctcccacccccttttcttttcctttcttttctcccaccctctctccctccctttcttttattcaatgcatagtagttgaaaaaatctaaagttagacctgattttacactgaagactagaggtagttactatcctattactgtacttagttggctatgctggcatgtcattatgggtaaaagtttgatggatttatttgtgagttatttggttatgaaaatctagagattgaagtttttcattagaaaataacacacataacaagtctatgatcattttgcatttctgtaatcacagaatagttctgcaatatttcatgtatattggaattgaagttcaattgaattttatctgtatttagtaaaaattaactttagctttgatactaatgaataaagctgggttttttatttatcatactatttccattttcttctctagtaatattgcaattttcattcttaactctttcctgtcctatcatttctactccttttctagtttctctcattctctccctttttccatatttgtgccattgtcttttgcccaatcttgttgaactgatttaattattttttgttgtgtgatatagttcagtttttacctaattaaatatttaaatttttttttttgcttttcaaaaagtaaatatatgttaagcaaaaaaaaaaaaaaaaattaaatacatctttataattccaacctccagagatcacatgagcttttttttttttaacacatttggtatatttttctattcttttattaagaaaatcacttttttcagtaaaagagcattaaaaaaactttaaaggactttaatcaacagtgctgatttgccctgcagaattttttttaccattgtacactcatgtcaactgtgcataaacttatttcactactactttgtcacatattttcctcttcttaaagtaaacttgagctgtggatattatttcagtattttaaattgtatctctttgttatcatgacgtcaaagacatttttgtagactttggttgtttgtaaacctagttgtgagttttgtttttcagtcctttacacacattttcattgctttgtttgcttttaatttattttttaaaaaatccatgaataggccaggcgtggtggctcacgcctgtaatcccagcactttgggaggccgaggcgggtggatcacgaggtcaggagatcgagaccatcctggccaacatggtgaaaccccatctctactaaaagtacaaaaattagctggatgtggtggtgtatgcctgtaatcccagctacttgggtggctgaggcaagagaatcgcttgaaccagggagtcggaggttgcagtgagccaagatcgtgccactgcactccagcctggtgacagagtgagactctgtctcaaaaagaaaatatatatatatatatatagatagatattttttcatggatatatatatatccatgagtaaatggaagttttgtcttttttttcccctggaaccctagccctgctaaaaaccttctaactttacctttctctatccttttctttatctacaactttttaatttttttaatcatctttaccattatgcttcatccttctgaactcaattgctttggataggcgagaagctgctttcaatttcatttccccatttttatctttagctaatgttctgtagcttgttttagatctgtgtctacatattatatgtatctctgtatgcatcaatatttgtatatatgcatgcatatatgtgtatgtatatttatgaatacatatacacaccatatacatacacttatgtatggtgtgtgcatatgtatgtgtagatatatgtacatacacactatagtggactggggagttagtatactgggaggagcatacatttagggtatgattcacatatttattttgtccttctcccattttccattaattaacaggattgactacagcaaagatgcccagtgttccactttcaagtgaccccttacctactcacaccactgcattctcacccgcaagcacctttgaaagagaaaatgacttctcagagaccacaacttctcttagtccagacaatacttccacccaagtatccccggactctttggataatgctagtgcttttaataccacaggttggcacacaaaagttgttaacttaaatatcagggaatgtcatttagaaaattctacagttatcagtacaacttgtctttaaattatttgcacagtttctaagtatgtgattttattcaagtgcagaaattgcaggaaattagtatctgtgaaatatagatcgactgaagtaattaatgcatgttgttagggagtggagagagaaaagaagggaagcaagatctccaaggacaatcaggaggggaaatttgttctagtatcctctgatctatacacactcgccatgattctcccgcttggcttcccgccacctggacagatgagaatttccctagttcagagattatcagttctactctccttggaaggtgtcttaaatgggagtcttcccatttctttgtttcactctagattctctttatccaaaaattgttgaagatagagaatgtattatttttaaatccactctgagaatcgacaacccaattttgttatttgagtttcttttaagagcatttgcatcattgaaaacatttttaattaaggttgtgagttctactggtaaattaaaggcaatgtagccatgttcccgggaaaaatcagattgatgcaagagatatttttgccaaggaggggcactatgctccttagaatactgatatatgtatatgctcatttaatgtttagcaataggtctgccagtgtattcagactcagatttaccatcagtagagtgttcatgcttttctgaaataatgtgttatgttgacttttttgtgggcaaacaggtttatagacatactctgataaaagatactaagctatttgaactgtttaacaatgccatttatcttcgtttgaaaaacaagcatatataataccatcacagaaattttgtttagggtacatcaaagtattttgagtaccttactgatgaagtttattggatatagtaagcagttaaataaatggtcagtgccttcctacagcaagtacaagactgtgtatttaatcttccatttgtttccctgtcaccatagcagagtagtaactaggacctgtctaaacactgtaaaaatttgaacacattgcccaaaatttttacaaaaggaatgcaaggatgaaggtgctgatgactaggtggaacatctcatgctattttattattttgtttattgcctgagtagtgtcacattgagttttccttttgaaggttctgtatttcacgtcacatgcacaaataaaaacatgcaacattcttttcattcccacatttttaaaacctaaaaccacttaagccataaatttacaggtagagcaaagtatgagaaaggtttaaagttgaatagattgaaaataaggatgaataattttaaaatactgatttgttctagcaaaataatactgatgttgaaattaccttgaaaagttcatgctttcaaataaaaacacactttcttttctagaaaataatcttttcatcaggtgatacttcaattatctattggaataaagtctatatgagttatttaatttatgattatgattgatttatactgctgaatgcagtcaatttttttcatttactgatataattgggggaaaatcctttaatctgcatttctaagaatattattacacactattcaaaattgttcatttttgaaaatggctacaatgaccatccatgtgcataacattaaatttaattatgtaattttattttataaagatagtttatgactatttcaaagcattttcaatatagatgggtatgtgtgtatatatatatttgtatatactgttaagtatatataaagtatatgtatgtgttgtgtgtatatattttaatcctatgtatacatacatatacatatatacatataggattaaagtatataaaatgtatactttatatgtacttaaaagacacacaatgaaaataccctttaaattctgttccttaaagatacctttttaaccattgttgtatatcctccaggctctcaacatatgattttgtgagtatgcaagagaccgtgtatgtaagcatggacatgtgagattgtttccacatgttttcaaacactagatattatcaaccttttaaaactctgccagtatgctagttagaaatatttcatgttgatttacatttaaaaaattgttcttaacactgaacactttttcatataccttttggcccttctgtatattaggtagatgtctgtcacatctcttgtccatttttaaatttcttcttttctttgtaatttgtaagagatactagtacattggaagattcctttcttattctccctacaaagaaatgtcccatctgtcagtttgtagagttgatggagaattcagaaagctcatagtgatgtgaaagtcaataaagccacctggaaacacgaattctctatggctgcatccagctcaggaaacctcccaaggctatgtaaatagaggactcaggtgcctgtcactttccagccaagcaaatttaaatactgacagacacattttaacagattcagttacttcacagtttggtaaactataatcgcaatttgctccttataacctcttagtaaattattcatctccagtgggggaagactgatgtaatgatctcactttcctaccttaggtgtttcatcagtacagacgcctcaccttcccacgcacgcagactcgcagacgccctctgctggaactgacacgcagacattcagcggctccgccgccaatgcaaaactcaaccctaccccaggcagcaatgctatctcaggtttgcgggtcctttagacttgtgcaaatatgaaaagtacatgacgactacctgtatttaagaatggtgtgaggaaatctaaccacttattcaatgtgcagctattgctagttgatgaatttggaatttcagtcactcttaggaatatgaaaccacagaacaaatgtccttttaacagagatgaaataatagtgagaattgtgagactacagcaaaaatctgctcaggaggaaagagttattcagaatagtctattttttatatatttcaggcaattaccattctacagggaaaactttttgttagaagtaagaaataatatgcataaatctttacttaaagactttgtaccaacaaacaaaagggtgaagagtgattcctattatcagtgaagggcagtgagaaattgtaaccacaatgaaactgttatttaaagaatgagaaaaaaagaaaggaatgggtttatttcccattcaaacattaagaatctttcaggatggcatctctgtgtttataacaacaatgcagaatatttcctcccttttcttttcaaaattagtgtccaaatcacttcttggtgtccttttatatgcaagaaaaacaagtatgtcttttgtcagatcacaaatccacacagtctcgtatataatttcagtgatctgagtgcttgaaagttaaagatataaatggtagacctatgtagctggtaggaacatggtcttgctttaggtaggaatcaaacacatcaaatagaataattattattttgcagtattaaaactgtgcccttggcataaaaatcattccaggcaatccacactctttaaacaagtgggagaagagccgccctcaccttcctcattccatctagtccagctgccatgggaaccacaataaaaatatttggagcttttagcaaacccacagatccagaaatagtggaggggcagaaactgtaaaacaacaaaaggggactgacccctggggctggttgtcacacagactagtctgctctgtcctgatcaaggaattcttcttctcaaagaagtggctaattccactgatgaaaaatctattaggattaatcaacctaattaaaattgtaaatgccgtccataaccaccactgagagtacctacataacaagggaaacgaagttttcaagtgaggaggagggaaggtaggaagtttcgggaggttgagagtggaagcctcaaaacagcttgggagcagggtctgctagagaggggagaacagatcaagtgagtgagaggagtgtggaaaagaaggtggaaaaaagctgatttcaaaactctgcagagggccagttctatgtctgaatgagttttttaaaggatgaataaatgagctttcctcactcttctacatattctgctggagccctcctctggggatccagagtggaaaacctcatgtttatgttgtttattctattctatggtttagttaaatttcgtggtttagtggcttttgaagactgagctgagaacccatgctcaattatttggaagatgcattttcaattctaatggaatgtatgtgtgaaattatagactgtactgcatttgtaattggtagacacctgcaagctcaaatcaaagccatgttcagaacgtgcatgcatgtatcactgcagaaatacagactctgcctgcaaatgtgagactaatctcacatcattgaactgatgaccccagggatcttgacagaaaataacccaacaagctcttgaatagagggcagctcatatttcttttgctttttccatggcaactagcatagtgctagtcatctagtaggaaccaaatgaatatacattgattgcctgtgctgtaattctggatgtgatgttgggcaaaggtgtaaaatacattaggtaatttgaagcctgaaaatggaaagttctaacctagtacaatgtgcagtttctttggctacaacactagattctataccaattagcaactatgtgattgaaaaataagagaatgatgccactgtaatgtggagtttgttggatttcaagccaatttgatttttcctggccagggaagcctgaattgtgaaagtagaattgtaaccttcagctggaaaggaagaaaaagaaaacctttgagctcatgctgtggcccaggcaggatcccattcagctctattttaagaaaattaaaactgagcacctgcacccagggatccctccccagagaggtgtgtgcctgcaaggctctcagcatgtatcaagttgcacttcctcctgtgccaaccttttacactcagagctctacctccatctacatggtctcagcaccactaagacagcaccagtctctactgctttgatgcattttttatattgcctaaggcagcctgcagcccagagtcttaggcttcttgggctgtccaaactatatatttttttaagttgtgctctgattatgaagctgcataggtttccagttgtctgcccctaaatgcatctttcccataagccctggtatttttggtacagttctgtagaatgcatgtgtcgtggtatagcagaagtgcttgaagatttgtttctctgccttatctttagtaattgtgtttatgttggctatctggctattgcccttgcgtgacagacacaagtgacagtgctgatggcccttctgattgcagatgtcccaggagagaggagtacagccagcacctttcctacagacccagtttccccattgacaaccaccctcagccttgcacaccacagctctgctgccttacctgcacgcacctccaacaccaccatcacagcgaacacctcaggtctgactatgctgctctagtagtgtcttcagttatagataatgaaatggaaactcaaaactttaatgtagctcttttattttgtgccagatattatttgtaggtttcccattttacaaatgttcacgtatcaacaccaaattatgcaaaagaaacttgccagtaagctttttctgggcatattttattttactattaatattataaaagtccatggcaaagaagaatcaataataggccttaatgtcatatagctctgggatcaaatccaatttcttcaacttcgtagctgattacagggcaaattactaatactttctgcatatcagatttgctttctgtaaaaatggacataataacactccttttttaattatgtcaaaataattaacgtgatgtctgaatatgtaaaaatctggtatgtaataaatattttaaaagagtaattgtgacgcttattagaatccaagtatggaaagccgtgaatgaaagggaaatgaatagtctgaggaagattgcatatcatcaactaagaattatatcaaggaatgaatagttttccctcaatttatacaatgtttagtttaaataacttgaaataaatctttgattcactttattattttaaaaacaagcgaatgtcaaatcaaacgaggactcctagagcaaagatgccaataggaaattatctttgctaaagagtttttctttcaccttttaatataacgaattaattagcttttattcttctattcattttcttgcagatgcctaccttaatgcctctgaaacaaccactctgagcccttctggaagcgctgtcatttcaaccacaacaataggtgatattaccctcagtcaggcagccacaccatccccatgtgcctggtgatgtgctctcacaagggccttccacccactctacctcgggctcctttctttaagttgcattaagtgtttgaatcctgagggtgatggaacagcaggaagatatttctctgcttagcagtgcaacagctgatgagatcaggatgtaattgttactgtcataattcatcagaaagcatgtgtgagaaacaaccacatctactagaactttttctcacaggggtttaggtcttagtaaggaaaagaacaagcccatcaaaggggctgtccattgcaagtggtgagcatcagacggctgatggcagagttcccgttaagcagtgagagggcgtggagataaaggaaagagaaactgaggaatggctgcagcaatggtggtatctgtgaatcagcaagtaagctgatcagagcttgcaagcccacaattctcctcaaattcttccaacccaaaatcaagatgagcagagatctcttagcttacacaaagcacatgttctcccaattattcaacttaaatgcctacactcacacaagatactgctaaatttgttgacagagcaatttgttaccctggatctagtagatgtgcaaagagcttacaaaagttaatctagagaatgaagcagtctttgcattttctctgacttttttttatgtaaatgaaaagtataaacttcgtactatgggggttataattatataaattaacattgagattaatcaaaatatgaagacctttaaaatatttttggctgtgtgaatcttcagccatgttgccataccgccaattagatgcgtacctaaaagtcttaatattgttaattgtatttattgggtatatttatgaaaaattttatagaattagctcattcctttataatgctttaagttttgaaatgaaaacctgtactaggcaaatccttcatattctgttaaatctaactagatagactttatgaagtagaagtattgtaaatcagctttcccaaaaatgacatggcagatattctaaagcaaaattttaataatttacattttttttctccattacagctactactccatctaagccaacatgtggtaagtttatttacttagaatcagcatacctcactttggaatagcactttaattacatctttctttattccaagctttcaggacccactagtaagctaaactcactggctctaatttctcaccgatgactagtctcaaattagtaaaaaattactagctacacatggacatagagttgggaatgatagacactgggaaatacaagagcgatgatggagggaggaagacaagggttgggaaactacctatattgggaactgtgcctacttgctgggcgtcgaattcaattttactgcaaacctcagcatcctgcaatatacctttgtaacaaacttgcacatataaccctggaatccaaaataaaagttgaaaactaagttttccagttagacaactttggtaaagccacttaatttaatttaggtatttgaaaaaaaaatggaataacagcaagtttgttggtgagggggagggggacaaggattcagtgtgatgataaatataaaatgtggataataccttcaaagcttatcaagaagaaaaatctctctttttctctctctttctgtcttgcttgttaggggctggctcaaagcagatacttgaaaacagtttgtctctctttttttttttctcattttcttccttgattctcagttgaagcaaagcggttcttcatggtcagggcttattcctccattcatttctaagtctaaccactggagtcactgccttcagtagctttccatacatttagtgtaaagagtggccttcatatgtctgtttaattaatatgatcttttgtaatccggttgtcattcatctctcctcccgcctcttgaatcattgcctccttatgttcttcacttaagtaatatggaaccactttcagttttcttttctttctttctttcattcgttagttctttctttcttttttttttttttttctcactctgttgcccgggctggagtgcagtggtacaatctcagcttactgcaacctctgcctcctgggttcaagtgattctcctgcctcagcctcccaagtagctgggactataggcacatgccaccgagcccagctgatttttgtatttttagtagagattgggattcaccatgttgcccacgctggtcttgaactcctgacctcaggtgatcaacctgactcggccttccaaaatgctaggattacaggcatgatccaccacgcctggcccacttacagatttgtaaacacatactgttccttcctgcctctgtggccactcctgctcttcctctacaattggaattctgctccaacctcatcccccaaaccccatgtctatttttctatttcctgctcatattttaaaacacaaactaagtcactttctctggaaatcctgtcctatacctccaaatggaacagatctctctctttctagtgccacattatttcctgcataatcttattttagaggtttgtatgtctcctgcaattcatgcttgtgtctgcctccacactggattatacatttctaaaagctgattatatctaacttgcctttgaattcctagtattggtgaccatgtcttacatatgacaagggcttaataatttttgttgaataaaaacaaatgaataaatttatatttgttgtaaagatatttttatcagtcagcagaaattgttgacactaaacaaaggtgctttggaggtatattatcaatcataattttacccaagttaaggaaagaatgagggcttctgatccctgagtaattaatgccccacatatatcaagaaacaggtggttaataactacgttttagaaaacaagaaaattataaagcaagaataaatttctcaaatgcatcatttatttgtgcatcaagtcaacaagtaactagtgagttcccattaatgatacatattatgcatactcctgaatttacagtgataataaaaatagcctagactttgctctcatggaagttccaagtccagctaggaagacagacacttatctggtaatcatccaaatataaatttacaagctgaggtccttgttagggcagtaaagcacagataattacgaaaaaaatgatatggaggcacctaatgtgttttttctttttcatgttttttggggatatttggttagttgatttgatattttggcatttgcattaatgtagttttatttattctggaaaaataacactcaatgttctattttcttttagatgaaaaatatgcaaacatcactgtggattacttatataacaaggaaactaaattatttacagcaaagctaaatgttaatgagaatgtggaatgtggaaacaatacttgcacaaacaatgaggtgcataaccttacagaatgtaaaaatgcgtctgtttccatatctcataattcatgtactgctcctgataagacattaatattagatgtgccaccaggtaaatatcaatttatttcttttaataaatttataaaaacagtacacttttgtgtgtggtgttctccagtggtcacaggagctagtctggtgagagaacagggctgagggaaaggaaattccttggaaacaagtgggtgaactttctgctgtcttaaccaagtaaaaatgatagagtcaaataagccttctgtttacatccattaatcaccacttctacttatttaacagggagatgtttatgtgcactaaatatagtttatcctgctaagtgattgtctgcaagctttctttattctcctctacttaaatgaagtattaattatatatgtacatatatttattcttttaagtacaaatttatctgaaatatattagggagaaacataaaggatttgatgtgtatgggaagaaccaaaatacattcataaaaaggaaggttatggtcatgttagtgagatcaagttggttttgtcagctaagctactgcttggaaagaggagggggtgacaggcgtcgggcagactctggggaagcatctcttagccaaatgcattctggaaaagggattccagagccgtgtaatttttttaaaaagtcatatcatttaataattcaagactattaataaatttgttaacatttaaatatgttaacatcaaatgtattttgaaaataaaatccatttaatttattcattttccctaaatattactgagataaattaccaattaaacacagaagatgacaatacttaaaaatgcatttcccaatagggaaactcccaatacactttataataatcattcaattaaaagtaagtaaagagtaaacaaaaaatttaagataaaaacaaaaatacaaaatggaatgagtgttttttaaaatgtgcgaaagctacaattttatcaatatgtttgcttgcatttcattttttaacgtggtataacttataaatgaaacactaccaaaatatatggtgctaaaaataataaagtaaataataaaagaaacaaatccctagagttattagacttttcccatagcaatctcaatccttgccaaattctatgtcattagcataatttcagtggctttaactgacatgttaggaatgaatgagggcttaggatacacattatgaaatactaatcaagtttatttctgtatcttcttgtcaggggttgaaaagtttcagttacatgattgtacacaagttgaaaaagcagatactactatttgtttaaaatggaaaaatattgaaacctttacttgtgatacacagaatattacctacagatttcagtgtggtaagaatataacattgaccagagaatttttttttgtggcacaatgttgttctagatattatttaatcttactctctgccctttctctcttcctccctgcctctcttgttctccctctgtttgtcttttttctttcttgtctttttcttggtctgtggtatatttagagtcaaataattaaattacctatacaattcaaacaaattcacaaaataaatgaatacttttcatgaaaaataaatatctaaaaattgaaagtcaattaatttacaataattttcttggcaattgttatacacaggcattgttgaagagatcatgaaagaagggtgttataaggaaatgataatacacaaactctgttatgaagtaaggaaaaaaaatacaggattgtatggttcaagagtttactttttccatcctgcatcaacaaaattcatacacaagttcaagaacacttaaataagaagaaagcagaaaaagaacagcaagtgcatctagggatatgtttggatttgaattgaggcaactaataattgagatagtatttttaaagtgtatttgaatttaatgaggtgaactctcccaccctttgacttaaagccatctgccaggccatagctggcatgacagacagatgtgctcaggtgtgcatgcgcatgcacgcatatccacagctacacacatagaggatggagcattgcgctgggtgtaatcatcacctaatcaccatagtatagattcatggccatcaggcaagcagacaaggaaaggaagagcaatcatgacagaccaatgataaaatgttctctctagacaatctattagatgaagactaggtgaggtgcaatttcaactttaagttgtatttgctatatacagattgggcatccctaatctgaaaatccagaatccaaaatgttctcagaatccagtactttttgagtgccaacatgatgcggctcaaacaagtgaaaaattttacacgtgacctaaagtgactggtcatagtcaaaatgcagaaacataacacagaatttagtcagcatccccagagaaaaataaatgacctcaagctatgtatatgaggtatatatgaaacataaatgaattttgcatttgaacttgtgtcctcttcccaatatattgtatcatctaaatgcaaatattccaaaatctgaaaaaaaaaactaaatccaaaacacttctggtgccaggaattttgaataagggaaactcagcctgtattttcataaaagttgaatgtaaaaattatttttagggttttttattattttggtaatttccacagatgtttcaatctgataaatattaaatagagaattataaatgtgaaattagaaaataaatgtgtgcgtgaaatattgcatcgatatattcattcgaaatatttctttatttcaggtaatatgatatttgataataaagaaattaaattagaaaaccttgaacccgaacatgagtataagtgtgactcagaaatactctataataaccacaagtttactaacgcaagtaaaattattaaaacagattttgggagtgagtatgttacttgcatttatatgtaaaattgcttctctcttcatgttcttataattatttgagaatcataggaaatgaattgtctttttgctgtttttgatactttttaagcatatgctttttatttcaatgaagcgcaatttatctatttttacttcttttgcttatgtttttggtgtcgtatatgaaagtccattgccaagtcatgcagatttatccatatgttttgttctaaaaattttatagcattggctcttaaatttagctctgttacccactttgagttaatatttgtatatggtgtgaggtaacagtctaatttcattttgttgcatatggccatctaatttttccagcgccatttgctgaaaatactatttattcccccactgaatagtcttgccattcttatcaaaaattagttgaccataatgatgggtttatttctgaactttcagttttattttattgatttatatgtcatacttacactgtcgattactgctgctttgtagtaaattttgaaactggaaactgtaagttcccccaaattgttacttttcctcaagattgtttagaatatctaagggaacttggaattctgtatgaattttaggatcaacttttcaatttttataaagaagccatctgggattctttcagggattgcattgaatctgtggataaatttgggaaatattgccatcttaaccatgttagtcttccagttcatgaacacaagatatctttccattaatttatgtcttctttaatttattttcaaaatgttttgtagttttcagtgcattagtgttataattcttctgttaaatttatttctagtttaagtttattcctggttataatgctgttgttttcttaatcacattttcaggtttgttactaatgtacaaaagtacaattgatttttctgtattgatcttgcagtctgtcacattactgaatttgtttattaatgataatattgagaaatttttgacaaaacttataaatgtaattctaaattttgttttgttttgattttgagacggagtctcgctctgttgcccaggctggagtgcagtggcgtgatctcggctcactgcaacctctgactcctgggttcaagcaattctcctgcctcggcctcccaagtagctgggactacaggtgcgtgccaccacgccctgctaattttctgtatttttagtagagatcaatctcctgacctcatgatccgcccaccttggcctcccaaagtgctggaattacaggcatgagccaccatgcccggcccgtgattctaagttttatgtaaaaaggatagttgaaggctaaagaggctgcctaaatccttgtctcctcatacttctccaaaataatatatagctacaagaacagcaaataaaactatgtaaaaactatatcctcagcataactagaaaattttaatgtatttttattagtaccacaattattacattctttataatcaatgcaacaaaatagaaatcccagaaaactatgttttatatttgaaaacagcacaaaatgttttcagtgggggaaaaatagtcttttcaactaatgatcctggtatctctgtagaaaaaaaatgaacatcagctctcacctctcaacaaacacaaaaattaattcaaaatggattccagacctaaatactaaagctataatttaaaaaattctaatcaaagacataggagaaaatgtgtagctttagcaaagatttcctagggcacaaaagcaagaaacataaaacttttttgatgaattggagtgcataaaaattgaatattcctgctctttggatgaggccactaaggaaataaaaaagcaataaatagtttgtaaaaaatcaaaattaattttttcaacaacagaagtttttccagaatatacagagagctctttcagctgcaaaataaggactaaaacagctcaattgaaaatggacaaacatttttaatatatacttcacaaaagaggatacacaggtggttaataagcacattaaatgatgctcagcatcattagttaactgagaaatacaaattaaaacaacactgagatgataatactatacatccattaaaatggctaaacttaagaatacggatactactaactattggtcaggatgtgcagccatgacccaggaatttcactccaggtatttaccaaagaggaaacatgacaaagcagatgcattcatagtagccaaaacctggaaacagcccaaatgtgtattcactgttgaatcctaggtaaaatgtggtgtatctttacaataactactgataattttttaaaattctaactatgacacatgcaactaagtgaatgaatcttcagaacattacattgagtgcaatatgttaggagtgaaaaagtacttactgtttgtttcattttatttacatgcaatgggtaaaaagacaaacttaatctgtagttaacagaaagttgatcagaaggtacgtgagtctggtcaaaggagctgagttgactgggaagtaccacagaaggacattttgggatcacagaaattttctttatcttgattgtggtgttggttatgtggatgtatacatttgttaaaaatgcattaaactgtatctcaaatgggtacattttaatgtaaattttacttcagacattttatttaaacatttatcagtttttctcagtttcaaatgactagttactggaagcaatgacaagtgctactcaatgactgctaaatttattggtgctatgaatgccagatttttagcacagcaaaatctacaaattccaggatttttaggtagtatctgggcaagaatatatatgaataatgtatatgaaaggaagagggggttcttagatatcttcaagtcagtggaatgcttaggtttcacagtgccaatctggtgtgacatttactttgttaaaggaatttactctaaaacaaattaaatgagcccagatgcatttctttaaattttattttgaattcatcatttgtcaaaatatggttatcaataatgcatgcttataatatgaagaatgctttatccatgtcttatttttcatattacataacattcttattcttttaacaggtccaggagagcctcagattattttttgtagaagtgaagctgcacatcaaggagtaattacctggaatccccctcaaagatcatttcataattttaccctctgttatataaaagagacaggtaatttgtgtagaatttaatttcatcagaaaagagaaatcaagaatttgaaagtactagaaatttttattgagccagtgagtcacaaagctctctgcttagagactgcataggcatagtatactccctgatcttagaattgcttccactcattcaaagctttccagccccagaaatgactaaaatccagaacattctaaatatttgcttgtccttcttggtcttagtttaaatctttgtgctccaaagcctagagacagaaaacctctggatgacaacactcatttctgtcttgcaagtattatgtaagtgatttgactcactttgaactcatcattcagcctcctaaacaaaccaacaaacaagcaaaccccttgtaaaacttgtttcagctaataatacagacaaaatgttgggtgaataaaaatgaacatgggcccatgtagccgctggggccagtttggtgtaatcttgggagcatagttctaagtttagaattagacttctgcagaagtaatgcaattaaaaaaaaaaagaagaagaaagaaatgtgctatgactagttcactcatgaaatgttcaaatgagatgctatttaagagaacaaatatcttctggacaatttaaagtatctaaattgtttgtagaaagtaacatcagtggagtatctcagagcagcctcaatgcctgggatagccctttctctattcttttatccataggttaaaataggaatgaagtgaacctcatagaattctgtcactctgtgctgtggggaaggaaccagacatacacttcaaaacttgaaaagtgaaaggctatttttcttcattatgttattttatattttaatggccttttcttgctagtgtctttaggtcttaataatcagactactaaagcaaagttaaatatgcatgtagttttcaaattaacattcaaaggccaaggaaaataaatatatactatatatttgaggttatgataaatttaaaagttaagtctatgtggaaggaaaaatggaaattccaggaagataaaacagcagaggtactgtctgcctcattggacacctcttttacaaacactttgtgtagcttctatgggaacacattgttcattttttttttctcttctctgaatcttctattcactatccctttctgcattcctcaatgtctacactctctctactagagagtattgtcgatgtcagagtatatggtagacattttatgcatttatggctcttttatatttttacagtttttttaaactgtatttccactgtatttgcataattagggtaaaaaggatgtaatgagttagtagcaactcattacagcaactagcatgggtccttcttattgggcaactaaatagtgttacccaaatttaacagctgtccacatagaacacttaaacgggattgaatggctgagaaggggaggctagctatcaggctgtgtgttttcttttctccaaagctgccgattggtgactgaatgcagctttggaccatgccctgacactgcataaagggctctttggagccagctctactctaaacagcgtgctccgcttttgttttctccttcatctcaaacatatacctgtctcctctcccatgttacctaaggcaaagagagttgataggattatagtatcgttaaggcaacttaacttttctcaccattttaaataaaattactattaaaaatccacaggaagaaagtctatgaaatttgcagtttactttttaatcagatattaaatttcacttcattacttcacaatttaattttttcagtgtctctaaaagagagggattaaaagaggagaaaaaatgcaattgacattaatttagttttattggtttagcaggtttttttaattatgtattatttaaagattttatcaactattttaataactcagtggagatgtgcatacatatcttcatagttcatatgatgaaactgaggttaacagaaaatgtgatagatgttcaagttcagtagcttgatctgtttcctttctgctcttggttttgtttgtttgtttgtttgagagggagtctccctctgtcgcccaggctggagtgcagtcatgcgatctcggctcactgcaagctccgcctcccaggttcacgccattctcccgcctcagcctccctagtagctgggactacaggcgcccgccaccacgcccggctaatttttttgtatttttagtagagacggggtttcactgtgttagccaggatagtctggatctcctgatctcgtgtgatccgatccgcccgcctcggcctcccaaagtgtgtttgtttatttttcctcacatttttagcttaagatattttggagaactgcagttttatctcgttaacttaatgatggcaagtgacagtgaagcttcttggtaattggggaattggggaagagatcttttgtgctttattggatttaaaggattatttttcaaaagttactgaaagcaataggcacctttcaagaccaccatgatgttgctggaaattattttgtgtaatgccttttatttttttaagaaaaaaaaaacagaacaaattgcttaatctctctgtggctcagttttgtcatctgtaaaatcagatgatagtgagtaccaactaatagttgcagtgatggttaaattaattatttcatgtataccccttgaaacagtgcttggcacatacagtgagttattatttttaaaaatcgttattgatattattattactgttgctgctatccagaaacatgttgccactctaatcatcctctttcctgatgtcacttggctactcaaaaatagcagcagctggtgatttttttacttaacaagtgctaagtcttctgcctgagtgtgaaaacacacttagacactgtcctacctctcatatgcctccccagccagagctgttgtcctgatcaggtttgtcactaaactcaaaaacattccttcttccgtttgtaatattttcttttctcccttacatgtattcagttccacttacctttcaatgaacagctgaattccacttccggcatgaaactccctcattctcacagctcccgttaattactgtagtgtccaaattactatgatagaatcaacccaatgactgatgatcaaatggattctgcatctaacattcaaaacagtagctaataccgatgttcaaagtttggaggttacatatcagaaaaggttttctaaaaaagaatcattctgaaacatgcaactcaagacttacagtatacactgggggctgtgttttctcagaaacaaaagagatcgtcttcacaaatgaatctgaacttattaaatattttatgtaccaaattaatgatataaaaccataatttttcaatatttaattttaccaatgataattgagtttgttcaatacactggctgataattgtaggtacttttgagtatcaaggatgtacttatttttcaatcactcaatagtttggagttcacttggaacaatgtgatgtagagaccaaattaattaggtacgtggtagtactgacttttaacgacttactaattttttttcacatttttcctcagaaaaagattgcctcaatctggataaaaacctgatcaaatatgatttgcaaaatttaaaaccttatacgaaatatgttttatcattacatgcctacatcattgcaaaagtgcaacgtaatggaagtgctgcaatgtgtcatttcacaactaaaagtgctcgtaagttatatgttttaatgcttctttccataaatggtaaaaagcaaggtatgaactttttagcctacaatatttctatctttattctagcaagcacatttacctggcacatttgttaacatctagggcttataaacacgtaaaatctaaaagtttaaaaaccgttatcctggattctctctcttcttcagatatagtcatagaattttaaggacaaagcataaaagcatcttaattggcatcagtttgtgcaatttcatgcagttaagtacttaaccaacttagattaaaacattcactgtttgctgttgtctttactatctggaaatattaattgtaatcagaaacctaacaatgtctcataaagcattagcctactaacctctgttcatctgataaaacatttcataaaatgtaatattttattagcattttcttctcttcgttaccctcaactacttactattctattttatgtcacattatccatttaaggtttcctttcaatggcatttggctcttgccactagtataatctctccatagtttccaggcccaaagttagatctgcttctggggcacatgttaacctccatcgaggacagggaagaagaaatgccgtgttttaaggcagcatctatagctccagagaccctaacgggcactagacttgtgaagaaatattgtgctatttggggctgaatataagacacttttaaggtcatttaggttttggtttgaaaagttctggtcctggagctctatgcttttgttgttttcctgagtttctgtatcacagaaaaagaagacaatttgtttctgttcctgaagaacccatctaggtgtttaccaggataacattagcactccgggaaagaagggtctagattgtgtaataggacttggaggtttcccaatcaacaacatttttcctctcctctccccaaacttccccctcttccccactcccttccctttttctctattctctaattctacacagtctccttcagggattgcaataactctcatggcttcatgtacaacctatatgctaatacttactgaataaatgagtgatttattcttcagggttttgatattgttttttaatttatgtactatcataacttccttatttataacccccaagctaacacttaaaatactttatactatatccaagtattgtcaagtaatttacatatgcatctattaaattattaataacaaatctttcttcattttgatagctccaagccaggtctggaacatgactgtctccatgacatcagataatagtatgcatgtcaagtgtaggcctcccagggaccgtaatggcccccatgaacgttaccatttggaagttgaagctggaaatactctggttagaaatgagtcgcataagaattgcgatttccgtgtaaaagatcttcaatattcaacagactacacttttaaggtaaaagtatgctctctacattactatagtaccaactacattataatgattgattcatagtacttaaataactttaagaccactgctcacatgagattgagaagctctgatgtgtaatggaatcacacttaaagagtctcaaatatttgactctaaaatttttattcctatagctcaagtcagtggtttaaagcaaatgtttcattggaatattttagaacttcaatatgacttaattatagctaaattattgcttctgtgttaagaagcacaacactttatgcacaacagattattactttaccaaatctaccttttctttactttggctttttatctttattaatgtggaatttttcaattgcaaaatttcacaggtaccttgaggttaggaaatatttgaaataaacactagacaatactagtgagcatacagaatttaaaacactcattatctcactgtctactgatcgtattttgtacatgtaacttcataatatacacatttatatgcacttaacacgtattatcaacattctgagtacacagttttcaaaatacagttttaaaactgtatttttaatatatcactatatcacacacacctttctatgttaaatatttaactactatgtagtttttaatgcctgtataatattctatgtatggctttatcacattctattaactataactatgttggtctctaatataaacaacattccgataacacacttattggtaaagcaaaatttttgaatgtctttaataatttatgtttcataaattcctaaaaatgcatttattgggtcaaaatgtattttgaggctttttggatatgtaactttttttttctataaaatttaccaaattgccctggtgtatcagtgtatgaaatgactgcttcttgagaggctcaccaacactgaatacgcctttctttttctttatttggtggttgaaatatggtattgatatctttcttttaatgaagtttctttacttattgttctttgtgttattctttgcctcttttatccagttttctccggagaaatgccttgaatattaatgatattaaactctttgtcacatgcgtaaaaatgttatcagtttataatttgccttttagttttcttcacagcactttgtcttacataattcccctttttatttttaaacaaatgtatctgtcacttttattcctgttaaatagaaatttccatagttaattttttaatatgatgttgacaaacggcctcatattctttttttgttttgttttgttttgttttgtttgtttgttttgttgttgttttttgttttgagagggagtcctgctctgtcacccaggctggagtgtggtggcgtgatctcggctcactgcaacctccgcctcccgggttcaaatgattctcctgcctcagcctcctgagtagctgggattacaggcacctgccaccacacctggcaaatttttgtattttcagtagagataggttttcaccatgttggccaggctggtctggaactcctgacctcaagtaatccgcctgcctcagcctcccaaattgttgggattacaggtgtgagccaccgtgcccggcccatattctttatcacttaaagaagtgttttcatatttataaactttttgattttgtttttgaactggaaatgtcggttggattttatcgatttttagggcattatgatagatgatgccatagttgtgatgccctggtgtgattagtttaaatgatgcaaaaccattgtcacattctaagagaaaaacccctgctctgtcattgtgtgttattctctcagagtattattgaaatcaacagcctattattgtctttattagtagatattcaaaaaggagatcattcagtgagtagagacggtgttggcataggcgttggatgacatcattcttattaaatttggtataaaggttacactgatctgataaaacacattgcttatatgttcctgtttttctgtatcatataactttttaaaaaaattttattattattttttgagaaagagtctcgctttgtcacccaggctggagtgaagtggcgtgatctcggctcctgcaacctccgcctcccaggttcaagcgattctcctgcctcagcctcccaagaagctgggattacaggcatgcaccaccatgcctggctaatttttgtatttttagtagagacgggggttcaccatgttggccaggctggcctagaactcctgatctcaagtgatctgcccaccttacctcccaaagtgctgggattacaggcgtgagctactgtgccaggcctatattatataactttaaatagtataggagtgatttgttcctgaaaaatttgtcttcattcctttcatgcagagaaattctttaagactcatttatatcttctttcaataggattagtcttttcagatattttactctttttgagtgagtgtgctatatatattttttcaaagaatagtcaacctaaaagaaatattttcttattgtcacatcattgtgtattatacttcattccccactgcttctccagtgcccattaagctccaggtgcactggtttctctataatttctcagaggcacctaggtgttactctttttagccacctccctccacgctcttcccacttcctagaatatgcctctcccactcttcaaatcgtataagttactatggaaaaatataggtgtacatcatattaaaatacaaccttaacgttcaaagtaggagataattattcagtttcgaattctcttcccccaatcttcaaaagatggtttttgttttctttattatacttgccataccttcttattatgcttatttctgtctccactatcatgttttgtgttcactccttcatgagagagcagtcatttcagctttttcaccattgtgatctctggttaataaattaatgaagttgatttattagtattacttttccatagatttattttgatgctcttcaggtggctttcggattaaaagtgttttcttccttgtaattttttttcatttttataaactaaagggaaaaaaaaggctatggattgtactttggtaaaattttgactgtaacccatgtctatatcgtttgtcactaatttctgaaggccttcacatgaaatgtaatcaatgattcttaaagtaaaacattttgattattgatgatttctaatgagtctgtagttataatttggaagagtttttaatatatccattatttaagagagtttttctacatttctggtgctttaatttcttattgctactaattattagctgataaaagttaattggcttttacaatttctgccttttaggatttgtagaataatttttacagctctatgtgtgatatttatgaatattctgtgaatattgggtaaattatatattctccataggataaaagcttagatatatatttgtcagatttattatatttattattattctcttttaatgatattattcaaatatattttacttaaatttttttggtcaaggattcttactgctcttttgctcttttcattttccctgtatatgtaaattgttttcacttcatttgtattacattttatgagacacaggtgtttatgcattatgcctatatagtaaattttactatatatccatttgcccttaaaaaaatgtatgtgcattttatgcataattctagtaaacagcttatggttgaatttccttttttaattaaatattagcctattaatagggaattttaactttatgaatattttgatgtattggattttatttcttcatccagtttcattattttaaataattatttaataattgtttaataactataaatatttttattgctaagtgagataagatatctttttgattgtcttttcaaatatatttgacaacatactgacataaccttgaagtttaaagcaaatcagcatacttttattgtatgcatggtatgaaagataatataaatgttttacattgtgatatataatatatatatatatataaattcacattagcaaactaattattttattttttgttactgaaattcaggcctattttcacaatggagactatcctggagaaccctttattttacatcattcaacatcttgtaagttatcactgggctatttattatatatattaagatatatattaatgcttataaagctatattattttacacttataatcacatttgattgttaaatgcttaaataatatctcttccgtaaatgtaatatttttaattgtcagtaaaaccatacatatatatgtaaatatatttaaatacaatatcttaaattcaagttaggagattcaattattaaaggtttgttgaattcataagaggatttatatacccaaactattaaattatgtttatgtttatgaaatatcgtcatgttagtaacatttttcgtgtactattttagattatctattttattctgtctcttcagcatatgtttagcagaagtgggccttagatacaagtctgtcttgatttacttaatggaagctaatataagcactccctaataacaatatacttatgtaaatatttatcactgatatttaaaatattttcatcaaagtaaaggtgtacatgaaaaattacttagaattaaatttcattataataatgaaaataacagctgcatgttacattccccacccacaattctgtttgccaggcaaccacttttaaccatttctatttttgggtctccttatagtttccttcatatatatatatatatatataaacaatattgtatactgctctttctagagttactaacattaccaattgatctgagcctatggaggaaggagacctagtactctactttgggctttctctactggttaacattgtaaatagaattatttaagcctgtatgtactttgttgtcagcaacttctaggtctttctatctttgccacttctagttcttcctctcttacatatgttacatatgcacatatgcatgtgcacaatcactggtatgaatgcaaagtcaaaagagaaaatataaaaacagcttattttccaaactgctttactaagccctctgcaaagttttagttctttctgctcagatttatgaaataaaaactccctgtgttaaatgtcaaaaaagtccagcaagatagctttgattttatttccacattacctttttcttttataatatctttataataaaaatgacttcattgactctttcctattaaattgtaaataatttatagcagtcatagactcagctgaacattcacactcacatcttaataggccagatctgaaacatttcacctggaaagacacagaacaaaaagcacagcatgctagcaagggagcctggcagtgggaatccttgcagcgggaatccttgcagcagtgcacacagcaatccagctacttttcttatgacactctcaaagacaactgagatatgagagaatgagaccacatgtgtaggtgtaggagctgcattccaaaaggaatcagtatctcttatactatttccatgggcatagcttccagacatgccaacaggggtgtgctcagttatgagcgggcactgcactcagggaaacccaaagctggtacttcccatgaggacaatagagttcacatatagcactccctgttcaggtgtagtttagcaatcaagggtcattttgccattagcaatgttgtctggtaaccagctaatattccacttttatcaggtttccaggtcaacggagccaaaaaattagccctcatctttttccacaaaggagacaacattgtattcactctctgctcacaatatcattatcctaagagataaataatatagtttcttttaaaatagtgatatctgttccaggaaaggacttgggctgtgaattgctagggtacagctactagggatgtgttgttgggtttccccggcataatattccaccacctgtactttgacatcattgtcaattgaactcctggggaccctttcttcttgctctgatctggactctcacatgccatcttgaaatattcccccatcagttttctggtttagatttgctgtatcacacatagttatttttttttctgtctgagttcactgatatatgttctctagtgtaagaaaaataattctaattctcccatacaaaaaaaatttttattctgctctggcacttgttcagtgtatcgacttggtataaaattctaagttaaaaattttagaatttaaaaattatttctgtcttattttcctgaatccaattttactttctaattccatcctgattctctctctctctctctctctctctctttttttggtctgttcccaagttttcctcccctggaaatgctaggtttctgtctttattcttggtcttacctgaattttttgtttgttttgttttgtttgtttttgtttttgtttttagagggagtttcgctcttgttgcccaggctggagtgcagtggcataatctcggctcactgcaacttctgcctcctgggttcaagtgattctcctgcttcagcttcctgagtagctgggattacaggcaggcaccaccacacctggctaatttttgtatttttagtagagaagggatttcaccatgttggttaggctagtcttgaactcttgatctcaaatgatccacctgccttggcctcccaaagtgctgggattacaggtgtgatccactgtgcctggccctgaatctttttcattcattttttctggatgctattgacctttgtaacctgaagatttatatatctgagaattctttgctccattttcttcccatagtctttggttgagtctattagtcataaaactcataagttgacttattattttggcattcccctttggtgttgatgttttccttaaaagcttggttcttattggtagtctagtcatagtcacagtgagacaacaggaaaggttgattagatgttctgtggtccttagaagatcttggtgactgaggagatttcctatgatattgctgatttatttttttctgatatcattcattatcaccaaaaactaattaatccccagaaattaatctccagaattaccctactccttgttgtgtggtaaagtgtgaaaaagtggttcttctcacagtaggacaggaagataggtgtccaactattgcatatgtggacaattacattgtcctcctaattttagtcctgtgcctcatcccttccctgtactgagcctgactttattctcagtctctcactgctttcatttaattttccttttgtcttctcctccctggtagtattttttcaagaagatattttttgttattgttgttgttgttgttattgtttttgtaaatagacatttgacttccatgttctgacccatgattcacatttactgcatatgtcactttcaaacctgagactcaggcattctgagtaaatggaatctattcctttgatttaggctgtggcctcctttcttttgttttctaccttctacaacttgttgaaattgctctacttctaatttcccttctctcattttcactgtcattataaatctatggcattttcagttttttaatattagcagggttcctggaaagaagggggaaacacatgtgtgcttagaatgcaagctttatctgaagacttggctattttattaagtttgttgagaaaagtctgatgctgcttaatatttttgtagaacttaatctaattattatggattggaatgctaacttacagtcatttgcagtttcttgcaaaatcttacttcagagtattctagaagttagatgttgcctctgatgaggtttttattcacaaaatctggaaacaatcatgctgattgatatatgtatactagtaatcactggtatggattgacaatttcagtgaaaggaatttcagatagagataagacaaggaacactttgggtcattttaggagcctattgcaataagaacttcttccctaaaaatgttcactgcaatccacctatatattcacattcatgtatcccatccatttttatatatgccggcagtataaatacccctttaaaggagataaaattatttctattttatatatgaggaaactcaagtttggataatttaatctatttgccctatgagtcaaagaaatgacagagcctgaattcaagctcaggtcttacagtctgtatctgaaattactttcaatattcctgtttgtatgagtttccagttacagaaattttgatcatgagatgaactgtttctggcagctgtttgcttgatagagtcatttccttctttccagttgtagaaaaactgtctcatgctcaaggcctccacttgccatacagaaaatacatcccctctacttccttatcaccctacttatttttttcagagtatatgaaaaaatgcataattatttcatttgttcacttacctttcttttttcttttcttttctttcctttttttttttttcttgacagagtcttgctctgtcgtccaggttggagtacagtggtgcaatcttggctcactgcaacctctgcctcctcggttcaagtgattctcatcccttagcctcccaagtagttggcattacagacacacaccatgcctggctaattttttgtatatttagtagagatgaggtttcaccatgttggccaggctgctctcaaactcctggcctcaagtgatccacacgcctcggcctcccaaagtgctggggttacaggggtaagccactgcgcctgtctgttcagttacctttctagtgtctgtttcccccaaagagaatgcaaatttcctgaaaactaatattatctctgccttatattctatagcatttccacggactgtcttcctttttatcttcacagcccttatatcttctcacctacatgaccatttacttatttcttctgttcattattaattatctatttttcttcactagagagtaagttccatgaggacaggacccttgtttttctttatgtagatatcctaagtacctagagctgagtttggcagatgaccaaaagccaaaaatattttttttgtgaatagtgaataattagtacttactacttcccagccaccgtgctacgtgtttactgtgaatcaacacctttagccacattttaggattttgggaaaggagggacaaagataataaggaatctggccaagttcccaactaagaagtggtagagctaggattggaagctaagcagtcgggctctggagctgaggctcttaagtcaccgcattattttgctgcattttcactacataagaaaaggtgaatatactggagatatttccaacacaccctctcttctatgccctttccctaggaaagggcaggatttcacattaaacttagtgaatatttaagtcagggtaagtcttatcctaactatagaatgaaaccatttttgtctcttagtgaatggattttacacctcagtgaacaggtaagagggtttatctttgtgaagtagaagtctttctcatccccttaagaggctacccacttctgcatataaagttaaactatatgagtttgtctccaaaatttataataactggattacctccttgatcccttcaaaatgaagtgtctgataaaaaaagagaattaaatttaaatgtgtcttatgaaagaacattatttaatcaaaagaaagataattattcttctattcttactctccttaaatataaaatgttttcattggttcagaacaatatagccaaaatcacagaattagaaatttattgtatttgaccttattctaaaatgtttattttttaaaacctcacaataaatttaaaaatattaaaatataaatactttggaggtgattattcaaccagtctagcaagttatttgacaatcgttctctgaatgtattatttttcatttctagataattctaaggcactgatagcatttctggcatttctgattattgtgacatcaatagccctgcttgttgttctctacaaaatctatgatctacataagaaaagatcctggtaagagttgattttaaatttttaaataataatggtattagtaatggtgcaaacgcatatccatatggcagtgatggaaccagttaaatgaaatatgtgaactagagagaagacagcatacagcccacttcatgacacaacttttaatcaaaaacttttagtatggttttattggtttgaattaaacattaatattattttctaaatttactaataatgttgtggacttgtttaataataaccagtgaaaagaatgtgtgtggtttttagtacaaagtgggtcagagggatctaggagtgtcaaaagaaaaagaaaggagggagatgtctggggaagttaatgtgtttctttggtcagaaacaaccacatcttatgaaaaacagaagatttaaaataaaatcatttagctacttatgtgagtttagcagacaattcttggttgttttctttcctccctcaccctcctctctcctctctgactctgctttctcccatccttctgtcctccctctgctcaaggctcttcctcccttccctcctttcctcttctcctctcctctcttccccttttcttatccctgacttccttcctttgttccttcaatatattcattaaatataagtaaaataccaattgaattttgtgcttcttgagaatatagaaacttatttttcctattttcacagcaatttagatgaacagcaggagcttgttgaaaggggtaagtatgtatatttttgctgatgactattccttcccctgcatttgaatccattcattttatttatttatttatttatatttattttaagacagagtctcattctgtctcccaggctgaagtgtggtggtgcaatctctgcttattgcagcctccgcctccctgttgaagcaattctcatgtgcctcagcttcccaagtatctgggattacagacacacatcaccaggcccagctaatttttgtatttttagtagagatgggatatcaccatgctgcccaagctggtcttgaactgctggtctcaagtaatccacccaccttggcctcccaaagtgctgggattataggcatgaaccattgcgcccgtccccattcattttaaataagaattgggcatttttagtttaacttggacttttgttgatacagtgataaaacttaaattcctttactcactcagcacctgtgaagttcccagtgtacgccaagcattgtgccaggtactgagagtactacagtgacaggcacagactctgcccttaaagggtttagaatctaatagaggaaagcagatatctcaacaaatatgacggtaatttgatacatgccctagtagttgaatgtgtatagttctatagatatatggaagatagaaaactgtgtgcaagggcagaaatctggtctgttaagattgtggggaaccaatggacaaatgagggagtggtggagggacgagtggatggaagtcacagagatggggagatgggatgtctcctcaagtccctgccagggtggaatggtggctgctcccactaaagacacatttatggattggacaaagaacagcaatttgacttgggagaagaaaacacatttgtttatcttttttttcaacatttatattctttaattttttaaaaatgtgatttctgatccagtaaaaggggacaaagtttcagaaattgaacctttgtttacaataaagaaatgtacttgctttctcatgcttaagacaggaataatttcagaactcctttgtctgtgttaatctgtgttggaagtgtttccctctggtaatagcaggtaccaggtctctatgcagaaactttagggctgaatctttggagctccttaaaaggctttatttttctttgcagaatgtaacactatctgatcccttattacatatttattcatttggtcattgactatcctctcctaactagaatgtaagctttgtgaaagcgtggaggcttttttcttattcactgctttatgcccagtaccaaagtgagtacctaggatttgataaatattagtgaataaataacactgacatagggtatcgtgaggattcattttgataggctgagggaggaatgaagagtacaatcagtaataaacacctgagcagaacaggaaaatccatctcaaggagttaaggtggacttggaaagtgtcaatgaaatattttatctcaaaattggtaccgattgcaccttggaacgcagtagaatttactcactcagaccccatgaaaccctgaatgtggccctcagttcagaatgaatgaataccaggcattcccaacaacctaaagaaacaattgcacatagccagtttgagagctgtgattgtatagaaagtttccatgggcaataagataaatgggtcaccctcatggataacttctttctttatctgataaactggtaaaattaatatgattactgaaagaaacactatcagtagtacatggaagagtaggagaaacataattttacatatgcgacagcttaaattctcttacctttctaaagctgttggttttcaagttccatatgcaattgtagctttttatggttagtatactttttaatcttcagtaagttatttcacaaacatggtatataatgtgtttcatatacttgaagcataacaaattaatacaacttgtttcaccatttagtgtaaacagatgatcaaattaagctgagtcatgggtataagggtattaatcatattgtcttatttcatttgcatgtttacagtatttcacaagttgaaaatgaaaatacaaagaaaaataatattgtattataaataaataattatagtaattgctataaaatgcatatagtcaaacgtgaatgtccttataatggtgatgtttggtctgggatcccttctcttaagcatagaaaatggggaagaacattctagtagagagaacaatataaagcccagaagagatctgaagtacaagattgaaaagtcattgatttataggtaaatgtttgtatgtgagtgagatttctcagatgaaatgtgtacgaggaggaaagaagctaaaggattgagtacacggtgtaaatttaatgaaatgtgtatgcccacctgaaagacacatgtaactagtattgaatctttaatatgtttccagatgatgaaaaacaactgatgaatgtggagccaatccatgcagatattttgttggaaacttataagaggaagattgctgatgaaggaagactttttctggctgaatttcaggtgtgtgttgcttttgttatatgatgataaattcgacatcaagacagttccactttaagtgtatttatattgccatttgcctttataatttatcccacttgatattgcaacataagcaaagtagatattattagcagatctctatgaaccagaagagagactcatagaggttgacgggattatagtgtagagctagtaaatattttaatgtagtgctttattgtattatgaagttgtgtcacaaaatgtatttggctgattttgtagttgtactctagatactcatccaagtatctgtttttaaatgaatttgatagtgacacaacaactaatcctaaatttgtccccactcaagagatttgttctgaaagttgtcaatcattaatttgtaagaaaaaagttttttttttaacataattcctgatcttaattttgattactctaagcaaatttttttatcaatatgaagaaaatattttacaggatatctcatttactcaaaacggtcattggtaagggggaaattatttttcctgaatctgctgtgatccaagaaatcgttgtttctttcagagcatcccgcgggtgttcagcaagtttcctataaaggaagctcgaaagccctttaaccagaataaaaaccgttatgttgacattcttccttgtgagtatttattgagtgctgaattcccatatattaggctacttgattattcactatttcacttgtttatttttcttttccttaaacagatgattataaccgtgttgaactctctgagataaacggagatgcagggtcaaactacataaatgccagctatattgatgtgagtaaaaatttgcatttttcttatacctacatatttcattcagctccttgtttgtcttggtaaaattttagaaatattattaaaaatattttgaagtgagcccatatgtcactgatataaacaaaaaattatcaatattagcaaggatagttatttattatgtgactattggtattaggtataacatagaattttcctctacaaacaaaattatattaagaattaatttaatatactctggtgtctattatgtgctagatattagactaaatattctatgcatatatttctcacaagaagtccacatttgcctcagccatgtgccgtataggtgaggactgggaggctcagtttagttaattaccttgttgttgttcacacaattggtaaatatttgagttgaaattcaaccagagtctgactgactccaaaatgttatgctttaatttcatcacactaaatttcagcagacattcctcatcaacatgatcatctatccattggatttatgcagaaatgtaaatgtccgtacgtggttaatttatttaaaatattttaaaatttaatttattatacaaatgttaattaatgtattacataggttaaataattttaaacagtataaaaatatatacagactgaaaaaattctttttgtctccccaaatctgccattttcccagtgtcctcacctaccagaaataactatattttctattcaaatatatatggtaattatggtatcaggttacttatgtttccccaatggaacttagagctccctgaaagcatgtgtcttctgcttttagataggtgattgacatattgtagctattcaataaatacttattaaataaatgaatgtatgcgcaataatgtgtcatgagatagaagtttcaggaagttacttaaattaatgttgaattcttgtgacccatgtttcaaatttaatccaatggcaaaggtcatccctctctgaagagctcctttagttactgaggtgaatttaggagtctgagataattctggaagaagccagtataatattttatctgcctctgtactcctttatcttggtaacaggagcagagaaagcagacatagtaggtaatgaaatgaaagttattatatctcttatctgaaatggcaaagaagtctagggaatcatattccagcagaagttaagaggtgaaaatgcgggtaaaatctaagaatgatttgtttaaagaaattgagtaaaaatcccaaaagtaactacatggctggtgagcttgtttaaatagtggtagatgatcctataagagttggcaggatataaaatgttgaaatgtctagagcactcttgtaaattaccacagcatcgcagatgaagatgaaacctagtattaaaattgtttgaagtttacagcaaagatacatgaaagtcatgaatattctttgcaaatgctaacatgtttagcacaattaaatgcctgaccaccaattaataagattcccttaatactttgaaactgcccagagaaattcacaatcacaaaatgatggatctgaagcaattcctctaactcacaatttttcctgttaatgagtaattgaatgttcagcaaatgacatatctctgcatgtgttttcaatagggtttcaaagaacccaggaaatacattgctgcacaaggtaatttctttgataatccaatattctttttgaaaaatttttatagcacttttaagaaaatttttcttatcagcttttatttgtttacctcctaggtcccagggatgaaactgttgatgatttctggaggatgatttgggaacagaaagccacagttattgtcatggtcactcgatgtgaagaaggaaacagggtaagaaccaagaagattcatagtgtgggtcttggggttaggaaaacaaggtgttgaatggcattttgaaaagccacatgtatctgcctgatgactaaaacagagagttctctattttaatcagtgttaacatttaatttaaaattttcatacatgtagaaaactaaaacttttaacatacaaatatatgtctatatgcataaaatttcaatgcttctgattaattgctagactcttaacttgattcctgtttctttgcagtattgttataagttcagtatatttcactgttttaacttcacaagaccttaatactcgaaacaaaactgaccttgggcagataggtggtgagtcatgtaatgtgactttaggaataaaagcctctctgtccccctacctaaaattaaccacaagcaatcatatcctttttgctgacaactgattatgtcctctcttaacatgcatctaagcctggaaagatcatcctgctaaaaagtatgaaggaaattcttcaggacacattagtgggaaatagaatatatttcaagcatcacagcttaaggtttatatgtgcttaaactatacaactgttttgagaatttcaaatgagtataggttttgttttcactgtttaaagaaagtttgataaaaaattggcttaaattaaaaattaaaatacttaataattttttaaaatgtagaacaagtgtgcagaatactggccgtcaatggaagagggcactcgggcttttggagatgttgttgtaaagatcaaccagcacaaaagatgtccagattacatcattcagaaattgaacattgtaaatgtgagtttgctttttacataatttttgttttgatacttttttataaaaatataattatggaatattaaaagtgagaaaataaaatatatcaggaaaaattatttttgataacctttaggatgaaagctgtggttagaacaatgacaaaaatcaatagggtcaaatttaagtcactggtcaagacgtttttgtccaactcaaatcgaaagaattatactgtattaattaattatctgttttaattattaaaaaaagagggaaggtccattaaatgtgttgaaaatataatcaaattattaaaagaataagcaatttgtcttcattgtcagtgagttcctacttttatgaaaaaaaattatattatttccataagagaaatgacagcattagagaacactgtaagaagtataaagttctaactatgcagcagagatagaatgtttagttcagaaaataaggaggtcattgtggccttagataatagttaaaatagagatcgtcatgcatgttatataattccattatatgaaaaatccacaataggcaagtcaataaagacagaaagtagatcagtggttgcctggagctgaggaggtcaaacagaaatggggagtggctgcaaataagaacaggctttcattttgtgatggtgaaaatgttctataattagatattggtgatggttgtactatttagtgaatgtaatatgaataccaaattgtacattttaaactggtgaactttatggtatgtaaaatgtgtatctcttatttccaacaaatgaattttatttttaattttttggggtacatggtaggtgtgtatattcatggggtaaatgagatgttttgattgaggcatacaatgcataacaatcacatcagggtaaatggggcatccatcatcccaagcatttatcttttctttgtgttacaaacaacccagttatactcttttggttattttgaaatgtataataaattattgttgaatagtcaccctgttgtgctatcaaatacaaggtcttattcattttatctaattatatttttgtacacattaaccatcaccatttccacccctgccatacccttccaatcctttggtaaccatcattctactctgtatatccaagagttcagttattttaaattttggctcccacaaataagtaacaacatatgaagtttgtatttctgtgtctggcttatttcacttaacgtaagtcctccaggtccatccatgttgttgcaaatgactagatcttacccctttttatggctgaataatacttcattgtatatatgtactacattttgtttatccattcatcagtcaactgatgcttaggttgtttccaaaagttgactactatgaatagtgctccaataaacgtgggagtgcagattatctcttcaatctactgtttcctttctttgcggtatatacctagcagtgggattgctggatcatatggtagtgctatttttagtttttttgagaaacctccaaacagttctacatagttgttgtactaatttactttctcaccaacattgtctgagggttttctttccttcacatccttgcaagcattcattcttggctatcttttatatataagttgttataactggagcatagtgataacttaatgtagttttgatttgcatttctctgatagtaaataatgttgaccacctttttatttatctgtttaccatttgtatgtcttcttttgagaaatgtctattcagatcttttgcctatttaaaaatcagattattagatttttcattataaagttctgtaagcttcttatgtattctggatattaatgctttgtcagatggatagttggcaaatattttccctcattctgtggcttgtctcttcactttgttgattgttttctttgctatacagaagctttctaacttgatgtaattctacttgttcatttttgctatggttgcctgtgcttgtggggtattgttgaataaaactttgcacaaaccaatgccctggagagtttccccaacattttcttttagtagtttcatagattaaggtcttagatctaagtctaatccattttttttatttaatgtttgtatacagcaagagatagggctttagtttcattcttccacatatgaatatccagttttcacagtacaatctattgtggagactgtcctttccccaatgcatattctgggtacctgtatcaaaaatgagtccactgtagagttgtttcattgctctatgtatgtttttatgccagtaccatgctgttctggttactatagctctgaagtataatttcaaattaggtattgtgattcctctagttttgttcttttcactcaggatggctttggctattctgggtcttttgtggtttcatataaatattaggattattttttctatttgtaaagaacattattggtattttgatagatattgcattgaatctgtagatagttttgagtagtatggacattttaataatactgagtctttcaattcatgaacatggaatagctttccattttttatgtcctcttcaatttcttgcatcaatgtttcatagttttcattgtagagatctttcacttctttggttaagtttattcctaggtatttatgttgtttttatctattgcaaacgagattactttcttgatttctttttcagattgttcaatgttagcatataaaaacactgcttgttttaatgttgattttatatctcatgaccttactgaatttgttaatcagttctaatagttttttggtggagtatttaggtttttccaaatataagataatggaatgtgcaaacaagtataattggacttcttcctttccaatttggatgccttgtgtttctttctcttgtctgatggctctagctgggacttccagttgaacaacagtggtgaaagtgggcatccttgtctttatccagatcttagaagaaaggctttcagttttttctcatttaatatgatgctagctgtgggtgtgtcatatatgactttcattctgttgaggtatattccttcgttaccctgttttttgaggtttcttattatgaagagatgttgaattttatggcataatttttcagcatcaattgaaatgatcatgtcttttgtccttcattctgttgatataatgtatcacaataattgatttgtgtatgttgaaccatccttgcatcccttggataaatgccacttgatcaggatgaatgatctttttaaagtgttgttgaattcagtttgctagtattttgttgaggatttttgcatcagtattcatcagggatattgaccggtagttttcttttttttgatgtgtctttgtctggttttggtatcagagtaatactggccttgcagaatgagtttggaagaattcctttctcttccattttttggaatagttagagtagaattggtactagttcttctttaaatgtttggtaaaatgtggtagtgaagccattaggtcccgggcttttctttgctgggaaacttttcatgacaacctccgtttcattacttgttgtctgttcaggttttgggtaccaaaaataatggcaacaacaacttttcaagacatggagagcaaaataacacatgaattgaaacaagaaaatggcaaaatgtggaggaatgaagttaaaatatagcattttcattatattacactttgcttgttagtttgtttacacaatgtctgttgtcttcagtgtaaaataatgcattataagatatgataaccccaaatccaaaagcattcaacagatacataaaaataaaaagcaagaaattaaaacagaccaccagagaaaatcaccttcacttaaaggaagacaggaagaaaagaaagaaggaagaggaggccacaaaacaaccataaaagacataacaaaatggcaggagtaagtctttatttatcagtaataacattgaatatcagtagactaaactctctaaacaaaatacatagagtggctgaatagatattaataaaacaagacccaacaatctgttgcttacaagaaacattcttcacctgtaaagacacaaatagacttaaaataagagatggaaaattatattctttgtaaatggaaacctaaaaagagaaggagtacctatacttatataacacaggtatatttcaacacaaaaactaataaaagagacaccgattgtctctacataatgataaaggagtcaattcagcaagaggatataacaattgtaaatatatatgcaactaatactggagcacacagatatataaagcaaatattgttagagctaaagagagagatagactccaatacaataatagttggagacttcaacactctactttcagcattaggcagatcacccaggaagaaaatcaacaaagaaacattggtcttaatgtgcattgtagaccaaatgaacctaatagacatttatagaacacttcaaccaatggctgaagaatacacattcttctcctcagcccatggatcattctcagggacataccttatgttatgctacaaaacaagtcttacaaaattaaaaaaaaattatataaacttttctttgactacagtagaactagaaatcaataacaagaataagtttggaaactatacaaactcatggagagtgaacaatatattcctcaatgaccactgattcaatgaggaaatcactaaggaaattttaaaatttttcaaaacaaatgaaaatggaaacacaacaaaccaaatcctgtgtgatacagtgaaagcagtactaagagaaaagtttgtaagagtaagcacctacattaaaaaagaaaaatttcaaataaacaacataatgatacatttcaaagaactagaaaagcaagagcaaactgaactgtaaattagaagaaaaaataataaagatcaaagtagaaataaatgaaactgaaataaaaaaatacaaagcatcaatgaaataaaatgttgtttttaaaaagagaaaattgacaggccaggtgcagtggctcatgcctgtaatcccagtactttaagaggacaagtcgggtgtatcatttgaggtcaggagtttgagaccagcctggccaatatggtgaaaccccgtctctactaaaaatacaaaaaaatattagccaggtgtggtggcatgcacctgtaatcccagttacttgggagactgaggcagtagaatcacttgaacctgggaagccgaggttgcagtgagccaagattgcatcattacactcaagcctgggctttgcagtgagactttatctcaaaaaaaaagataaaattgacaaacctttagtcagactaaggaaaaaagagtggagactcaaatgcgtacagtcagagatgaaaaaagagacattgccactgatacttcagaaatttaaaagattatgagatgctactatgagcagttatatgctaatgaattggaaaacttagaagaaatggataaattcctagatacatgcaacctatcaagattgtaaaatgtctcttgatagagctgtttaaaaaactacaagtctttacatgggggttaagattttctcttaatttcatttattgtagggcttttagtaatctaaattttatttttgtatagtctagctatattttctacaggagaaacagacttagtctatatatctccgtaggtcttcttaggtttccatggtattactaattgttatgtctatagagtgctgtgaaacaatcctatcaatagtttctggccaaacacttgtttgactaagccacaaaggcacctgctccatagatatgaggatatatttctagattgatgcctatctggctacattctgtagtctgggtttactggtgttaattaactcagtttgtgtgtttcttttgttatctaaatgtagatggttctttatacctggccatagaattatgacttatgcatcttatggtggttaccttgaaattagaacaaacctgagctctaatctggggctgactttcctcagtcgtctctctacattctgtgttgacaatgctaccatgtgaaggcctaaggaatacaatgttcatcaaataattaatcagactttgctcacatatgaattagttctgtttgctggcctatcaagcagaagtattttaaacagttgtgagaatgacctttaccaaatcattttaaacacaaatccaaaaagcttccacccatgcaccccacttttatggtgtatgtttattttgggttttttttgcttgacagcatgcaagttcctagaaattttggttatacttttaaagaaagtattaccttacttaccttactgttaagttattgcttacagggtagtacatgcaagtcctgcacaatatcttaactactagttattgattagaaaggaaaacacaaccatggttgagaaaatatataagacacctgaggaaactatgaactcttttgagtagtttatgtttacacgaggagactttgtactggtactcccttccacttatttatgtttcatagtttgctttaaaaaaatcatctcaaagaaaatattatctcttgactagaaaaaagaaaaagcaactggaagagaggtgactcacattcagttcaccagctggccagaccacggggtgcctgaggatcctcacttgctcctcaaactgagaaggagagtgaatgccttcagcaatttcttcagtggtcccattgtggtgcactgcaggtaggaaaaacgaacaaaaaaaaaaaacaacaacaaaaaaactccaacagaatccacctgcctagggctgttagagacatctttccctttggcaattgctattttgggaaacaacctatgggagaagcttagattcttatattggcttcacacctgacagcttttccatgatcatgcctctgcttttttttgcttggtttgccagtgctggtgttgggcgcacaggaacctatatcggaattgatgccatgctagaaggcctggaagccgagaacaaagtggatgtttatggttatgttgtcaagctaaggcgacagagatgcctgatggttcaagtagaggtatgttctaacctttagtgattattctcactttggttttttggacttaaatcttttccaagtgataataatgatattttttaaaaatccaaattcttcacaacctcaaacagtagatgatttcctgaaaactaaaacgtggtaatcaccagaaatacttagaagcatttttcattagtgcctaaaagtactgtggaagaaagatgaccacaaaatatataatttttaaaataatgaactactgttaacatatatcagattggcaaaaaaagtaaaaatgctgaaaatagatttggcatcatctcataaaattaaactgaagagacagaatagtatagtaatcaacagctggttttagaaactacacttacaggtttcaaatcttgcttttaattattaatacgagggtgagtggtattgtttattaagtaattttagtctgactgcacctcagttaagtcatctgtaaaatggagacaatgataatacctcacagacttataaccacaaaagtaatacaaataaagcacttaaacaagtccctggcccatgctatgcatttggtgattgtaagtgatggtaattactgaaaatgtctgtatttgacccagcaaaatcacatatatgcatatacccaagagaagcatcaactagaaacatttgcaagaatgtgcattgcattcagcattgtcaaaatagcaaaaaaaaaaaaaaaaaaaaagtgaaatacatatcaatgaaagaatggaaacaccgtaaatatgtatcaataggggaataggaagacaaaatgtggacatgtgaactctctgtacaacaaatgctatgttgtggtagaaagcaatgatctaggtttgtgtctgtctgtttggagagatgctcagatgaaaacaatgagtgagtaaagctgccatacgaaacattcaagatataatttatgtgatttaaaaaaaacatgaaaatgtacaatgcttgtgattacagatacatagatagcagtgtagaaacataaaaacaaattgttaaccaggtaaaaagaaattatttacagtggaaaataaagtacagtggaaagacagtgccaaactcagggaactaaaggtggcggttaaagaggattatcagaagtataccatttccttgaaaatactggattcaaacaaaataagcagtaaagagtagttaaatctgggtttggcccattggattacaaaaaaataattttcttattaaaagaatacttttcttattttaagttctaaaaactataaaaaaaggttttctaaggaataacaacttgcttttttatctcttgaatatactgtgaaatttattatagttttacattcagtaatttggcttactgacccaataatcactaaaggaagtaacatacaatgttctttagtttttaggaataaaagttgtgcaatacagagtacatggataatctatttgcaaagtaattcttttctgaaaaaataatctgaaaatagaatttgctcatattccagaaaactctgagagtgaacttccagaatatttaaatattatagatatcaatttactttgccatgaattgttccaatatgagcaaatttatggggaatgtatattttatttaaatatgacttggaggactctagattatcagttaactatctgtatttgttcttgaaattgtaggcccagtacatcttgatccatcaggctttggtggaatacaatcagtttggagaaacagaagtgaatttgtctgaattacatccatatctacataacatgaagaaaagggatccacccagtgagccgtctccactagaggctgaattccaggtaatgatagtgacaacaataataataattacagataacttttattcagtgtcatctactttctaggtgtttgctatgcacttgacatagtgcttgcatttagtcttcaccagaaccaaaggagcacagatgagaaaactaggacacagtgagttaagagaaatgcctgaatctacacaactattacataggagatttctttagacccagaaatctgattctattgctaatacttttagccattcctcattaagctggtataaaatgaagtgtcaaaataatagtatatagccacaaaactggtctgccaaaggcaatacagcatatcacctttaaaaatcgtatctggttttggtttgtaaaggaaatcattagaagagtttatgactgcttaggaagttgaactggctggagctggtagacacacagtaaaggataagtacatgtgtcttaacctatttattaggcaattattctcacagctaacctagcatgtagttcactataatttcagagagtttgcatagctgtcctcaaattgctcagttgtcaaaaaaatgttttgtgttttttttgttccacctatgatttccaggttactgagtcattccataatctaccaaactggtaaattcagagtttctaaagaccaggagtgtgcttttaatcacatgcagaaccatttaatgtttaggatcaaagtggggttaaggtgggggtggaggtggagcatgcaataatgaccaagtgactcaatcccccagaagacctgtacttataatggaagaactagcagacacagggtagtctcaaacagagtagtgttttattgttgttttcttgcttttctagctgataaattaaccttattcaatatacctgccctactaatccacataaacacataagctgttagagacagttatacatttaagttaaacattcttatgaatgtttatttactatagaaaagacagacaatttttttcactaaataaatgtgcttgagtttctgctatgtgccaagtacaattctaggcacaagagtcaaaatgatctgcaagtggacatgggaagaaggatgagaggatgtgatccagatcacagatggaagctgtgaaattattccatttaagcagacagtaagacagaagatgagagtagaaatgcaagtcggttggtaaatttggtattgggaagttgaggcagctcttgcctgatgatctttcatttttcaagaaaatgtgaggctaggtcatcagttgagagttgagagatacaagggcgagtagggcaaagaagagctcaatgcttgaagggtataaactagttacctcaaagtataaaaacaatctccctaggcagaggcagtaagattgccagaagttatcatttgatcacctgaaatttatgattataagtttaaagaggaattagtcagttggttgtattgttttctatggcagcattgagctctttgggggtagaggctgtgtatgcagatagttgagttaaacctatctaggttttgaaaagtgactatttgaaaatagtgaggcaaacgagttgagggtgtttacaaatgaatgatgactgaggtggaaaataaaaagcaaattggccacatgagggaggtgagagaaagtagtaaggataataagttggagactttgatagaattacagattgctaggttgaacatatcagaataaatgactaggaataataggggtaattttcaatagcacagatagttgaacttatgattttagaggtgatgtaatatttggaatgaaacctacaaaggtggaatgatgaaagtggatgactgggaagtggagggaaagtcatgggaggtgaagaagctaagaaatgaagagactagagtcttggatagattattcttgtcaatgttgaattaaccaaaaatgatgacagaccttggaaagaagagaatatacttagccaagcctaaaactaaatgaggtggagtgattcagaaatcaatacctgacacttcccagtgaagccggtggatagaagctagtatagtatgatggcaggaatatcaaagtgcttggttgatttgaaagcaaatgagtagaaatggtttgcaagtagaatcagggatcaaggagaacacgtatcttttcttgaagctgtgaggtaaatggggtgtgaggaggaaagtcaactttttcttaaaagggctgctgagttattggtggtgtccttagctgacatccaggttttaattggtggaaagaaaaaaaaaagggtgaagtgactgttgggagaagatgattaagataaatgggagttcacagatgacagacgatgggcatcagagggcagggaggaaggcactgatgggttagatgtaagagactgggttgtatctgaggatacaaataaccattcaggaataaaaatctggggaatgtggatgcactgggaagcttagacttgtgatggcaagtgaaacaggtagagatttaagagtgacagatcctttgtgtcttagatgaaggtgagccattaattccacctataatcctgagtattgctacagggcataggctgcctcggtgactacactcacaagagcacaaggtgttgtaacagtttccaaaacatctggtccttcatgcagctcatggtggtgttcaagtggcctaaaattcagtgatgatattttctttcactcaattacgtagcaaagaatgaggtttgaaacagggtgccataattagtttgaatgagggtactatgctgaaaaaatatatgtctatatacacacacgtatctacatgcgtgtgtgtgtatataaaatcttaccgaattgtacatgaggagccttctcagtttcagttatttgtaacattatctattatcattaaatattattcacttgacaaatacttatttaaggactagtggaaagactgtaggcaggggtgtcttccagaagaaattggtatttaaactgatacctagagggtaagaaaagttattagagcaaccaaaaggggaaagggtagttcaagcaagaaaaaaaaaaaaaagtgtttatgtgccaagagttgaagaacagcttggcccttccaagaattgaggaagctggtttggtagaagtattgagggacccagtaaggtgtaaggctggagaaacagtcaggggcgtatcaataaagactttttatgctattttgaggaggtttgttgtcctcttatagtgatggaaagctgttcatcttcagaagagcatcttctgttttgtgttttagaaggattagagcaggcgagattgaagacaaagaggccagttaggaaattgttgatgttttacaagcgagaaatgaaggcagactggattaagtaggaagaaagaaaactaaaaggatttgtgtatagaaatgatggatcttttctgactaattaggaactgtgggtgagaggaaagcaatctggaaggtgtaaacaaattaagaatgaactttcaaaacatgtgccaagtctcctaagaatgtgttgtctccaaagtttatttctgatcatttaaaataacttaccattgcttttgcaatatagatcaacatcggtctagtggtttcaatttatataagaacaaactatattatttttctatcaagcagctctgaagaaggagacatagtctgttacatatatatctttagtgcatactagccctgtcaaaaggactaaatgcctgagcaatttaaagaaaaaaaatcagaggcaaaccgaaaaattatggcctatagggagcatatgcaaatttcacaaaaattaatgaaatgcttttccttagggagcatcttatgatgcaataagccaatatttacattttaaaggagtttttctgttttttttttttttttcagagacttccttcatataggagctggaggacacagcacattggaaatcaagaagaaaataaaagtaaaaacaggaattctaatgtcatcccatgtatgtagtttatttttttattttttgtatcagataaagttaagctcttttggatttgtttaatgtgggacacacagtcatataaattatcttgaagcaagttttcaacatttggttgttaatagggaagaagttactaggtattaaaatactagttattgcaagaacttataatcctgaacatttacaatgggctttggagggtagactgtattcagtgttttctttttaccaattatttcagaaatgggttgtcataaaagagaaatatataaagctgggagaaaaaagagcaagtctcttttacccattttctttcatttttagtttatttcagttatttactccagggtaattgacaaatagtaaaaattacatccatttgttctctatatgtttcctttttatcccttataactgggaggttgaaagtaaggggaaaatactctataaattctaaatcttcaaatttaacagatcaaaatatgcacagtttcaatacttgaattctactatttaagcatattaaaatgatcacatatggtaattttattcagctgcataaactaaaattagcatggataaaatataacacaagttgataaattagatgaccaaataaatcagatcagtgcatggttgacctagttaattttcataggagtccttatgaatgtagtttaaaatatggaattgatggtgatatggttaatcaaatcatttgaccaagttattataaattatagaaattaagaaacagtgagaaattataggtcaaataattttctgggctaaataattaatcaaagctacccatataagattgttaatttaatattactggagtataattgagggaaaaaatctacgctatgtattttgtaaacttatatcaagcagaattataatagtccatgggaaattaaagtatatgtatcaaagattaaataatcatatataatgatatgatatctctttgttgtttgacatggaattatgttccatgttttttcctggaatcctttttcttagacttttgttgtataatttgtttatcgacaagtactgaattttatataggatcttatttcatgtagatcagtaagttttcataatacaatctgtccctttttaaatactttcaaatttccacatgacaatgaagaagaaatttaattttttcaaggaagacttactactgatttatttcacatagatgactataacagagtgccacttaaacatgagctggaaatgagtaaagagagtgagcatgattcagatgaatcctctgatgatgacagtgattcagaggaaccaagcaaatacatcaatgcatcttttataatggtaggtacttaaattgccaaaacccaagatccaaacattttaaaataatatctatgttattagggccattcattaagcgattttataaaagaataatgagcttggtcataactacatatagattgacatgagagtttcaatttcaatgctacaatttaacttaatgaaagatttaaaaatactataacctaataacctgagacaaaataagataatgctattggttatattttatgacaaatatagctataatcacatcaattttaaaaatagtaaaatttgagcaaatacaagtatttgaaaatgtttatacatactcagatacccaaattgtaggcaatgacaaatttgtatatttgtatggttagaaacttttcattcagataaactgaattattaggtgagtctgtgtcatatccccccacttttttaattaactgagaattcaaacaatgaaactttagtcatttattaaatatttattatttatacactgttggatttacttattttccaaagtttcctaaagcacacattcatagaatattagtttaattaggaaatataataagaatgtaaagacactaattaaaattagtatagacacgatgaaggtaatttgaaatgcttaagtaattcctttttacaatcacattaacctttatagagaaacaaaaatgtgtgtcttttgtggaaaggaaaatttgtttcgcaagatatgttgtaatcttgatttcacattattagctaagaattactattatctgtataattattttacatatagctattacattgtttcttgtaagaaacataagaatattactatttgtatgtaacagcattgatatcaaactgactatatttccaaatggttactttaagaatctactgagctctcttctgtagtaacgaagtcccaccctttttttgtctaaaaagagctactggaaacctgaagtgatgattgctgctcagggaccactgaaggagaccattggtgacttttggcagatgatcttccaaagaaaagtcaaagttattgttatgctgacagaactgaaacatggagaccaggtttgtacttttgaggattttcttttaagcctttctgtcataaaacgtcattctctagtcttggattgcttgcttcatcgccatacccacgtctttttttatccctccatcacataattctgtctgctcagtcttacccctttcaccctggtgttggcctccatcagctgtgtctggattctgacagtctctcctgtttgtcccctccagtcttgcatgctgctcacagattagccaggatgcagcaatgtcagcgtcacagcaaataacagctacattttcacgctgttttcctcattttctcaagataaaagccaagatctttttgtgatatccagcaccctggacaatcaccccctcatgtgtctttcatcttcctcccatttttatgttttccatcctctccactctggacaagcaggtttcatgcccaagcctaaacacgccatttgcattgtcatcactgagtctaaacttattgatattccatgtaactaaatgtgtgctgtcttccagttttgaccctattcttttaacaagaccaaactcctgaaaaatgtatctatatcatcctttctttattcccatataatatttattgccataaaagtctatagttgaaggtgaatctaagctataatttgatttttttacttaatgcttgtgacagatattttatccttttcttaatgtcttcagttattattaaaatttccctggtggtagatctcactcagctttagcaccaaccacattatctgacatatgttcaagcctattcagtgaataaccttataagtatgcaaaagatttatgcttttttatgcccctctctctcccctaaatctcactctttctcaccctcacctggtccccttcccctgtacatggaaagttgctttttatgttttttgttttaaaggaatataagtccagatttctagcatggaattcccacaatcctttccttcatataaattgtgaaagctgggaaacaggatggaagtaccggcaggactccctgtctttgtcagaaattgtggggttgtagttggtagacaacagtttgtagtaagaagaaacacttttgtggttcatctactcttcaatctggccctttccttagctatgtagacaaaatatataaagctgcttatggtgttggtcaacaagatgacagagacaaagctccaaaagatgcagcctccttcctcaagaaccactgaagggacagtgggacctgagttattgaaagggtcatgaataacattgactcatgccagccataaatattgaagaggtcatgataagcatgtggaaaagaggagcaaacctcaaagacctacactaaggaaaacagctgttccgggggtgtcccagtcacctcgattgtgctcagcttcccttttcttacacaaggaaacaccacatatttattaaatgggtcgccagcacttaaatagattctggatttttataagtaggtttcaattttagaacacaataattttcatttaatagaaaagaggcacagacagagaaagaaagggagaaagagggagactgatcctttgcatatttcaaataggaaacaaattgttgaattgtcttcttttatctaggaaatctgtgctcagtactggggagaaggaaagcaaacatatggagatattgaagttgacctgaaagacacagacaaatcttcaacttatacccttcgtgtctttgaactgagacattccaaggtatggaaacaatttggggagtatatttctttgatataatggatctggtagcaaaatgaatataaattactctatgcaggcaaggccatcatataaataatgtttcagaataacattttaaaattatttaaatagaagtaactgtgaagaaaatatgactatcaaattagaaaataagctgaacttcactccagttaatgctctcttcaattctgattttagaggaaagactctcgaactgtgtaccagtaccaatatacaaactggagtgtggagcagcttcctgcagaacccaaggaattaatctctatgattcaggtcgtcaaacaaaaacttccccagaagaattcctctgaagggaacaagcatcacaagagtacacctctactcattcactgcaggtgcgtgggatttggtagaatgtgctctcaaaatcataatgcttgacttctcggttcacatgttgtcttatctagttatcctcatatatgaaacacataaccacagtaaaaacttcttatggagtcggtcactctcttggttgtttccacaacacaactattgtagaaatataatagaagtgattatattatagtgcaataattttaagttgtgttttttaatacttggtgtcatgtcatctttgattccttggtagctaacattgagccaggaatgtcatttgtgtgaatgaattaatgaatggaagggtgtgtgaacagataggtagatgggtatcaccttacacatatacccatatacattgatctactctattaggtgtcacaaagacacctaatatgtttaatgaacacaaagtttattaaacatattttaagttaaatattaactgaaatcacaaagcttagcaattttgatttgaaactcattatttaattttctaaactgaaccaaaggcaaagattgtggtaatatcaataatactactagattttattagtttcttcatctgtgataggtgcttacatattcaccttaaataagcaatataattgaaagaaagatatataatataaaagtttacatgaaaaagaatattgaagtaaatgagaaacgaaaaatagtaaagtaaaatgagaaatgtttatctagtgaaaaacttttggaatttttgaaaaagtctaattgttattattggaattgcatatactagaatcaagccttaagaaatatatgaattttcagcatttatgtggaaagaaagctgaggaagggaagtttacactgtaaaactatatatgtttcttagaatatgatttatgtacaataactaaagtgtcctgctgataacatattgtttaaattgaatctttatgataatgctttatacttctcattgtttggtaaactatttgattgccctctttttagtgaataattctactaggtattacttttctactgatgcagaagtgaaaacatttgtgaaacgtggtagagaggcagaagagtgaagaagagcatgtgttctagtaatttacaaaatattaggtctaatatttctgattacatcagctttctcttctccaaatcttggtttccttatctatcatactggcattctgatattggtttcaacaacttcagatgtaaataaaaatgcattaaaatccataaaatactaaataaaagaaaatatatttgtaaagtcgaagacaaataagttttcaattccaggattatcacactcttaaattgaaaaatttgcctaaaaatgcatttagcgtaaataatttggttcttgaaagaggttggaataagataattatgataaacatgaagcaaaaaatatattctctctcttcctgtttttattctaatatcaccctttttggtgagaagtaggattattttctatcttttctttcttttatagggatggatctcagcaaacgggaatattttgtgctttgttaaatctcttagaaagtgcggaaacagaagaggtagtggatatttttcaagtggtaaaagctctacgcaaagctaggccaggcatggtttccacattcgtaagtatccttcaccattgcttttaacatgctcggaattttttttttctttttgacggtttccttttttcttttctcctctcctttcctctcgtttgttcttttttcccctttccttttctcttctctattttctttcctattcttttagcttttctacttttacatgataattcacattaaattattataagtctaaataagagcctaaagtttactagcactttgttgtgacagttcatgaagagcctttccctaaatgctcatgaatttcttaattttctttccttcactcctgtatcgatttgtgttgtgtaacaaaccacccccaaatttgggagcctaaacaaataacatttattatggttcagtagtctaatgatatgctggaatgttctgctggtgccctcaggctcaggcaatagagaccaggctgactcatgtgtctgccttcagctgatgtgtgccctacagtttggctggtctaaagtgacctacactgccagtaggctggcatgtggctgccatttagctatggcaacaacagtgagtgggccacatgtccctcctcatccagaagactagcccaggcctattcacattaaagcagcaagttccacaagggaaagaagacttgtgtgagaccacttgaggcccaggcttaaaagtgacacacatgtcttcttctgtatgttattagccaaataaataagtcataaagcctgcccagattcaaggggtagggaaatagactccacttcttgagagggcctgcaaattcacattgcaaagaaatgtggatacaggaaggaaaataagttttatattcttgtaatcgatctatcgtgtataccctctatgtggtagtaactgtagatggtcatctgggaattaatccttattcacagtgtaaacttaattactcactaaaatatataaagcttttaatcatgtatgatattgagatttcatatcttggtacttaaaaatgtatcaaatgcttgctatgtgctcttgctataaagagctaattggtatgagggaaagccaggtatttactaatcaatgtagtgagtaaaatgacagaaaaattataagaagaacatgaatgagggcatttaatttaaactttaggaatcaagaaacgcttctcgaagcagtgattcctgccctgattcttaaataatgtgtaggcattagacaggaggataagtacaaaacgtggcatcatgagcaaaggcatggaaatggcccatgagcggagtgaacactggtttggggttgctccaaggtaaagttcaaaaagtatcctgcagtcaaccctttagcaccataaagaaactaaattatttagatgtttttatgagaacatatcaaaaagtacttttctgtcatccaatacttccacaaataaatcattagttcttgctaatcttcatctggcataaaaataatgacatcaactttcttcatgtaatttcccacttaattcctttactaggagcaatatcaattcctatatgacgtcattgccagcacctaccctgctcagaatggacaagtaaagaaaaacaaccatcaagaagataaaattgaatttgataatgaagtggacaaagtaaagcaggatgctaattgtgttaatccacttggtgccccagaaaagctccctgaagcaaaggaacaggctgaaggttctgaacccacgagtggcactgaggggccagaacattctgtcaatggtcctgcaagtccagctttaaatcaaggttcataggaaaagacataaatgaggaaactccaaacctcctgttagctgttatttctatttttgtagaagtaggaagtgaaaataggtatacagtggattaattaaatgcagcgaaccaatatttgtagaagggttatattttactactgtggaaaaatatttaagatagttttgccagaacagtttgtacagacgtatgcttattttaaaattttatctcttattcagtaaaaaacaacttctttgtaatcgttatgtgtgtatatgtatgtgtgtatgggtgtgtgtttgtgtgagagacagagaaagagagagaattctttcaagtgaatctaaaagcttttgcttttcctttgtttttatgaagaaaaaatacattttatattagaagtgttaacttagcttgaaggatctgtttttaaaaatcataaactgtgtgcagactcaataaaatcatgtacatttctgaaatgacctcaagatgtcctccttgttctactcatatatatctatcttatatagtttactattttacttctagagatagtacataaaggtggtatgtgtgtgtatgctactacaaaaaagttgttaactaaattaacattgggaaatcttatattccatatattagcatttagtccaatgtctttttaagcttatttaattaaaaaatttccagtgagcttatcatgctgtctttacatggggttttcaattttgcatgctcgattattccctgtacaatatttaaaatttattgcttgatacttttgacaacaaattaggttttgtacaattgaacttaaataaatgtcattaaaataaataaatgcaatatgtattaatattcattgtataaaaatagaagaatacaaacatatttgttaaatatttacatatgaaatttaatatagctatttttatggaatttttcattgatatgaaaaatatgatattgcatatgcatagttcccatgttaaatcccattcataactttcattaaagcatttactttgaatttctccaatgcttagaatgtttttaccaggaatggatgtcgctaatcataataaaattcaaccattatttttttcttgtttataatacattgtgttatatgttcaaatatgaaatgtgtatgcacctattgaaatatgtttaatgcatttattaacatttgcaggacacttttacaggccccaattatccaatagtctaataattgtttaagatctagaaaaaaaaaatcaagaatagtggtatttttcatgaagtaataaaaactcgttttggtgaa

SEQ ID NO: 12 - DNA, 22 bp, Artificial Sequence
  sgRNA Target sequence
ggcttaaactcttggcatttgg